European Patent Application EP 4 220 176 A2, published August 2, 2023. Title: BIOMARKERS. Applicant: ST GEORGE'S HOSPITAL MEDICAL SCHOOL. Application EP 23164742.1, filed February 27, 2018. The sequence listing filed with the application follows.

SEQUENCE LISTING (69 sequences)

SEQ ID NO: 1 - protein, 179 aa, Homo sapiens
MAKTAMAYKEKMKELSMLSLICSCFYPEPRNINIYTYDDMEVKQINKRASGQAFELILKPPSPISEAPRTLASPKKKDLSLEEIQKKLEAAEERRKSQEAQVLKQLAEKREHEREVLQKALEENNNFSKMAEEKLILKMEQIKENREANLAAIIERLQEKERHAAEVRRNKELQVELSG

SEQ ID NO: 2 - protein, 187 aa, Homo sapiens
MAKTAMAYKEKMKELSMLSLICSCFYPEPRNINIYTYDDMEVKQINKRASGQAFELILKPPSPISEAPRTLASPKKKDLSLEEIQKKLEAAEERRKSQEAQVLKQLAEKREHEREVLQKALEENNNFSKMAEEKLILKMEQIKENREANLAAIIERLQEKLVKFISSELKESIESQFLELQREGEKQ

SEQ ID NO: 3 - RNA, 2232 nt, Homo sapiens
  source 1..2232: mol_type = mRNA
agctcctaggaagcttcagggcttaaagctccactctacttggactgtactatcaggcccccaaaatggggggagccgacagggaaggactgatttccatttcaaactgcattctggtactttgtactccagcaccattggccgatcaatatttaatgcttggagattctgactctgcgggagtcatgtcaggggaccttgggagccaatctgcttgagcttctgagtgataattattcatgggctcctgcctcttgctctttctctagcacggtcccactctgcagactcagtgccttattcagtcttctctctcgctctctccgctgctgtagccggaccctttgccttcgccactgctcagcgtctgcacatccctacaatggctaaaacagcaatggcctacaaggaaaaaatgaaggagctgtccatgctgtcactgatctgctcttgcttttacccggaacctcgcaacatcaacatctatacttacgatgatatggaagtgaagcaaatcaacaaacgtgcctctggccaggcttttgagctgatcttgaagccaccatctcctatctcagaagccccacgaactttagcttctccaaagaagaaagacctgtccctggaggagatccagaagaaactggaggctgcagaggaaagaagaaagtctcaggaggcccaggtgctgaaacaattggcagagaagagggaacacgagcgagaagtccttcagaaggctttggaggagaacaacaacttcagcaagatggcggaggaaaagctgatcctgaaaatggaacaaattaaggaaaaccgtgaggctaatctagctgctattattgaacgtctgcaggaaaaggagaggcatgctgcggaggtgcgcaggaacaaggaactccaggttgaactgtctggctgaagcaagggagggtctggcacgccccaccaatagtaaatccccctgcctatattataatggatcatgcgatatcaggatggggaatgtatgacatggtttaaaaagaactcattataaaaaaaaaaaaacaaaaaaaatcaaaaattaaaaaaaatcaatgcggtctctttgcagaatgttttgcttgatgtttaaaaaataccttggatcttattttgtaaatacttacatttttgttaaaaaatacaagtattgcattatgcaagttatttcataatcttacatgtcctgtaacaggcttttgatgttgtgtctttccactcaaatgaatttgctaggtctgttctttttgaagctccccatgtctaactccattccaaaagaaaaatgaggtcagtagacagtctatggtgctagaaacccaccattgcctaatgacctagaaggctttgttgtctctgagcttgactaagaccatacctagatcacaggtattatgactccacatgaaccttcacatttgttcgctcataatctacttactgcctaaaaactacaaaaccaggctaagaaataccaccagtcatagcatttacttctgcttctcctggattatgtgctacaaatgtgctttggctttagaaagggatggatgagaagacagacctgagaccaatctgggtagaagcaaaaagttgaaccttttaaagtgctgaacacaaatccaaattcgaatggttcaagcagccgtgaaatcgctcttcataaagtgggcttaattctctagtttaagttcttttgatggaatgaattaattaatgtgtcaggtggcttatttgtggatgccatgattgatgatgttcattttaagctcttacctatagtacaagtacatgatgctactgaatatttttccacttggaaactgtgagctggttgttgcattaaaacacacatacaaacaaaatcaaaaacactgcggactttcactcaagctggtctttcttccccagtgtaaggcaatcctgcctactaacaacaccaacaacaaaacactccatctgtgaagctgacgcagttaagggggctaggcagggcatttgtgccaactaagaatcaccagatacccaccataagtacctatcgcagttttgaagtcgtttctccccaactcccaactcctgaaggttgctgcctgcatatttactcttcattagtgctattttcctgtatgtcattgtgagcaagctgtgattaataaagaattggagttctgtgaactaataaaggtttggtctgttaaaaaaaaa

SEQ ID NO: 4 - RNA, 2314 nt, Homo sapiens
  source 1..2314: mol_type = mRNA
agctcctaggaagcttcagggcttaaagctccactctacttggactgtactatcaggcccccaaaatggggggagccgacagggaaggactgatttccatttcaaactgcattctggtactttgtactccagcaccattggccgatcaatatttaatgcttggagattctgactctgcgggagtcatgtcaggggaccttgggagccaatctgcttgagcttctgagtgataattattcatgggctcctgcctcttgctctttctctagcacggtcccactctgcagactcagtgccttattcagtcttctctctcgctctctccgctgctgtagccggaccctttgccttcgccactgctcagcgtctgcacatccctacaatggctaaaacagcaatggcctacaaggaaaaaatgaaggagctgtccatgctgtcactgatctgctcttgcttttacccggaacctcgcaacatcaacatctatacttacgatgatatggaagtgaagcaaatcaacaaacgtgcctctggccaggcttttgagctgatcttgaagccaccatctcctatctcagaagccccacgaactttagcttctccaaagaagaaagacctgtccctggaggagatccagaagaaactggaggctgcagaggaaagaagaaagtctcaggaggcccaggtgctgaaacaattggcagagaagagggaacacgagcgagaagtccttcagaaggctttggaggagaacaacaacttcagcaagatggcggaggaaaagctgatcctgaaaatggaacaaattaaggaaaaccgtgaggctaatctagctgctattattgaacgtctgcaggaaaagctggtcaagtttatttcttctgaactaaaagaatctatagagtctcaatttctggagcttcagagggaaggagagaagcaatgagaggcatgctgcggaggtgcgcaggaacaaggaactccaggttgaactgtctggctgaagcaagggagggtctggcacgccccaccaatagtaaatccccctgcctatattataatggatcatgcgatatcaggatggggaatgtatgacatggtttaaaaagaactcattataaaaaaaaaaaaacaaaaaaaatcaaaaattaaaaaaaatcaatgcggtctctttgcagaatgttttgcttgatgtttaaaaaataccttggatcttattttgtaaatacttacatttttgttaaaaaatacaagtattgcattatgcaagttatttcataatcttacatgtcctgtaacaggcttttgatgttgtgtctttccactcaaatgaatttgctaggtctgttctttttgaagctccccatgtctaactccattccaaaagaaaaatgaggtcagtagacagtctatggtgctagaaacccaccattgcctaatgacctagaaggctttgttgtctctgagcttgactaagaccatacctagatcacaggtattatgactccacatgaaccttcacatttgttcgctcataatctacttactgcctaaaaactacaaaaccaggctaagaaataccaccagtcatagcatttacttctgcttctcctggattatgtgctacaaatgtgctttggctttagaaagggatggatgagaagacagacctgagaccaatctgggtagaagcaaaaagttgaaccttttaaagtgctgaacacaaatccaaattcgaatggttcaagcagccgtgaaatcgctcttcataaagtgggcttaattctctagtttaagttcttttgatggaatgaattaattaatgtgtcaggtggcttatttgtggatgccatgattgatgatgttcattttaagctcttacctatagtacaagtacatgatgctactgaatatttttccacttggaaactgtgagctggttgttgcattaaaacacacatacaaacaaaatcaaaaacactgcggactttcactcaagctggtctttcttccccagtgtaaggcaatcctgcctactaacaacaccaacaacaaaacactccatctgtgaagctgacgcagttaagggggctaggcagggcatttgtgccaactaagaatcaccagatacccaccataagtacctatcgcagttttgaagtcgtttctccccaactcccaactcctgaaggttgctgcctgcatatttactcttcattagtgctattttcctgtatgtcattgtgagcaagctgtgattaataaagaattggagttctgtgaactaataaaggtttggtctgttaaaaaaaaa

SEQ ID NO: 5 - DNA, 540 bp, Homo sapiens
  source 1..540: mol_type = other DNA
atggctaaaacagcaatggcctacaaggaaaaaatgaaggagctgtccatgctgtcactgatctgctcttgcttttacccggaacctcgcaacatcaacatctatacttacgatgatatggaagtgaagcaaatcaacaaacgtgcctctggccaggcttttgagctgatcttgaagccaccatctcctatctcagaagccccacgaactttagcttctccaaagaagaaagacctgtccctggaggagatccagaagaaactggaggctgcagaggaaagaagaaagtctcaggaggcccaggtgctgaaacaattggcagagaagagggaacacgagcgagaagtccttcagaaggctttggaggagaacaacaacttcagcaagatggcggaggaaaagctgatcctgaaaatggaacaaattaaggaaaaccgtgaggctaatctagctgctattattgaacgtctgcaggaaaaggagaggcatgctgcggaggtgcgcaggaacaaggaactccaggttgaactgtctggttaa

SEQ ID NO: 6 - protein, 961 aa, Homo sapiens
MLAPRGAAVLLLHLVLQRWLAAGAQATPQVFDLLPSSSQRLNPGALLPVLTDPALNDLYVISTFKLQTKSSATIFGLYSSTDNSKYFEFTVMGRLNKAILRYLKNDGKVHLVVFNNLQLADGRRHRILLRLSNLQRGAGSLELYLDCIQVDSVHNLPRAFAGPSQKPETIELRTFQRKPQDFLEELKLVVRGSLFQVASLQDCFLQQSEPLAATGTGDFNRQFLGQMTQLNQLLGEVKDLLRQQVKETSFLRNTIAECQACGPLKFQSPTPSTVVPPAPPAPPTRPPRRCDSNPCFRGVQCTDSRDGFQCGPCPEGYTGNGITCIDVDECKYHPCYPGVHCINLSPGFRCDACPVGFTGPMVQGVGISFAKSNKQVCTDIDECRNGACVPNSICVNTLGSYRCGPCKPGYTGDQIRGCKAERNCRNPELNPCSVNAQCIEERQGDVTCVCGVGWAGDGYICGKDVDIDSYPDEELPCSARNCKKDNCKYVPNSGQEDADRDGIGDACDEDADGDGILNEQDNCVLIHNVDQRNSDKDIFGDACDNCLSVLNNDQKDTDGDGRGDACDDDMDGDGIKNILDNCPKFPNRDQRDKDGDGVGDACDSCPDVSNPNQSDVDNDLVGDSCDTNQDSDGDGHQDSTDNCPTVINSAQLDTDKDGIGDECDDDDDNDGIPDLVPPGPDNCRLVPNPAQEDSNSDGVGDICESDFDQDQVIDRIDVCPENAEVTLTDFRAYQTVVLDPEGDAQIDPNWVVLNQGMEIVQTMNSDPGLAVGYTAFNGVDFEGTFHVNTQTDDDYAGFIFGYQDSSSFYVVMWKQTEQTYWQATPFRAVAEPGIQLKAVKSKTGPGEHLRNSLWHTGDTSDQVRLLWKDSRNVGWKDKVSYRWFLQHRPQVGYIRVRFYEGSELVADSGVTIDTTMRGGRLGVFCFSQENIIWSNLKYRCNDTIPEDFQEFQTQNFDRFDN

SEQ ID NO: 7 - protein, 935 aa, Homo sapiens
TPQVFDLLPSSSQRLNPGALLPVLTDPALNDLYVISTFKLQTKSSATIFGLYSSTDNSKYFEFTVMGRLNKAILRYLKNDGKVHLVVFNNLQLADGRRHRILLRLSNLQRGAGSLELYLDCIQVDSVHNLPRAFAGPSQKPETIELRTFQRKPQDFLEELKLVVRGSLFQVASLQDCFLQQSEPLAATGTGDFNRQFLGQMTQLNQLLGEVKDLLRQQVKETSFLRNTIAECQACGPLKFQSPTPSTVVPPAPPAPPTRPPRRCDSNPCFRGVQCTDSRDGFQCGPCPEGYTGNGITCIDVDECKYHPCYPGVHCINLSPGFRCDACPVGFTGPMVQGVGISFAKSNKQVCTDIDECRNGACVPNSICVNTLGSYRCGPCKPGYTGDQIRGCKAERNCRNPELNPCSVNAQCIEERQGDVTCVCGVGWAGDGYICGKDVDIDSYPDEELPCSARNCKKDNCKYVPNSGQEDADRDGIGDACDEDADGDGILNEQDNCVLIHNVDQRNSDKDIFGDACDNCLSVLNNDQKDTDGDGRGDACDDDMDGDGIKNILDNCPKFPNRDQRDKDGDGVGDACDSCPDVSNPNQSDVDNDLVGDSCDTNQDSDGDGHQDSTDNCPTVINSAQLDTDKDGIGDECDDDDDNDGIPDLVPPGPDNCRLVPNPAQEDSNSDGVGDICESDFDQDQVIDRIDVCPENAEVTLTDFRAYQTVVLDPEGDAQIDPNWVVLNQGMEIVQTMNSDPGLAVGYTAFNGVDFEGTFHVNTQTDDDYAGFIFGYQDSSSFYVVMWKQTEQTYWQATPFRAVAEPGIQLKAVKSKTGPGEHLRNSLWHTGDTSDQVRLLWKDSRNVGWKDKVSYRWFLQHRPQVGYIRVRFYEGSELVADSGVTIDTTMRGGRLGVFCFSQENIIWSNLKYRCNDTIPEDFQEFQTQNFDRFDN

SEQ ID NO: 8 - RNA, 3281 nt, Homo sapiens
  source 1..3281: mol_type = mRNA
tcccccgcccggccgcaccataaagcgcccggccgctgccgcggagcccagcagccagctccccagcaccgcacggcggggacgcgagcgcgcccccgacggcagcccggacgccgagcacgggtcacctgcggcgccggcccgggcgccgaccgaggttcaacgcacggcccggggacccccaggcggggccaacgccgccgtcgcccccggcctcgcggggagcaggaagagccaacatgctggccccgcgcggagccgccgtcctcctgctgcacctggtcctgcagcggtggctagcggcaggcgcccaggccaccccccaggtctttgaccttctcccatcttccagtcagaggctaaacccaggcgctctgctgccagtcctgacagaccccgccctgaatgatctctatgtgatttccaccttcaagctgcagactaaaagttcagccaccatcttcggtctttactcttcaactgacaacagtaaatattttgaatttactgtgatgggacgcttaaacaaagccatcctccgttacctgaagaacgatgggaaggtgcatttggtggttttcaacaacctgcagctggcagacggaaggcggcacaggatcctcctgaggctgagcaatttgcagcgaggggccggctccctagagctctacctggactgcatccaggtggattccgttcacaatctccccagggcctttgctggcccctcccagaaacctgagaccattgaattgaggactttccagaggaagccacaggacttcttggaagagctgaagctggtggtgagaggctcactgttccaggtggccagcctgcaagactgcttcctgcagcagagtgagccactggctgccacaggcacaggggactttaaccggcagttcttgggtcaaatgacacaattaaaccaactcctgggagaggtgaaggaccttctgagacagcaggttaaggaaacatcatttttgcgaaacaccatagctgaatgccaggcttgcggtcctctcaagtttcagtctccgaccccaagcacggtggtgcccccggctccccctgcaccgccaacacgcccacctcgtcggtgtgactccaacccatgtttccgaggtgtccaatgtaccgacagtagagatggcttccagtgtgggccctgccccgagggctacacaggaaacgggatcacctgtattgatgttgatgagtgcaaataccatccctgctacccgggcgtgcactgcataaatttgtctcctggcttcagatgtgacgcctgcccagtgggcttcacagggcccatggtgcagggtgttgggatcagttttgccaagtcaaacaagcaggtctgcactgacattgatgagtgtcgaaatggagcgtgcgttcccaactcgatctgcgttaatactttgggatcttaccgctgtgggccttgtaagccggggtatactggtgatcagataaggggatgcaaagcggaaagaaactgcagaaacccagagctgaacccttgcagtgtgaatgcccagtgcattgaagagaggcagggggatgtgacatgtgtgtgtggagtcggttgggctggagatggctatatctgtggaaaggatgtggacatcgacagttaccccgacgaagaactgccatgctctgccaggaactgtaaaaaggacaactgcaaatatgtgccaaattctggccaagaagatgcagacagagatggcattggcgacgcttgtgacgaggatgctgacggagatgggatcctgaatgagcaggataactgtgtcctgattcataatgtggaccaaaggaacagcgataaagatatctttggggatgcctgtgataactgcctgagtgtcttaaataacgaccagaaagacaccgatggggatggaagaggagatgcctgtgatgatgacatggatggagatggaataaaaaacattctggacaactgcccaaaatttcccaatcgtgaccaacgggacaaggatggtgatggtgtgggggatgcctgtgacagttgtcctgatgtcagcaaccctaaccagtctgatgtggataatgatctggttggggactcctgtgacaccaatcaggacagtgatggagatgggcaccaggacagcacagacaactgccccaccgtcattaacagtgcccagctggacaccgataaggatggaattggtgacgagtgtgatgatgatgatgacaatgatggtatcccagacctggtgccccctggaccagacaactgccggctggtccccaacccagcccaggaggatagcaacagcgacggagtgggagacatctgtgagtctgactttgaccaggaccaggtcatcgatcggatcgacgtctgcccagagaacgcagaggtcaccctgaccgacttcagggcttaccagaccgtggtcctggatcctgaaggggatgcccagatcgatcccaactgggtggtcctgaaccagggcatggagattgtacagaccatgaacagtgatcctggcctggcagtggggtacacagcttttaatggagttgacttcgaagggaccttccatgtgaatacccagacagatgatgactatgcaggctttatctttggctaccaagatagctccagcttctacgtggtcatgtggaagcagacggagcagacatattggcaagccaccccattccgagcagttgcagaacctggcattcagctcaaggctgtgaagtctaagacaggtccaggggagcatctccggaactccctgtggcacacgggggacaccagtgaccaggtcaggctgctgtggaaggactccaggaatgtgggctggaaggacaaggtgtcctaccgctggttcctacagcacaggccccaggtgggctacatcagggtacgattttatgaaggctctgagttggtggctgactctggcgtcaccatagacaccacaatgcgtggaggccgacttggcgttttctgcttctctcaagaaaacatcatctggtccaacctcaagtatcgctgcaatgacaccatccctgaggacttccaagagtttcaaacccagaatttcgaccgcttcgataattaaaccaaggaagcaatctgtaactgcttttcggaacactaaaaccatatatattttaacttcaattttctttagcttttaccaacccaaatatatcaaaacgttttatgtgaatgtggcaataaaggagaagagatcatttttaaaaaaaaaaaaaaa

SEQ ID NO: 9 - RNA, 3115 nt, Homo sapiens
  source 1..3115: mol_type = mRNA
gtgaaacgcgggggcgtggctaagggagggaagggtaatttgggggctcttgagagatgagagaaacaacgactggagggattaagaagaactcttaggagcagcttggcctaaaggctgtgtgggacgtgcctgctttgccttcgccttccaccatgatctctttgaccttctcccatcttccagtcagaggctaaacccaggcgctctgctgccagtcctgacagaccccgccctgaatgatctctatgtgatttccaccttcaagctgcagactaaaagttcagccaccatcttcggtctttactcttcaactgacaacagtaaatattttgaatttactgtgatgggacgcttaaacaaagccatcctccgttacctgaagaacgatgggaaggtgcatttggtggttttcaacaacctgcagctggcagacggaaggcggcacaggatcctcctgaggctgagcaatttgcagcgaggggccggctccctagagctctacctggactgcatccaggtggattccgttcacaatctccccagggcctttgctggcccctcccagaaacctgagaccattgaattgaggactttccagaggaagccacaggacttcttggaagagctgaagctggtggtgagaggctcactgttccaggtggccagcctgcaagactgcttcctgcagcagagtgagccactggctgccacaggcacaggggactttaaccggcagttcttgggtcaaatgacacaattaaaccaactcctgggagaggtgaaggaccttctgagacagcaggttaaggaaacatcatttttgcgaaacaccatagctgaatgccaggcttgcggtcctctcaagtttcagtctccgaccccaagcacggtggtgcccccggctccccctgcaccgccaacacgcccacctcgtcggtgtgactccaacccatgtttccgaggtgtccaatgtaccgacagtagagatggcttccagtgtgggccctgccccgagggctacacaggaaacgggatcacctgtattgatgttgatgagtgcaaataccatccctgctacccgggcgtgcactgcataaatttgtctcctggcttcagatgtgacgcctgcccagtgggcttcacagggcccatggtgcagggtgttgggatcagttttgccaagtcaaacaagcaggtctgcactgacattgatgagtgtcgaaatggagcgtgcgttcccaactcgatctgcgttaatactttgggatcttaccgctgtgggccttgtaagccggggtatactggtgatcagataaggggatgcaaagcggaaagaaactgcagaaacccagagctgaacccttgcagtgtgaatgcccagtgcattgaagagaggcagggggatgtgacatgtgtgtgtggagtcggttgggctggagatggctatatctgtggaaaggatgtggacatcgacagttaccccgacgaagaactgccatgctctgccaggaactgtaaaaaggacaactgcaaatatgtgccaaattctggccaagaagatgcagacagagatggcattggcgacgcttgtgacgaggatgctgacggagatgggatcctgaatgagcaggataactgtgtcctgattcataatgtggaccaaaggaacagcgataaagatatctttggggatgcctgtgataactgcctgagtgtcttaaataacgaccagaaagacaccgatggggatggaagaggagatgcctgtgatgatgacatggatggagatggaataaaaaacattctggacaactgcccaaaatttcccaatcgtgaccaacgggacaaggatggtgatggtgtgggggatgcctgtgacagttgtcctgatgtcagcaaccctaaccagtctgatgtggataatgatctggttggggactcctgtgacaccaatcaggacagtgatggagatgggcaccaggacagcacagacaactgccccaccgtcattaacagtgcccagctggacaccgataaggatggaattggtgacgagtgtgatgatgatgatgacaatgatggtatcccagacctggtgccccctggaccagacaactgccggctggtccccaacccagcccaggaggatagcaacagcgacggagtgggagacatctgtgagtctgactttgaccaggaccaggtcatcgatcggatcgacgtctgcccagagaacgcagaggtcaccctgaccgacttcagggcttaccagaccgtggtcctggatcctgaaggggatgcccagatcgatcccaactgggtggtcctgaaccagggcatggagattgtacagaccatgaacagtgatcctggcctggcagtggggtacacagcttttaatggagttgacttcgaagggaccttccatgtgaatacccagacagatgatgactatgcaggctttatctttggctaccaagatagctccagcttctacgtggtcatgtggaagcagacggagcagacatattggcaagccaccccattccgagcagttgcagaacctggcattcagctcaaggctgtgaagtctaagacaggtccaggggagcatctccggaactccctgtggcacacgggggacaccagtgaccaggtcaggctgctgtggaaggactccaggaatgtgggctggaaggacaaggtgtcctaccgctggttcctacagcacaggccccaggtgggctacatcagggtacgattttatgaaggctctgagttggtggctgactctggcgtcaccatagacaccacaatgcgtggaggccgacttggcgttttctgcttctctcaagaaaacatcatctggtccaacctcaagtatcgctgcaatgacaccatccctgaggacttccaagagtttcaaacccagaatttcgaccgcttcgataattaaaccaaggaagcaatctgtaactgcttttcggaacactaaaaccatatatattttaacttcaattttctttagcttttaccaacccaaatatatcaaaacgttttatgtgaatgtggcaataaaggagaagagatcatttttaaaaaaaaaaaaaaa

SEQ ID NO: 10 - RNA, 3166 nt, Homo sapiens
  source 1..3166: mol_type = mRNA
tgaaacgcgggggcgtggctaagggagggaagggtaatttgggggctcttgagagatgagagaaacaacgactggagggattaagaagaactcttaggagcagcttggcctaaaggctgtgtgggacgtgcctgctttgccttcgccttccaccatgatcgtaagttttctgagaccccctcagccatgtttcctgtagagcctgtggagtttctttgaccttctcccatcttccagtcagaggctaaacccaggcgctctgctgccagtcctgacagaccccgccctgaatgatctctatgtgatttccaccttcaagctgcagactaaaagttcagccaccatcttcggtctttactcttcaactgacaacagtaaatattttgaatttactgtgatgggacgcttaaacaaagccatcctccgttacctgaagaacgatgggaaggtgcatttggtggttttcaacaacctgcagctggcagacggaaggcggcacaggatcctcctgaggctgagcaatttgcagcgaggggccggctccctagagctctacctggactgcatccaggtggattccgttcacaatctccccagggcctttgctggcccctcccagaaacctgagaccattgaattgaggactttccagaggaagccacaggacttcttggaagagctgaagctggtggtgagaggctcactgttccaggtggccagcctgcaagactgcttcctgcagcagagtgagccactggctgccacaggcacaggggactttaaccggcagttcttgggtcaaatgacacaattaaaccaactcctgggagaggtgaaggaccttctgagacagcaggttaaggaaacatcatttttgcgaaacaccatagctgaatgccaggcttgcggtcctctcaagtttcagtctccgaccccaagcacggtggtgcccccggctccccctgcaccgccaacacgcccacctcgtcggtgtgactccaacccatgtttccgaggtgtccaatgtaccgacagtagagatggcttccagtgtgggccctgccccgagggctacacaggaaacgggatcacctgtattgatgttgatgagtgcaaataccatccctgctacccgggcgtgcactgcataaatttgtctcctggcttcagatgtgacgcctgcccagtgggcttcacagggcccatggtgcagggtgttgggatcagttttgccaagtcaaacaagcaggtctgcactgacattgatgagtgtcgaaatggagcgtgcgttcccaactcgatctgcgttaatactttgggatcttaccgctgtgggccttgtaagccggggtatactggtgatcagataaggggatgcaaagcggaaagaaactgcagaaacccagagctgaacccttgcagtgtgaatgcccagtgcattgaagagaggcagggggatgtgacatgtgtgtgtggagtcggttgggctggagatggctatatctgtggaaaggatgtggacatcgacagttaccccgacgaagaactgccatgctctgccaggaactgtaaaaaggacaactgcaaatatgtgccaaattctggccaagaagatgcagacagagatggcattggcgacgcttgtgacgaggatgctgacggagatgggatcctgaatgagcaggataactgtgtcctgattcataatgtggaccaaaggaacagcgataaagatatctttggggatgcctgtgataactgcctgagtgtcttaaataacgaccagaaagacaccgatggggatggaagaggagatgcctgtgatgatgacatggatggagatggaataaaaaacattctggacaactgcccaaaatttcccaatcgtgaccaacgggacaaggatggtgatggtgtgggggatgcctgtgacagttgtcctgatgtcagcaaccctaaccagtctgatgtggataatgatctggttggggactcctgtgacaccaatcaggacagtgatggagatgggcaccaggacagcacagacaactgccccaccgtcattaacagtgcccagctggacaccgataaggatggaattggtgacgagtgtgatgatgatgatgacaatgatggtatcccagacctggtgccccctggaccagacaactgccggctggtccccaacccagcccaggaggatagcaacagcgacggagtgggagacatctgtgagtctgactttgaccaggaccaggtcatcgatcggatcgacgtctgcccagagaacgcagaggtcaccctgaccgacttcagggcttaccagaccgtggtcctggatcctgaaggggatgcccagatcgatcccaactgggtggtcctgaaccagggcatggagattgtacagaccatgaacagtgatcctggcctggcagtggggtacacagcttttaatggagttgacttcgaagggaccttccatgtgaatacccagacagatgatgactatgcaggctttatctttggctaccaagatagctccagcttctacgtggtcatgtggaagcagacggagcagacatattggcaagccaccccattccgagcagttgcagaacctggcattcagctcaaggctgtgaagtctaagacaggtccaggggagcatctccggaactccctgtggcacacgggggacaccagtgaccaggtcaggctgctgtggaaggactccaggaatgtgggctggaaggacaaggtgtcctaccgctggttcctacagcacaggccccaggtgggctacatcagggtacgattttatgaaggctctgagttggtggctgactctggcgtcaccatagacaccacaatgcgtggaggccgacttggcgttttctgcttctctcaagaaaacatcatctggtccaacctcaagtatcgctgcaatgacaccatccctgaggacttccaagagtttcaaacccagaatttcgaccgcttcgataattaaaccaaggaagcaatctgtaactgcttttcggaacactaaaaccatatatattttaacttcaattttctttagcttttaccaacccaaatatatcaaaacgttttatgtgaatgtggcaataaaggagaagagatcatttttaaaaaaaaaaaaaaa

SEQ ID NO: 11 - RNA, 3109 nt, Homo sapiens
  source 1..3109: mol_type = mRNA
ggagcgatgtatgcccagagtctgctcttgacatccctgagaaagacgcagaattactctacttgccctgccacctgcattttctgctctgactttgcttgaacgacaaaaagaaagtttatttcaaggattggcttgatgtcttaatttctgagtctttgaccttctcccatcttccagtcagaggctaaacccaggcgctctgctgccagtcctgacagaccccgccctgaatgatctctatgtgatttccaccttcaagctgcagactaaaagttcagccaccatcttcggtctttactcttcaactgacaacagtaaatattttgaatttactgtgatgggacgcttaaacaaagccatcctccgttacctgaagaacgatgggaaggtgcatttggtggttttcaacaacctgcagctggcagacggaaggcggcacaggatcctcctgaggctgagcaatttgcagcgaggggccggctccctagagctctacctggactgcatccaggtggattccgttcacaatctccccagggcctttgctggcccctcccagaaacctgagaccattgaattgaggactttccagaggaagccacaggacttcttggaagagctgaagctggtggtgagaggctcactgttccaggtggccagcctgcaagactgcttcctgcagcagagtgagccactggctgccacaggcacaggggactttaaccggcagttcttgggtcaaatgacacaattaaaccaactcctgggagaggtgaaggaccttctgagacagcaggttaaggaaacatcatttttgcgaaacaccatagctgaatgccaggcttgcggtcctctcaagtttcagtctccgaccccaagcacggtggtgcccccggctccccctgcaccgccaacacgcccacctcgtcggtgtgactccaacccatgtttccgaggtgtccaatgtaccgacagtagagatggcttccagtgtgggccctgccccgagggctacacaggaaacgggatcacctgtattgatgttgatgagtgcaaataccatccctgctacccgggcgtgcactgcataaatttgtctcctggcttcagatgtgacgcctgcccagtgggcttcacagggcccatggtgcagggtgttgggatcagttttgccaagtcaaacaagcaggtctgcactgacattgatgagtgtcgaaatggagcgtgcgttcccaactcgatctgcgttaatactttgggatcttaccgctgtgggccttgtaagccggggtatactggtgatcagataaggggatgcaaagcggaaagaaactgcagaaacccagagctgaacccttgcagtgtgaatgcccagtgcattgaagagaggcagggggatgtgacatgtgtgtgtggagtcggttgggctggagatggctatatctgtggaaaggatgtggacatcgacagttaccccgacgaagaactgccatgctctgccaggaactgtaaaaaggacaactgcaaatatgtgccaaattctggccaagaagatgcagacagagatggcattggcgacgcttgtgacgaggatgctgacggagatgggatcctgaatgagcaggataactgtgtcctgattcataatgtggaccaaaggaacagcgataaagatatctttggggatgcctgtgataactgcctgagtgtcttaaataacgaccagaaagacaccgatggggatggaagaggagatgcctgtgatgatgacatggatggagatggaataaaaaacattctggacaactgcccaaaatttcccaatcgtgaccaacgggacaaggatggtgatggtgtgggggatgcctgtgacagttgtcctgatgtcagcaaccctaaccagtctgatgtggataatgatctggttggggactcctgtgacaccaatcaggacagtgatggagatgggcaccaggacagcacagacaactgccccaccgtcattaacagtgcccagctggacaccgataaggatggaattggtgacgagtgtgatgatgatgatgacaatgatggtatcccagacctggtgccccctggaccagacaactgccggctggtccccaacccagcccaggaggatagcaacagcgacggagtgggagacatctgtgagtctgactttgaccaggaccaggtcatcgatcggatcgacgtctgcccagagaacgcagaggtcaccctgaccgacttcagggcttaccagaccgtggtcctggatcctgaaggggatgcccagatcgatcccaactgggtggtcctgaaccagggcatggagattgtacagaccatgaacagtgatcctggcctggcagtggggtacacagcttttaatggagttgacttcgaagggaccttccatgtgaatacccagacagatgatgactatgcaggctttatctttggctaccaagatagctccagcttctacgtggtcatgtggaagcagacggagcagacatattggcaagccaccccattccgagcagttgcagaacctggcattcagctcaaggctgtgaagtctaagacaggtccaggggagcatctccggaactccctgtggcacacgggggacaccagtgaccaggtcaggctgctgtggaaggactccaggaatgtgggctggaaggacaaggtgtcctaccgctggttcctacagcacaggccccaggtgggctacatcagggtacgattttatgaaggctctgagttggtggctgactctggcgtcaccatagacaccacaatgcgtggaggccgacttggcgttttctgcttctctcaagaaaacatcatctggtccaacctcaagtatcgctgcaatgacaccatccctgaggacttccaagagtttcaaacccagaatttcgaccgcttcgataattaaaccaaggaagcaatctgtaactgcttttcggaacactaaaaccatatatattttaacttcaattttctttagcttttaccaacccaaatatatcaaaacgttttatgtgaatgtggcaataaaggagaagagatcatttttaaaaaaaaaaaaaaa

SEQ ID NO: 12 - protein, 1257 aa, Homo sapiens
MENSERAEEMQENYQRNGTAEEQPKLRKEAVGSIEIFRFADGLDITLMILGILASLVNGACLPLMPLVLGEMSDNLISGCLVQTNTTNYQNCTQSQEKLNEDMTLLTLYYVGIGVAALIFGYIQISLWIITAARQTKRIRKQFFHSVLAQDIGWFDSCDIGELNTRMTDDIDKISDGIGDKIALLFQNMSTFSIGLAVGLVKGWKLTLVTLSTSPLIMASAAACSRMVISLTSKELSAYSKAGAVAEEVLSSIRTVIAFRAQEKELQRYTQNLKDAKDFGIKRTIASKVSLGAVYFFMNGTYGLAFWYGTSLILNGEPGYTIGTVLAVFFSVIHSSYCIGAAVPHFETFAIARGAAFHIFQVIDKKPSIDNFSTAGYKPESIEGTVEFKNVSFNYPSRPSIKILKGLNLRIKSGETVALVGLNGSGKSTVVQLLQRLYDPDDGFIMVDENDIRALNVRHYRDHIGVVSQEPVLFGTTISNNIKYGRDDVTDEEMERAAREANAYDFIMEFPNKFNTLVGEKGAQMSGGQKQRIAIARALVRNPKILILDEATSALDSESKSAVQAALEKASKGRTTIVVAHRLSTIRSADLIVTLKDGMLAEKGAHAELMAKRGLYYSLVMSQDIKKADEQMESMTYSTERKTNSLPLHSVKSIKSDFIDKAEESTQSKEISLPEVSLLKILKLNKPEWPFVVLGTLASVLNGTVHPVFSIIFAKIITMFGNNDKTTLKHDAEIYSMIFVILGVICFVSYFMQGLFYGRAGEILTMRLRHLAFKAMLYQDIAWFDEKENSTGGLTTILAIDIAQIQGATGSRIGVLTQNATNMGLSVIISFIYGWEMTFLILSIAPVLAVTGMIETAAMTGFANKDKQELKHAGKIATEALENIRTIVSLTREKAFEQMYEEMLQTQHRNTSKKAQIIGSCYAFSHAFIYFAYAAGFRFGAYLIQAGRMTPEGMFIVFTAIAYGAMAIGETLVLAPEYSKAKSGAAHLFALLEKKPNIDSRSQEGKKPDTCEGNLEFREVSFFYPCRPDVFILRGLSLSIERGKTVAFVGSSGCGKSTSVQLLQRLYDPVQGQVLFDGVDAKELNVQWLRSQIAIVPQEPVLFNCSIAENIAYGDNSRVVPLDEIKEAANAANIHSFIEGLPEKYNTQVGLKGAQLSGGQKQRLAIARALLQKPKILLLDEATSALDNDSEKVVQHALDKARTGRTCLVVTHRLSAIQNADLIVVLHNGKIKEQGTHQELLRNRDIYFKLVNAQSVQ

SEQ ID NO: 13 - protein, 131 aa, Homo sapiens
MVDENDIRALNVRHYRDHIGVVSQEPVLFGTTISNNIKYGRDDVTDEEMERAAREANAYDFIMEFPNKFNTLVGEKGAQMSGGQKQRIAIARALVRNPKILILDEATSALDSESKSAVQAALEKDTPRYSF

SEQ ID NO: 14 - protein, 126 aa, Homo sapiens
MVDENDIRALNVRHYRDHIGVVSQEPVLFGTTISNNIKYGRDDVTDEEMERAAREANAYDFIMEFPNKFNTLVGEKGAQMSGGQKQRIAIARALVRNPKILILDEATSALDSESKSAVQAALEKKK

SEQ ID NO: 15 - protein, 812 aa, Homo sapiens
MVDENDIRALNVRHYRDHIGVVSQEPVLFGTTISNNIKYGRDDVTDEEMERAAREANAYDFIMEFPNKFNTLVGEKGAQMSGGQKQRIAIARALVRNPKILILDEATSALDSESKSAVQAALEKASKGRTTIVVAHRLSTIRSADLIVTLKDGMLAEKGAHAELMAKRGLYYSLVMSQDIKKADEQMESMTYSTERKTNSLPLHSVKSIKSDFIDKAEESTQSKEISLPEVSLLKILKLNKPEWPFVVLGTLASVLNGTVHPVFSIIFAKIITMFGNNDKTTLKHDAEIYSMIFVILGVICFVSYFMQGLFYGRAGEILTMRLRHLAFKAMLYQDIAWFDEKENSTGGLTTILAIDIAQIQGATGSRIGVLTQNATNMGLSVIISFIYGWEMTFLILSIAPVLAVTGMIETAAMTGFANKDKQELKHAGKIATEALENIRTIVSLTREKAFEQMYEEMLQTQHRNTSKKAQIIGSCYAFSHAFIYFAYAAGFRFGAYLIQAGRMTPEGMFIVFTAIAYGAMAIGETLVLAPEYSKAKSGAAHLFALLEKKPNIDSRSQEGKKPDTCEGNLEFREVSFFYPCRPDVFILRGLSLSIERGKTVAFVGSSGCGKSTSVQLLQRLYDPVQGQVLFDGVDAKELNVQWLRSQIAIVPQEPVLFNCSIAENIAYGDNSRVVPLDEIKEAANAANIHSFIEGLPEKYNTQVGLKGAQLSGGQKQRLAIARALLQKPKILLLDEATSALDNDSEKVVQHALDKARTGRTCLVVTHRLSAIQNADLIVVLHNGKIKEQGTHQELLRNRDIYFKLVNAQSVQ

SEQ ID NO: 16 - RNA, 2247 nt, Homo sapiens
  source 1..2247: mol_type = mRNA
attgcttctcggccttttggctaagatcaagtgtaatctgtgttcttttttatttggtcatatcttccattctttcttacctaattcctctaatatctctctgtgagcctaaaccaataattatatattacattctattgtctttcttatataactgcagaaagataaatatcactttgtttgttcctgtaggttttctttagtgtaatccatagcagttattgcattggagcagcagtccctcactttgaaaccttcgcaatagcccgaggagctgcctttcatattttccaggttattgataagaaacccagtatagataacttttccacagctggatataaacctgaatccatagaaggaactgtggaatttaaaaatgtttctttcaattatccatcaagaccatctatcaagattctgaaaggtctgaatctcagaattaagtctggagagacagtcgccttggtcggtctcaatggcagtgggaagagtacggtagtccagcttctgcagaggttatatgatccggatgatggctttatcatggtggatgagaatgacatcagagctttaaatgtgcggcattatcgagaccatattggagtggttagtcaagagcctgttttgttcgggaccaccatcagtaacaatatcaagtatggacgagatgatgtgactgatgaagagatggagagagcagcaagggaagcaaatgcgtatgattttatcatggagtttcctaataaatttaatacattggtaggggaaaaaggagctcaaatgagtggagggcagaaacagaggatcgcaattgctcgtgccttagttcgaaaccccaagattctgattttagatgaggctacgtctgccctggattcagaaagcaagtcagctgttcaagctgcactggagaaggatacccccaggtattcattttgacctaatttcacctcaagtggagaatcgctgaccttgaaccagcgcccttcgacagctctggcccctcaaacctcaccctgacctcctgctgcctatgagctactgcacatacctcaaggccatatgcagttgtggccctgcaccaaattacactgaatctaggaggggagttggcagtggcggtatgaaaaaccattgaacagttttctcgatggcctgactcccttataaaccagagccttcagaccccttacaaggcttaatggcacattttactttgcatttgcttggaagtgagttaagcgtttttttttctctaagaaaatcgcaggcttctttttttaaaatgctgactttatggaaccagaaacggatactggcaggctaaatgtccactgcttcttgaaaaatctcttagttactattatttagtagcaaatcagattgtgcaagtttgaacgcttgtttccctcccataataacaatgccacatgttgcttgtgtgataaataatctttgtttactgtggacacttcggcaatttggttcatcttggtacagaaaatacaaagacaggactaatattttattcattttttatacttagtaactaggacagggatctgtatttagactatattcaagcctcgctctgtcacccatgcttgagtgcaacctctgcccactgtgttcaagcgattctcctgcctcagcctcctgagtagctgggagtacaggcgtgcatcaccacacccagctaatttttgtatttttagtagagacaaggttttgccatgttgaccaggctggtctcaaactcctgacctcaggtgatccgcccacctcggcctcccaaagtgctgggattacaggtgtgcgtctccgcgcccggccagttacataagattttaaaaaatgtattgtaataggctctctgattgtttagaaggtttcatgttgtgcccgcagtattttcatccactggtaatcactttaggtaatcaaaactagttcagacttttaaaataaatagttgcttggtgacatgataaactaataaatgttattcttattggttaatatgaaacatctatcaaaagtgaaaaaagaagaatgcagaatgtttgtaaactgattccaaaattacacaaaatagcaactgtgaaaaaaatgaaggcaatatatgaaaataataacagctatgtggcataattatgggggaatttaacttatttcaaaaattcatttactgtccctgtttttcagttgtttaaaggagaaagagattaaatcaatgtagaaata

SEQ ID NO: 17 - RNA, 5401 nt, Homo sapiens
  source 1..5401: mol_type = mRNA
tgtagagagagaaagagaaaacacgctcatgtaattgtggtgactggcacttccaaaatccacaagccagactagaaggctggaaattctggcaaaaaattgataccttgtatctgaaagctttatcctatcctcttcagaagacttcagtcttttctcttaaggacttcaactgactggatggggcccactcaaaacagcatctaaggaattaaaaagaagtaaattgtaaataagatggaaaattcagaaagagctgaagaaatgcaagaaaattatcagagaaatggaactgcagaagaacagccaaaactgagaaaggaagcagttggatctattgagatattccgctttgctgatggactggacatcacactcatgatcctgggtatactggcatcactggtcaatggagcctgccttcctttaatgccactggttttaggagaaatgagtgataaccttattagtggatgtctagtccaaactaacacaacaaattatcagaactgtactcagtctcaagagaagctgaatgaagatatgactctgttgaccctgtattatgttggaataggtgttgctgccttgatttttggttacatacagatttccttgtggattataactgcagcacgacagaccaagaggattcgaaaacagttttttcattcagttttggcacaggacatcggctggtttgatagctgtgacatcggtgaacttaacactcgcatgacagatgacattgacaaaatcagtgatggtattggagataagattgctctgttgtttcaaaacatgtctactttttcgattggcctggcagttggtttggtgaagggctggaaactcaccctagtgactctatccacgtctcctcttataatggcttcagcggcagcatgttctaggatggtcatctcattgaccagtaaggaattaagtgcctattccaaagctggggctgtggcagaagaagtcttgtcatcaatccgaacagtcatagcctttagggcccaggagaaagaacttcaaaggtatacacagaatctcaaagatgcaaaggattttggcataaaaaggactatagcttcaaaagtgtctcttggtgctgtgtacttctttatgaatggaacctatggacttgctttttggtatggaacctccttgattcttaatggagaacctggatataccatcgggactgttcttgctgttttctttagtgtaatccatagcagttattgcattggagcagcagtccctcactttgaaaccttcgcaatagcccgaggagctgcctttcatattttccaggttattgataagaaacccagtatagataacttttccacagctggatataaacctgaatccatagaaggaactgtggaatttaaaaatgtttctttcaattatccatcaagaccatctatcaagattctgaaaggtctgaatctcagaattaagtctggagagacagtcgccttggtcggtctcaatggcagtgggaagagtacggtagtccagcttctgcagaggttatatgatccggatgatggctttatcatggtggatgagaatgacatcagagctttaaatgtgcggcattatcgagaccatattggagtggttagtcaagagcctgttttgttcgggaccaccatcagtaacaatatcaagtatggacgagatgatgtgactgatgaagagatggagagagcagcaagggaagcaaatgcgtatgattttatcatggagtttcctaataaatttaatacattggtaggggaaaaaggagctcaaatgagtggagggcagaaacagaggatcgcaattgctcgtgccttagttcgaaaccccaagattctgattttagatgaggctacgtctgccctggattcagaaagcaagtcagctgttcaagctgcactggagaaggcgagcaaaggtcggactacaatcgtggtagcacaccgactttctactattcgaagtgcagatttgattgtgaccctaaaggatggaatgctggcggagaaaggagcacatgctgaactaatggcaaaacgaggtctatattattcacttgtgatgtcacaggatattaaaaaagctgatgaacagatggagtcaatgacatattctactgaaagaaagaccaactcacttcctctgcactctgtgaagagcatcaagtcagacttcattgacaaggctgaggaatccacccaatctaaagagataagtcttcctgaagtctctctattaaaaattttaaagttaaacaagcctgaatggccttttgtggttctggggacattggcttctgttctaaatggaactgttcatccagtattttccatcatctttgcaaaaattataaccatgtttggaaataatgataaaaccacattaaagcatgatgcagaaatttattccatgatattcgtcattttgggtgttatttgctttgtcagttatttcatgcagggattattttacggcagagcaggggaaattttaacgatgagattaagacacttggccttcaaagccatgttatatcaggatattgcctggtttgatgaaaaggaaaacagcacaggaggcttgacaacaatattagccatagatatagcacaaattcaaggagcaacaggttccaggattggcgtcttaacacaaaatgcaactaacatgggactttcagttatcatttcctttatatatggatgggagatgacattcctgattctgagtattgctccagtacttgccgtgacaggaatgattgaaaccgcagcaatgactggatttgccaacaaagataagcaagaacttaagcatgctggaaagatagcaactgaagctttggagaatatacgtactatagtgtcattaacaagggaaaaagccttcgagcaaatgtatgaagagatgcttcagactcaacacagaaatacctcgaagaaagcacagattattggaagctgttatgcattcagccatgcctttatatattttgcctatgcggcagggtttcgatttggagcctatttaattcaagctggacgaatgaccccagagggcatgttcatagtttttactgcaattgcatatggagctatggccatcggagaaacgctcgttttggctcctgaatattccaaagccaaatcgggggctgcgcatctgtttgccttgttggaaaagaaaccaaatatagacagccgcagtcaagaagggaaaaagccagacacatgtgaagggaatttagagtttcgagaagtctctttcttctatccatgtcgcccagatgttttcatcctccgtggcttatccctcagtattgagcgaggaaagacagtagcatttgtggggagcagcggctgtgggaaaagcacttctgttcaacttctgcagagactttatgaccccgtgcaaggacaagtgctgtttgatggtgtggatgcaaaagaattgaatgtacagtggctccgttcccaaatagcaatcgttcctcaagagcctgtgctcttcaactgcagcattgctgagaacatcgcctatggtgacaacagccgtgtggtgccattagatgagatcaaagaagccgcaaatgcagcaaatatccattcttttattgaaggtctccctgagaaatacaacacacaagttggactgaaaggagcacagctttctggcggccagaaacaaagactagctattgcaagggctcttctccaaaaacccaaaattttattgttggatgaggccacttcagccctcgataatgacagtgagaaggtggttcagcatgcccttgataaagccaggacgggaaggacatgcctagtggtcactcacaggctctctgcaattcagaacgcagatttgatagtggttctgcacaatggaaagataaaggaacaaggaactcatcaagagctcctgagaaatcgagacatatattttaagttagtgaatgcacagtcagtgcagtgatgctgttgaggtagcacatattttgatgttcgtgtaatgcaaagaaggagtacttaataattacttggcaagctttgatctcttttattgcatatatcaatacctagaatcatgctactcaagtacatacatgttctattcacacaccatctgaccttcagatttttaaaaggaagcaaaaatttgcttatttcatgtaagtgaaataatgcttatatccttcactttataaaactattctagcacatttgcttgtaaagcagttttctacaaggtgaatttatttcccatcaacttctgctataaaatcggaaatatgtttccagggggaatattatccaattaaccatgttgaaggttttagcaaaggcagtgtaagatagagtggggcctgtagcattgcagggagagtgtctttcacttggaattttgttttgcagcacatattacagtagttttgctagtcccttttctccagaccgtagggatttctctcaataagtattcactatttctctaaattttattctatttttttgttgagcagggaatagaaaggattacgatgtaaaatttctgggaggattaggtagctatctcctacttcaccagtaagtgaagtgcctcacatgagccatcccaaagattcattattccaaaccttgggtttggcagtataagtcacaggcctacctgtttatgaaaacttacttacttaaaataagagctacttttgggccgggtgcggtggctcacgcctgtaatcccagaactttgggaggccgaggagggcggatcacttgaggtcaggagttcgagaccagcctggccaacatggtgaaaccccgtctctactaaaaacacaaaaattagccaatcttggtggcgggcacctggaatcccagctacttgggaggctgaggcaggagaatcatttgaacctaggaggcagaggttgcagtgagccgagatctcaccactgcactccagcctgcgcaacagagcgagactccatctcaaaaaataataaataagagctaattttattgtgggtgaaaatttttaaacgtctttctctataataaaataatttccttaaattttatatatactttatcatatataatgtgtgaatgattttaaagttctgtgtaaataacaatattggtaaaatgagttacattttcaacttacttaaatatgtaatgtcacctggtgattttatctttattcttcagtgtattttcttccatttacacatttagctagcctccctaaagtgtactctaccaataattgaaatcttgttaaacaaaattaaaaccatttatatattatgctgctttctttaaaatgcaaaataaaaataagattggggacttgagaatca

SEQ ID NO: 18 - RNA, 4375 nt, Homo sapiens
  source 1..4375: mol_type = mRNA
attgcttctcggccttttggctaagatcaagtgtaatctgtgttcttttttatttggtcatatcttccattctttcttacctaattcctctaatatctctctgtgagcctaaaccaataattatatattacattctattgtctttcttatataactgcagaaagataaatatcactttgtttgttcctgtaggttttctttagtgtaatccatagcagttattgcattggagcagcagtccctcactttgaaaccttcgcaatagcccgaggagctgcctttcatattttccaggttattgataagaaacccagtatagataacttttccacagctggatataaacctgaatccatagaaggaactgtggaatttaaaaatgtttctttcaattatccatcaagaccatctatcaagattctgaaaggtctgaatctcagaattaagtctggagagacagtcgccttggtcggtctcaatggcagtgggaagagtacggtagtccagcttctgcagaggttatatgatccggatgatggctttatcatggtggatgagaatgacatcagagctttaaatgtgcggcattatcgagaccatattggagtggttagtcaagagcctgttttgttcgggaccaccatcagtaacaatatcaagtatggacgagatgatgtgactgatgaagagatggagagagcagcaagggaagcaaatgcgtatgattttatcatggagtttcctaataaatttaatacattggtaggggaaaaaggagctcaaatgagtggagggcagaaacagaggatcgcaattgctcgtgccttagttcgaaaccccaagattctgattttagatgaggctacgtctgccctggattcagaaagcaagtcagctgttcaagctgcactggagaaggcgagcaaaggtcggactacaatcgtggtagcacaccgactttctactattcgaagtgcagatttgattgtgaccctaaaggatggaatgctggcggagaaaggagcacatgctgaactaatggcaaaacgaggtctatattattcacttgtgatgtcacaggatattaaaaaagctgatgaacagatggagtcaatgacatattctactgaaagaaagaccaactcacttcctctgcactctgtgaagagcatcaagtcagacttcattgacaaggctgaggaatccacccaatctaaagagataagtcttcctgaagtctctctattaaaaattttaaagttaaacaagcctgaatggccttttgtggttctggggacattggcttctgttctaaatggaactgttcatccagtattttccatcatctttgcaaaaattataaccatgtttggaaataatgataaaaccacattaaagcatgatgcagaaatttattccatgatattcgtcattttgggtgttatttgctttgtcagttatttcatgcagggattattttacggcagagcaggggaaattttaacgatgagattaagacacttggccttcaaagccatgttatatcaggatattgcctggtttgatgaaaaggaaaacagcacaggaggcttgacaacaatattagccatagatatagcacaaattcaaggagcaacaggttccaggattggcgtcttaacacaaaatgcaactaacatgggactttcagttatcatttcctttatatatggatgggagatgacattcctgattctgagtattgctccagtacttgccgtgacaggaatgattgaaaccgcagcaatgactggatttgccaacaaagataagcaagaacttaagcatgctggaaagatagcaactgaagctttggagaatatacgtactatagtgtcattaacaagggaaaaagccttcgagcaaatgtatgaagagatgcttcagactcaacacagaaatacctcgaagaaagcacagattattggaagctgttatgcattcagccatgcctttatatattttgcctatgcggcagggtttcgatttggagcctatttaattcaagctggacgaatgaccccagagggcatgttcatagtttttactgcaattgcatatggagctatggccatcggagaaacgctcgttttggctcctgaatattccaaagccaaatcgggggctgcgcatctgtttgccttgttggaaaagaaaccaaatatagacagccgcagtcaagaagggaaaaagccagacacatgtgaagggaatttagagtttcgagaagtctctttcttctatccatgtcgcccagatgttttcatcctccgtggcttatccctcagtattgagcgaggaaagacagtagcatttgtggggagcagcggctgtgggaaaagcacttctgttcaacttctgcagagactttatgaccccgtgcaaggacaagtgctgtttgatggtgtggatgcaaaagaattgaatgtacagtggctccgttcccaaatagcaatcgttcctcaagagcctgtgctcttcaactgcagcattgctgagaacatcgcctatggtgacaacagccgtgtggtgccattagatgagatcaaagaagccgcaaatgcagcaaatatccattcttttattgaaggtctccctgagaaatacaacacacaagttggactgaaaggagcacagctttctggcggccagaaacaaagactagctattgcaagggctcttctccaaaaacccaaaattttattgttggatgaggccacttcagccctcgataatgacagtgagaaggtggttcagcatgcccttgataaagccaggacgggaaggacatgcctagtggtcactcacaggctctctgcaattcagaacgcagatttgatagtggttctgcacaatggaaagataaaggaacaaggaactcatcaagagctcctgagaaatcgagacatatattttaagttagtgaatgcacagtcagtgcagtgatgctgttgaggtagcacatattttgatgttcgtgtaatgcaaagaaggagtacttaataattacttggcaagctttgatctcttttattgcatatatcaatacctagaatcatgctactcaagtacatacatgttctattcacacaccatctgaccttcagatttttaaaaggaagcaaaaatttgcttatttcatgtaagtgaaataatgcttatatccttcactttataaaactattctagcacatttgcttgtaaagcagttttctacaaggtgaatttatttcccatcaacttctgctataaaatcggaaatatgtttccagggggaatattatccaattaaccatgttgaaggttttagcaaaggcagtgtaagatagagtggggcctgtagcattgcagggagagtgtctttcacttggaattttgttttgcagcacatattacagtagttttgctagtcccttttctccagaccgtagggatttctctcaataagtattcactatttctctaaattttattctatttttttgttgagcagggaatagaaaggattacgatgtaaaatttctgggaggattaggtagctatctcctacttcaccagtaagtgaagtgcctcacatgagccatcccaaagattcattattccaaaccttgggtttggcagtataagtcacaggcctacctgtttatgaaaacttacttacttaaaataagagctacttttgggccgggtgcggtggctcacgcctgtaatcccagaactttgggaggccgaggagggcggatcacttgaggtcaggagttcgagaccagcctggccaacatggtgaaaccccgtctctactaaaaacacaaaaattagccaatcttggtggcgggcacctggaatcccagctacttgggaggctgaggcaggagaatcatttgaacctaggaggcagaggttgcagtgagccgagatctcaccactgcactccagcctgcgcaacagagcgagactccatctcaaaaaataataaataagagctaattttattgtgggtgaaaatttttaaacgtctttctctataataaaataatttccttaaattttatatatactttatcatatataatgtgtgaatgattttaaagttctgtgtaaataacaatattggtaaaatgagttacattttcaacttacttaaatatgtaatgtcacctggtgattttatctttattcttcagtgtattttcttccatttacacatttagctagcctccctaaagtgtactctaccaataattgaaatcttgttaaacaaaattaaaaccatttatatattatgctgctttctttaaaatgcaaaataaaaataagattggggacttgagaatca

SEQ ID NO: 19 - RNA, 1724 nt, Homo sapiens
  source 1..1724: mol_type = mRNA
attgcttctcggccttttggctaagatcaagtgtaatctgtgttcttttttatttggtcatatcttccattctttcttacctaattcctctaatatctctctgtgagcctaaaccaataattatatattacattctattgtctttcttatataactgcagaaagataaatatcactttgtttgttcctgtaggttttctttagtgtaatccatagcagttattgcattggagcagcagtccctcactttgaaaccttcgcaatagcccgaggagctgcctttcatattttccaggttattgataagaaacccagtatagataacttttccacagctggatataaacctgaatccatagaaggaactgtggaatttaaaaatgtttctttcaattatccatcaagaccatctatcaagattctgaaaggtctgaatctcagaattaagtctggagagacagtcgccttggtcggtctcaatggcagtgggaagagtacggtagtccagcttctgcagaggttatatgatccggatgatggctttatcatggtggatgagaatgacatcagagctttaaatgtgcggcattatcgagaccatattggagtggttagtcaagagcctgttttgttcgggaccaccatcagtaacaatatcaagtatggacgagatgatgtgactgatgaagagatggagagagcagcaagggaagcaaatgcgtatgattttatcatggagtttcctaataaatttaatacattggtaggggaaaaaggagctcaaatgagtggagggcagaaacagaggatcgcaattgctcgtgccttagttcgaaaccccaagattctgattttagatgaggctacgtctgccctggattcagaaagcaagtcagctgttcaagctgcactggagaagaaaaaataatacaacaaagacgtattgataatctaccacactatctacgttgaggtatctggaaccacagtggtatgaattgcactatctccctaatctttacactaattctggctaaaagacagcatcagctcaaattttcctgatcagttttttagcaggctttggctgccaaaatctcttctgtgttttaagtctgaagcaattacagttgaatattttgttgttgttcactatgaggagtatatcggttttaggtcacatgaatgatctagtagagatgtatttttctagtacacttgatagtaccttgaatatgtacagtacatgtaggcccattttatggacctctgaggcacagttttttcccttttaagttattagatatttctgtgatttatttgatgcactcagatacaaattcatgctataataagttaaattgtaacataatatctaccttaatcaaatatttatagtttaggccaggagcctggcaaagtaaagatgacacagatgaaatgcttgataagtaaataaatatgagaagagatatatattaaaacacctgtgaagtgaatcccctgtgaagaaaagaaggtctctaacaatataaacctgtatcaggaaaccctgtgattctgattctgtgcacagaaggatacatggaattctcagaccttttctagttgcaaccttttaattgtttgactttatattctgtcctctcaaattctccttagactgtgacgtgttaatgctctcttttatattttctaattaaattccatacacattaatttgag

SEQ ID NO: 20 - protein, 471 aa, Homo sapiens
MHPGVLAAFLFLSWTHCRALPLPSGGDEDDLSEEDLQFAERYLRSYYHPTNLAGILKENAASSMTERLREMQSFFGLEVTGKLDDNTLDVMKKPRCGVPDVGEYNVFPRTLKWSKMNLTYRIVNYTPDMTHSEVEKAFKKAFKVWSDVTPLNFTRLHDGIADIMISFGIKEHGDFYPFDGPSGLLAHAFPPGPNYGGDAHFDDDETWTSSSKGYNLFLVAAHEFGHSLGLDHSKDPGALMFPIYTYTGKSHFMLPDDDVQGIQSLYGPGDEDPNPKHPKTPDKCDPSLSLDAITSLRGETMIFKDRFFWRLHPQQVDAELFLTKSFWPELPNRIDAAYEHPSHDLIFIFRGRKFWALNGYDILEGYPKKISELGLPKEVKKISAAVHFEDTGKTLLFSGNQVWRYDDTNHIMDKDYPRLIEEDFPGIGDKVDAVYEKNGYIYFFNGPIQFEYSIWSNRIVRVMPANSILWC

SEQ ID NO: 21 - RNA, 2735 nt, Homo sapiens
  source 1..2735: mol_type = mRNA
acaacagtccccaggcatcaccattcaagatgcatccaggggtcctggctgccttcctcttcttgagctggactcattgtcgggccctgccccttcccagtggtggtgatgaagatgatttgtctgaggaagacctccagtttgcagagcgctacctgagatcatactaccatcctacaaatctcgcgggaatcctgaaggagaatgcagcaagctccatgactgagaggctccgagaaatgcagtctttcttcggcttagaggtgactggcaaacttgacgataacaccttagatgtcatgaaaaagccaagatgcggggttcctgatgtgggtgaatacaatgttttccctcgaactcttaaatggtccaaaatgaatttaacctacagaattgtgaattacacccctgatatgactcattctgaagtcgaaaaggcattcaaaaaagccttcaaagtttggtccgatgtaactcctctgaattttaccagacttcacgatggcattgctgacatcatgatctcttttggaattaaggagcatggcgacttctacccatttgatgggccctctggcctgctggctcatgcttttcctcctgggccaaattatggaggagatgcccattttgatgatgatgaaacctggacaagtagttccaaaggctacaacttgtttcttgttgctgcgcatgagttcggccactccttaggtcttgaccactccaaggaccctggagcactcatgtttcctatctacacctacaccggcaaaagccactttatgcttcctgatgacgatgtacaagggatccagtctctctatggtccaggagatgaagaccccaaccctaaacatccaaaaacgccagacaaatgtgacccttccttatcccttgatgccattaccagtctccgaggagaaacaatgatctttaaagacagattcttctggcgcctgcatcctcagcaggttgatgcggagctgtttttaacgaaatcattttggccagaacttcccaaccgtattgatgctgcatatgagcacccttctcatgacctcatcttcatcttcagaggtagaaaattttgggctcttaatggttatgacattctggaaggttatcccaaaaaaatatctgaactgggtcttccaaaagaagttaagaagataagtgcagctgttcactttgaggatacaggcaagactctcctgttctcaggaaaccaggtctggagatatgatgatactaaccatattatggataaagactatccgagactaatagaagaagacttcccaggaattggtgataaagtagatgctgtctatgagaaaaatggttatatctattttttcaacggacccatacagtttgaatacagcatctggagtaaccgtattgttcgcgtcatgccagcaaattccattttgtggtgttaagtgtctttttaaaaattgttatttaaatcctgaagagcatttggggtaatacttccagaagtgcggggtaggggaagaagagctatcaggagaaagcttggttctgtgaacaagcttcagtaagttatctttgaatatgtagtatctatatgactatgcgtggctggaaccacattgaagaatgttagagtaatgaaatggaggatctctaaagagcatctgattcttgttgctgtacaaaagcaatggttgatgatacttcccacaccacaaatgggacacatggtctgtcaatgagagcataatttaaaaatatatttataaggaaattttacaagggcataaagtaaatacatgcatataatgaataaatcattcttactaaaaagtataaaatagtatgaaaatggaaatttgggagagccatacataaaagaaataaaccaaaggaaaatgtctgtaataatagactgtaacttccaaataaataattttcattttgcactgaggatattcagatgtatgtgcccttcttcacacagacactaacgaaatatcaaagtcattaaagacaggagacaaaagagcagtggtaagaatagtagatgtggcctttgaattctgtttaattttcacttttggcaatgactcaaagtctgctctcatataagacaaatattcctttgcatattataaaggataaagaaggatgatgtctttttattaaaatatttcaggttcttcagaagtcacacattacaaagttaaaattgttatcaaaatagtctaaggccatggcatccctttttcataaattatttgattatttaagactaaaagttgcattttaaccctattttacctagctaattatttaattgtccagtttgtcttggatatataggctattttctaaagacttgtatagcatgaaataaaatatatcttataaagtggaagtatgtatattaaaaaagagacatccaaatttttttttaaagcagtctactagattgtgatcccttgagatatggaaggatgcctttttttctctgcatttaaaaaaatcccccagcacttcccacagtgcctattgatacttggggagggtgcttggcacttattgaatatatgatcggccatcaagggaagaactattgtgctcagagacactgttgataaaaactcaggcaaagaaaatgaaatgcatatttgcaaagtgtattaggaagtgtttatgttgtttataataaaaatatattttcaacagacaaaaaaaaaaaaaaaaaa

SEQ ID NO: 22 - protein, 1261 aa, Homo sapiens
MSGSKSVSPPGYAAQKTAAPAPRGGPEHRSAWGEADSRANGYPHAPGGSARGSTKKPGGAVTPQQQQRLASRWRSDDDDDPPLSGDDPLAGGFGFSFRSKSAWQERGGDDCGRGSRRQRRGAASGGSTRAPPAGGGGGSAAAAASAGGTEVRPRSVEVGLEERRGKGRAADELEAGAVEGGEGSGDGGSSADSGSGAGPGAVLSLGACCLALLQIFRSKKFPSDKLERLYQRYFFRLNQSSLTMLMAVLVLVCLVMLAFHAARPPLQLPYLAVLAAAVGVILIMAVLCNRAAFHQDHMGLACYALIAVVLAVQVVGLLLPQPRSASEGIWWTVFFIYTIYTLLPVRMRAAVLSGVLLSALHLAIALRTNAQDQFLLKQLVSNVLIFSCTNIVGVCTHYPAEVSQRQAFQETRECIQARLHSQRENQQQERLLLSVLPRHVAMEMKADINAKQEDMMFHKIYIQKHDNVSILFADIEGFTSLASQCTAQELVMTLNELFARFDKLAAENHCLRIKILGDCYYCVSGLPEARADHAHCCVEMGMDMIEAISLVREVTGVNVNMRVGIHSGRVHCGVLGLRKWQFDVWSNDVTLANHMEAGGKAGRIHITKATLNYLNGDYEVEPGCGGERNAYLKEHSIETFLILRCTQKRKEEKAMIAKMNRQRTNSIGHNPPHWGAERPFYNHLGGNQVSKEMKRMGFEDPKDKNAQESANPEDEVDEFLGRAIDARSIDRLRSEHVRKFLLTFREPDLEKKYSKQVDDRFGAYVACASLVFLFICFVQITIVPHSIFMLSFYLTCSLLLTLVVFVSVIYSCVKLFPSPLQTLSRKIVRSKMNSTLVGVFTITLVFLAAFVNMFTCNSRDLLGCLAQEHNISASQVNACHVAESAVNYSLGDEQGFCGSPWPNCNFPEYFTYSVLLSLLACSVFLQISCIGKLVLMLAIELIYVLIVEVPGVTLFDNADLLVTANAIDFFNNGTSQCPEHATKVALKVVTPIIISVFVLALYLHAQQVESTARLDFLWKLQATEEKEEMEELQAYNRRLLHNILPKDVAAHFLARERRNDELYYQSCECVAVMFASIANFSEFYVELEANNEGVECLRLLNEIIADFDEIISEDRFRQLEKIKTIGSTYMAASGLNDSTYDKVGKTHIKALADFAMKLMDQMKYINEHSFNNFQMKIGLNIGPVVAGVIGARKPQYDIWGNTVNVASRMDSTGVPDRIQVTTDMYQVLAANTYQLECRGVVKVKGKGEMMTYFLNGGPPLS

SEQ ID NO: 23 - protein, 911 aa, Homo sapiens
MKSQKEGCCSRGDLSIQTGPGGEWAPRRLVSNVLIFSCTNIVGVCTHYPAEVSQRQAFQETRECIQARLHSQRENQQQERLLLSVLPRHVAMEMKADINAKQEDMMFHKIYIQKHDNVSILFADIEGFTSLASQCTAQELVMTLNELFARFDKLAAENHCLRIKILGDCYYCVSGLPEARADHAHCCVEMGMDMIEAISLVREVTGVNVNMRVGIHSGRVHCGVLGLRKWQFDVWSNDVTLANHMEAGGKAGRIHITKATLNYLNGDYEVEPGCGGERNAYLKEHSIETFLILRCTQKRKEEKAMIAKMNRQRTNSIGHNPPHWGAERPFYNHLGGNQVSKEMKRMGFEDPKDKNAQESANPEDEVDEFLGRAIDARSIDRLRSEHVRKFLLTFREPDLEKKYSKQVDDRFGAYVACASLVFLFICFVQITIVPHSIFMLSFYLTCSLLLTLVVFVSVIYSCVKLFPSPLQTLSRKIVRSKMNSTLVGVFTITLVFLAAFVNMFTCNSRDLLGCLAQEHNISASQVNACHVAESAVNYSLGDEQGFCGSPWPNCNFPEYFTYSVLLSLLACSVFLQISCIGKLVLMLAIELIYVLIVEVPGVTLFDNADLLVTANAIDFFNNGTSQCPEHATKVALKVVTPIIISVFVLALYLHAQQVESTARLDFLWKLQATEEKEEMEELQAYNRRLLHNILPKDVAAHFLARERRNDELYYQSCECVAVMFASIANFSEFYVELEANNEGVECLRLLNEIIADFDEIISEDRFRQLEKIKTIGSTYMAASGLNDSTYDKVGKTHIKALADFAMKLMDQMKYINEHSFNNFQMKIGLNIGPVVAGVIGARKPQYDIWGNTVNVASRMDSTGVPDRIQVTTDMYQVLAANTYQLECRGVVKVKGKGEMMTYFLNGGPPLS

SEQ ID NO: 24 - RNA, 3326 nt, Homo sapiens
  source 1..3326: mol_type = mRNA
gccacgctgtcctccctcctccgctccctgcgccccacccctggcggccgcgctgcctggcagcccgggaagccgcggcacagctgctcggcgcctgcagctccggctcgggggctggaaccgaagcgggggcggcgggagcgcggagaccacagcccccggggagaggcggagggggtccctggcctgggcggagaggctgagctgagtgcgcgtgagaaagagggctgcaccgctgctcggcgcggactctgccagccccagcttcagccccggctcaggtcgccgcagcccgggagcctccccgcttgcgccccaaggcacgcgcggcacagccatgaacaccaacgatgccaaggagtatctggcccggagggaaatccctcagctttttgagagccttttgaatggactgatgtgttctaagcccgaagatccagtagaatacttggaaagttgtttacaaaaagtaaaggaactgggtggctgtgacaaggtgaaatgggatacatttgtaagccaggaaaagaagaccttacctccactaaatggaggacagtcacggagatcctttctaagaaatgtaatgcctgaaaactcaaactttccatatcggcggtatgaccggctccctccaatccatcaattctccatagaaagtgacacggatctctctgagactgcagagttgattgaggagtatgaggtttttgatcctaccagacctcgaccaaaaatcattcttgttataggtggtccaggaagtggaaagggtactcagagtttgaaaattgcagaacgatatggattccaatacatttctgtgggagaattattaagaaagaagatccacagtaccagcagcaataggaaatggagtcttattgccaagataattacaactggagaattggccccacaggaaacaacaattacagagataaaacaaaaattgatgcaaatacctgatgaagagggcattgttattgatggatttccaagagatgttgcccaggctctatcttttgaggaccaaatctgtacccccgatttggtggtattcctggcttgtgctaatcagagactcaaagaaagattactgaagcgtgcagaacagcagggccgaccagacgacaatgtaaaagctacccaaaggagactaatgaacttcaagcagaatgctgctccattggttaaatacttccaggaaaaggggctcatcatgacatttgatgccgaccgcgatgaggatgaggtgttctatgacatcagcatggcagttgacaacaagttatttccaaacaaagaggctgcagcaggttcaagtgaccttgatccttcgatgatattggacactggagagatcattgatacaggatctgattatgaagatcagggtgatgaccagttaaatgtatttggagaggacactatgggaggtttcatggaagatttgagaaagtgtaaaattattttcataattggtggtcctggctctggcaaaggcacacagtgtgaaaagctggtggaaaaatatggatttacacatctctcaactggcgagctcctgcgtgaggaactggcatcagaatctgaaagaagcaaattgatcagagacattatggaacgtggagacctggtgccctcaggcatcgttttggagctcctgaaggaggccatggtggccagcctcggggacaccaggggcttcctgattgacggctatcctcgggaggtgaagcaaggggaagagttcggacgcaggattggagacccacagttggtgatctgtatggactgctcggcagacaccatgaccaaccgccttctccaaaggagccggagcagcctgcctgtggacgacaccaccaagaccatcgccaagcgcctagaagcctactaccgagcgtccatccccgtgatcgcctactacgagacaaaaacacagctacacaagataaatgcagagggaacaccagaggacgtttttcttcaactctgcacagctattgactctattttctgaaggcaaaaatgcatgtttgttagaatggaaacagaaaaacattaaaaagttcattccttaacacaatgtttcaagttaaaccttttgtgtcaccgcccccaccaaccaccacctcctaaatcctgacagcactgtttgcttcccagctagacctgtgtgagaggtgtctggaaatcatgcatggtgtatttgggactatatcaacctattctccacacttcagacaactgtctgcactcacggcacacacactttgtatcatgcaggccacactcagagctagtcagtacatgaacagtggtgcggtgccagtctgtgtccgttgtgatcacaggccttgctagaccctgatcatctggttctcctctcattaagcatccctaacccccagtcacaccttcctcttacatactgttccccaatggaggcccctggcataggggacagccctgggcatcttcctttggtgtctggctgttttgtcaactctcatccactggtggctcagagccataaggtgggttgattacacaatgccttgtacatgatatagaggcatcaagcaagtaaaatttgacagaaattttaaaatatgaagatgtatagctttcccaagatgatggtaaaacccaggttagtcatcagtaaccttctctattattattattttttagaaacttggaatactgtcgtcatggctaagagaacaaatctgataaattgtgtaacctagtctcttctctacatggtgatgcatttcagcaattataaattaatataaatgaccaaaagtaacttaaaagcatgagatatttgctatttcattcattgggcacatatcaaattataattttgattttaaatggtcacccatgtatttatttgttgccaagcaagtaaaaaaataccctaacaaacctgatgtgggtgggaggggcatgtcagtaagtggtgtgttcaatgtgtttgtttcatatgggccctttccaggagtttgcaaaccttgtcatacccatatgcaaaactgtgtttccttgcattaaaccagtgaagtttgggttctcttttgtgctatcaatcagttgtaaaatcagagctgcttatatattctactggaataactgcatcttccactcagtcactacaaaaaagcatagtttcagtttgcatgaatttttttttttttcttcaatggctgtgcagataaggatccatttctgggatagaattgtattttttaagtcatttttttttcttgaaatggatatgtacaaataaaataaatggaagacaggataaa

SEQ ID NO: 25 - RNA, 3937 nt, Homo sapiens
  source 1..3937: mol_type = mRNA
agtcttccagcagggttctgaaagcagcctgctcccatcgcgcccctcggatgtggacacccagggtgggctgcagaccgcggccgggccgcactctctgggggcgagggccaggtcaggtggctgcactgtcgcccagcagcgagtaaagactcgaaactgagggagccagagccctagtcactctgctggtcgagggtcggaaccgctgggggaaagaggaaatgtggacgaaggcagcccttcctggagacagcttggaagagagggatgaagatgcaaaaagcaaaacccaacctatcaagtgccacctccccggtgacaggcccccagccttgctctgcgctttcgctgaatgaactcctgagcacgtttttcccgttgcctaggaagggttgggccgcaggtttcgccagtgctcgacaacccacctggagatagcgggtcggggagggagctgcgaggggggcggactcctgttgctcagtcttcagaccgcagcacagcatcatctgcaccgggacccgggaatggggggacacttggagactgagagagaggaggctcgaggaatgaaccttggtctgttctaagccacaacccctgtctcaggtcgtttggcttcctttccttctctttgtatttgaatttaaaaacattcctgaatctcaagtgcttttgcttgaagtaggggggaggaggagaaaagaatagaagcaagccaggcttcctaagcgagctctgaaaggagaaatccattcactgcaaacctcgttccccatttctgaaaacggatagactgatatcgtaaactaaaggtcatgagggtttttccccccggtttgggggatttgttctgttaaaaggaattttaaagcaccacttgagaaaataattttgcctcagtttccctaaactatctttaaaatgggttgccataattacaggtcttcttttctctcacctctataagccaccgttttcaggtcatctgaagtcaagatttccagccttttgaatggactgatgtgttctaagcccgaagatccagtagaatacttggaaagttgtttacaaaaagtaaaggaactgggtggctgtgacaaggtgaaatgggatacatttgtaagccaggaaaagaagaccttacctccactaaatggaggacagtcacggagatcctttctaagaaatgtaatgcctgaaaactcaaactttccatatcggcggtatgaccggctccctccaatccatcaattctccatagaaagtgacacggatctctctgagactgcagagttgattgaggagtatgaggtttttgatcctaccagacctcgaccaaaaatcattcttgttataggtggtccaggaagtggaaagggtactcagagtttgaaaattgcagaacgatatggattccaatacatttctgtgggagaattattaagaaagaagatccacagtaccagcagcaataggaaatggagtcttattgccaagataattacaactggagaattggccccacaggaaacaacaattacagagataaaacaaaaattgatgcaaatacctgatgaagagggcattgttattgatggatttccaagagatgttgcccaggctctatcttttgaggaccaaatctgtacccccgatttggtggtattcctggcttgtgctaatcagagactcaaagaaagattactgaagcgtgcagaacagcagggccgaccagacgacaatgtaaaagctacccaaaggagactaatgaacttcaagcagaatgctgctccattggttaaatacttccaggaaaaggggctcatcatgacatttgatgccgaccgcgatgaggatgaggtgttctatgacatcagcatggcagttgacaacaagttatttccaaacaaagaggctgcagcaggttcaagtgaccttgatccttcgatgatattggacactggagagatcattgatacaggatctgattatgaagatcagggtgatgaccagttaaatgtatttggagaggacactatgggaggtttcatggaagatttgagaaagtgtaaaattattttcataattggtggtcctggctctggcaaaggcacacagtgtgaaaagctggtggaaaaatatggatttacacatctctcaactggcgagctcctgcgtgaggaactggcatcagaatctgaaagaagcaaattgatcagagacattatggaacgtggagacctggtgccctcaggcatcgttttggagctcctgaaggaggccatggtggccagcctcggggacaccaggggcttcctgattgacggctatcctcgggaggtgaagcaaggggaagagttcggacgcaggattggagacccacagttggtgatctgtatggactgctcggcagacaccatgaccaaccgccttctccaaaggagccggagcagcctgcctgtggacgacaccaccaagaccatcgccaagcgcctagaagcctactaccgagcgtccatccccgtgatcgcctactacgagacaaaaacacagctacacaagataaatgcagagggaacaccagaggacgtttttcttcaactctgcacagctattgactctattttctgaaggcaaaaatgcatgtttgttagaatggaaacagaaaaacattaaaaagttcattccttaacacaatgtttcaagttaaaccttttgtgtcaccgcccccaccaaccaccacctcctaaatcctgacagcactgtttgcttcccagctagacctgtgtgagaggtgtctggaaatcatgcatggtgtatttgggactatatcaacctattctccacacttcagacaactgtctgcactcacggcacacacactttgtatcatgcaggccacactcagagctagtcagtacatgaacagtggtgcggtgccagtctgtgtccgttgtgatcacaggccttgctagaccctgatcatctggttctcctctcattaagcatccctaacccccagtcacaccttcctcttacatactgttccccaatggaggcccctggcataggggacagccctgggcatcttcctttggtgtctggctgttttgtcaactctcatccactggtggctcagagccataaggtgggttgattacacaatgccttgtacatgatatagaggcatcaagcaagtaaaatttgacagaaattttaaaatatgaagatgtatagctttcccaagatgatggtaaaacccaggttagtcatcagtaaccttctctattattattattttttagaaacttggaatactgtcgtcatggctaagagaacaaatctgataaattgtgtaacctagtctcttctctacatggtgatgcatttcagcaattataaattaatataaatgaccaaaagtaacttaaaagcatgagatatttgctatttcattcattgggcacatatcaaattataattttgattttaaatggtcacccatgtatttatttgttgccaagcaagtaaaaaaataccctaacaaacctgatgtgggtgggaggggcatgtcagtaagtggtgtgttcaatgtgtttgtttcatatgggccctttccaggagtttgcaaaccttgtcatacccatatgcaaaactgtgtttccttgcattaaaccagtgaagtttgggttctcttttgtgctatcaatcagttgtaaaatcagagctgcttatatattctactggaataactgcatcttccactcagtcactacaaaaaagcatagtttcagtttgcatgaatttttttttttttcttcaatggctgtgcagataaggatccatttctgggatagaattgtattttttaagtcatttttttttcttgaaatggatatgtacaaataaaataaatggaagacaggataaa

SEQ ID NO: 26 - protein, 350 aa, Homo sapiens
MLEGAELYFNVDHGYLEGLVRGCKASLLTQQDYINLVQCETLEDLKIHLQTTDYGNFLANHTNPLTVSKIDTEMRKRLCGEFEYFRNHSLEPLSTFLTYMTCSYMIDNVILLMNGALQKKSVKEILGKCHPLGRFTEMEAVNIAETPSDLFNAILIETPLAPFFQDCMSENALDELNIELLRNKLYKSYLEAFYKFCKNHGDVTAEVMCPILEFEADRRAFIITLNSFGTELSKEDRETLYPTFGKLYPEGLRLLAQAEDFDQMKNVADHYGVYKPLFEAVGGSGGKTLEDVFYEREVQMNVLAFNRQFHYGVFYAYVKLKEQEIRNIVWIAECISQRHRTKINSYIPIL

SEQ ID NO: 27 - RNA, 2370 nt, Homo sapiens
  source 1..2370: mol_type = mRNA
gcaaatcttcaggggccgtccaggactacagagctgtttcaccctaccttggcttcaatctcttcccccatgctcgaaggtgcggagctgtacttcaacgtggaccatggctacctggagggcctggttcgaggatgcaaggccagcctcctgacccagcaagactatatcaacctggtccagtgtgagaccctagaagacctgaaaattcatctccagactactgattatggtaactttttggctaatcacacaaatcctcttactgtttccaaaattgacactgagatgaggaaaagactatgtggagaatttgagtatttccggaatcattccctggagcccctcagcacatttctcacctatatgacgtgcagttatatgatagacaatgtgattctgctgatgaatggtgcattgcagaaaaaatctgtgaaagaaattctggggaagtgccaccccttgggccgtttcacagaaatggaagctgtcaacattgcagagacaccttcagatctctttaatgccattctgatcgaaacgccattagctccattcttccaagactgcatgtctgaaaatgctctagatgaactgaatattgaattgctacgcaataaactatacaagtcttaccttgaggcattctataaattctgtaagaatcatggtgatgtcacagcagaagttatgtgtcccattcttgagtttgaggccgacagacgtgcttttatcatcactcttaactcctttggcactgaattgagcaaagaagaccgagagaccctctatccaaccttcggcaaactctatcctgaggggttgcggctgttggctcaagcagaagactttgaccagatgaagaacgtagcggatcattacggagtatacaaacctttatttgaagctgtaggtggcagtgggggaaagacattggaggacgtgttttacgagcgtgaggtacaaatgaatgtgctggcattcaacagacagttccactacggtgtgttttatgcatatgtaaagctgaaggaacaggaaattagaaatattgtgtggatagcagaatgtatttcacagaggcatcgaactaaaatcaacagttacattccaattttataacccaagtaaggttctcaaatgtagaaaattataaatgttaaaaggaagttattgaagaaaataaaagaaattatgttatattatctagactacacaaaagtaagccacactatatcttcatgagttgcaaatccatggaaacacagtaaaccagccctgaaacaaagcatttccttgttttcagtggtattagatcttgtttccacatgtctgtctcattcttcactgggccttacaggttagttttaattaactctatggtatttttcttattcttgtttgatcatgttaaaaattggacctaataaaagtattttattcttgcttttccatgcttctctacaggtccaaatactgaatgtctcctttactttttctcttttaaatttttttctagacagggtctcactctgtcacctaggctacagtgcagtggtgtgatcacagctcactgcagcctcgacttcccaggctcaagtgatcctcccagctctcagcctccaaagtagctggcactacaagtgtacacccccacacaaggctaagttttgtattttttgtagagacagggtttcaacatattatccaggctggtgtcgaattcctgggctccagggatccacagtcccccttggcctcccaaagtgttgggattacatgcatgagccactgtgctgggcttcatttacattttaactgtctgttccttgcctagattcacagaaatccaaagctgtatgtagtcaacatggttcacaagtgttggaaaatgtgttttttgttttgttttgttttgtttcgttttgttttgagacagagtttccctctgtcgcccaggctagagtgcaatggcgtgatctcggctcactgcaacctccacctcccagattcaagcaactctctgcctcagcctcccgagtagctgggattacaagcacccaccactacactcagctaattttttgtatttttagtagagccggggtttcaccatcttggccaggctgatcttgaactcctgagctcatgatccacccgcctcagcctcccaaagtgctgggattacaggccccttgttcagccactgcacctggccccttattttgtttttgttttctaatatactttgatgtaatcagcttgagaaagcaacacaatttcaaatcctatcttctagatgcaagcagtgttaaatttgttaataaatttgcttttcacacctttctttaaataaaaggtatatctctc

SEQ ID NO: 28 - protein, 199 aa, Homo sapiens
MPEQSNDYRVAVFGAGGVGKSSLVLRFVKGTFRESYIPTVEDTYRQVISCDKSICTLQITDTTGSHQFPAMQRLSISKGHAFILVYSITSRQSLEELKPIYEQICEIKGDVESIPIMLVGNKCDESPSREVQSSEAEALARTWKCAFMETSAKLNHNVKELFQELLNLEKRRTVSLQIDGKKSKQQKRKEKLKGKCVIM

SEQ ID NO: 29 - RNA, 4386 nt, Homo sapiens
  source 1..4386: mol_type = mRNA
atttaagcaggagcagcagcctctgcagcagttggcacatctgagaaggcagagattgaagagagtaggaggagcgtgcagcggcggtgacagtgccaggccggagcggctcaggccagcgcaggtgcaggggctgcgagcgggtggagcgcgagggcgctgggcgcagggagcacggccggtgggcggtgcagggcgcacggcgggcgagcagctgacagcatcgtcacggcggcgggagggagtgcgctgcgcctgcctccgggaggagccgcatccacacaccctgcgctgccctgtcctgcgcgagtggagctctgaagaagctctgagcggagttgtgttcttccccaggtgcgtcctggctgagagttggagctctccagcaacatgcctgagcagagtaacgattaccgggtggccgtgtttggggctggcggtgttggcaagagctccctggtgttgaggtttgtgaaaggcacattccgggagagctacatcccgacggtggaagacacctaccggcaagtgatcagctgtgacaagagcatatgcacattgcagatcaccgacacgacggggagccaccagttcccggccatgcagcggctgtccatctccaaagggcacgccttcatcctggtgtactccattaccagccgacagtccttggaggagctcaagcccatctacgaacaaatctgcgagatcaaaggggacgtggagagcatccccatcatgctggtggggaacaagtgtgatgagagccccagccgcgaggtgcagagcagcgaggcggaggccttggcccgcacatggaagtgtgccttcatggagacctcagccaagctcaaccataacgtgaaggagcttttccaggagctgctcaacctggagaagcgcaggaccgtgagtctccagatcgacgggaaaaagagcaagcagcagaaaaggaaagagaagctcaaaggcaagtgcgtgatcatgtgaaggcccttcctgcgggaggagcagctgtgtgtccccggcacctcactcccccaaaatgacacccaccgtcgtcagggtagcatgtataatgcccacgtgttaaacattgcatttaatcgagatgcgtcctattgtccttaagagggcgtttcacaccaccaacagtaagccacccactctggagtcacagaatctgccaggcggttcaagtgaaaaccaacacactcagcatccctgggaactgagaggtgccagcaattgctgaaggtggcgatgaacacccgaaggtgggagggaggactggtacccacaaagcaacatgtaccgagaggactaaatgtcatctacgtgcatgtgagagcgtgttaacctagagttacctgcaccaaccccagacagaagccaatcacatctttgggggaggggaggggcaggaagaggtgagaagatcagatggtccaaagtggaccacacttggtccattttacacttttttaaaggggattaaaaaacacagcctctcccccaaagggtgtccgttcttaattcccacctggcctgttaggagccttgctaccctgaggggatgtgttcaccttacctagacctagttaggaagtatcattttaagctattagagtatttatcttcatgtgcagggataagtgcactaacagtgtgctgctctgtcggaagttcttcagtttttaagtgaggatatcgtgacagtattaaaacatcgcaataatgttcctgtgtgttatacatcgagggttttagaaatgtgattttcttcttttgacctgtgaggagtataacttctttcagccctcagattttaaatacaagcaaataaactcactatttttagacgtttttttcctccaaggtggttttcttctcttaaataactcgatctgtacccagctgggtagcagccagcaaaggccatcagacaaccagaagcacatccatttttgtagtgtcacaaacatgtatatgccacactttgcaccttaatgaaatactttgaaacagaagttattcactgtgtttttgatgatctatctgtattggaaatatgttcctggaaaatgcatttaaataatagtaaattctcttgcatgttccattatacgtgtcttctaagagctgttcaatacagtattcactctagaaacaattatctttttctcttaatgattttgtgtgcatctttaatctttcaagccaaattacagctatttcaggtttcctgtgttagcttggggataggatggtggctggagacaggcaggcttctctgccctgggaagagcccactcagcttaattgctctgccatcgtagagcctggttggacttggcttcctgaaaactcccactgatagtgcctgttagatctcctgtttgtttcagttggcagaacatttactggccccaactgtggcatcatcctctcagcagtcttcctgtcacccgcctggcaggcagaaggagctgcagtcccacgtgggcctgcctgggggggtgggggctgcatggctgttgggtggcagtgtcagcacagggagggcttaagttggggatgtttgaccaggccacctcctgcaactgctgtttctcctgtccctcctatgcagggcttgcagcagcagcagtgtggccatctccatcccccaaagcacacttgctctctcaatatgtcctagttttcttcagccttttctggttcagttcccttgtcctgatctcatcctctctggtctcccaataactcacccttgggatgtgtttagagcgtgggaggtgcctttgagaactgcttgactccatgatctcctagaacaaaaccgccctgactttacagggggaacactcatgctgagctgagaaagcagagaagtggcgtgggagccagctgggggtgaagagcatttgggccagtcccgtggcccccttcagattcctcaagcaggattgttctgttctaaaaagctgttgcacagcattcgcaatgagatctttagttggcggattttctggaacatttgtttttcaacttgtcccgacattttttttctgtttctattctgagagagagatgatcaagttttaatttgggtataggttaaatggaagaagaaacagaacttcatggccaaagtagacctatagattttgattgggttctttgttaacagtagaatgcgatctttgccactgactgtagtattaataaggttttaatgtgagatattcctgcaaaccatcccatttctactgattgtaagtcagaatttcttttatccctttcaaatcagtttctacatgtttaagtgttcagggcttcatcagcatgagaagtttgtaattactgaaagtctgatttcattcaggacacattttttccttcatattttttctgtgaatttataggctaggaaggctattgaagcctcaattatgggtcttcattttgagatcgttttctatgagctgaactgaggatatcaatggttatctcaaaatcgtcttttaggagatccccaattgactcagagtttgaggagttagtatcacagaattagatttttttaaagcatttgtacgtttccattcccaaatatgtagctgtggttcttgaaaacacatcctacattgcatatgggcatagcagtttttgacccaggcagaataagttaatatttaattaaatattgctttgaagatggcgctctgggcatgagcatggggctccatgacttcccttctatccccatgagcccctcctccatccagcgacaagccatgggcatgcatacaatgcagcaagaccaacacaagagcaatattgaattgttcattctatctaaaattacatgtatataaaatatataatttatcttcctgcatttttgaagtataaagtcataaattgtacatatctgtaagctagtatatttgtttcactgtttgtaatatttaagaaatgctcattctttgtagaacaaaaatgtattaaatattttaaaaattgctctgtgatacttaatttttttccccaaaatttgtaatgtgttgcttctacataagttctctggaaatatctacaactaataggacacatgtaaatccttgaagacacatcctggaattcataccccacaaggacagtgtgtatacaaagtatttgcagagcatgacttttatatgtgtgggatatcaatgtgtatatttatatttaaagtgtatttattgttacaagtctattctctattatattttatttactctgcggttataaaaatcacccttgcatacaagtttctagttgccagtgatgttctggaaataatgggagatattacaataaagctacagttatgacaccctg

SEQ ID NO: 30 - protein, 1186 aa, Homo sapiens
MKKFNFRKVLDGLTASSPGSGSSSGSNSGGGAGSGSVHPAGTAGVLREEIQETLTSEYFQICKTVRHGFPHQPTALAFDPVQKILAIGTRTGAIRILGRPGVDCYCQHESGAAVLQLQFLINEGALVSASSDDTLHLWNLRQKRPAILHSLKFNRERITYCHLPFQSKWLYVGTERGNTHIVNIESFILSGYVIMWNKAIELSTKTHPGPVVHLSDSPRDEGKLLIGYENGTVVFWDLKSKRAELRVYYDEAIHSIDWHHEGKQFMCSHSDGSLTLWNLKSPSRPFQTTIPHGKSQREGRKSESCKPILKVEYKTCKNSEPFIIFSGGLSYDKACRRPSLTIMHGKAITVLEMDHPIVEFLTLCETPYPNEFQEPYAVVVLLEKDLIVVDLTQSNFPIFENPYPMDIHESPVTCTAYFADCPPDLILVLYSIGVKHKKQGYSNKEWPISGGAWNLGAQTYPEIIITGHADGSIKFWDASAITLQMLYKLKTSKVFEKQKVGEGKQTCEIVEEDPFAIQMIYWCPESRIFCVSGVSAYVIIYKFSRHEITTEIVSLEVRLQYDVEDIITPEPETSPPFPDLSAQLPSSRSLSGSTNTVASEGVTKDSIPCLNVKTRPVRMPPGYQAELVIQLVWVDGEPPQQITSLAVSSAYGIVAFGNCNGLAVVDFIQKTVLLSMGTIDLYRSSDLYQRQPRSPRKNKQFIADNFCMRGLSNFYPDLTKRIRTSYQSLTELNDSPVPLELERCKSPTSDHVNGHCTSPTSQSCSSGKRLSSADVSKVNRWGPGRPPFRKAQSAACMEISLPVTTEENRENSYNRSRSSSISSIDKDSKEAITALYFMDSFARKNDSTISPCLFVGTSLGMVLIISLNLPLADEQRFTEPVMVLPSGTFLSLKGAVLTFSCMDRMGGLMQPPYEVWRDPNNIDENEKSWRRKVVMNSSSASQEIGDHQYTIICSEKQAKVFSLPSQTCLYVHNITETSFILQANVVVMCSSACLACFCANGHIMIMSLPSLRPMLDVNYLPLTDMRIARTFCFTNEGQALYLVSPTEIQRLTYSQEMCDNLQDMLGDLFTPIETPEAQNRGFLKGLFGGSGQTFDREELFGEASAGKASRSLAQHIPGPGSIEGMKGAAGGVMGELTRARIALDERGQRLGELEEKTAGMMTSAEAFSKHAHELMLKYKDKKWYQF

SEQ ID NO: 31 - protein, 74 aa, Homo sapiens
MKKFNFRKVLDGLTASSPGSGSSSGSNSGGGAGSGSVHPAGTAGVLREEIQETLTSEYFQICKFGMVFLISPQH

SEQ ID NO: 32 - RNA, 9382 nt, Homo sapiens
  source 1..9382: mol_type = mRNA
ctgactgctcggttaggacctcggagagcgccaggcgccgcgaccagagggcccagagaagcggccggagcccgcctacctcggccccctcagcttcccgggctggcaggcggctagaggcgtctgaggaagtgtttaaaatgaagaagtttaatttccgaaaagttttggatggcttaactgcctcctcccctggcagtggtagcagcagtggcagtaacagtggtggtggggctggaagtggttccgtacatccggcggggactgcaggggttctcagagaggaaattcaggaaactttgacttcggagtatttccagatttgcaagacagttcggcatggttttcctcatcagcccacagcattagcctttgatccagttcagaaaatcttggctattgggacgagaacaggtgctatacgaatactcgggagacctggtgttgattgctattgccaacatgaaagtggtgcagctgtcctacagctccaatttttgatcaatgagggtgccttggtcagtgcaagttcagatgatacacttcatttgtggaaccttagacaaaaaaggccagccatactccattctcttaaatttaaccgggaacgaattacttactgtcatctacctttccagagtaaatggctttatgttggaacagaaagaggaaatacacatattgtaaatattgaatctttcattctttctggatatgttatcatgtggaacaaggcaattgaactatccactaagactcatccaggtccagttgtacatttaagcgatagcccaagagatgaaggcaaactgctaataggttatgaaaatggtactgtagtattctgggacttgaaatctaaaagagcagaactgagagtttattatgatgaggctattcattcaattgattggcatcatgagggcaaacagttcatgtgcagccattcagatggtagtttgactttatggaacctgaaaagcccaagtcgccctttccagaccacaattccacatggaaaaagtcaaagagaaggaagaaaatctgaatcttgtaaaccaattcttaaagtagaatacaagacctgcaaaaacagcgaaccattcataatattctctggtgggctgtcctatgacaaagcttgtagaagaccaagtttaaccatcatgcatggaaaagcaattacagtacttgaaatggatcatcctattgttgaatttctaactttatgtgaaacgccctatccaaatgaatttcaagaaccctatgctgtcgtggtacttctggagaaagatctcattgtagttgatctgacacaaagcaattttccaatctttgaaaatccatatcccatggacattcatgaatcaccagttacatgcacagcatactttgcagattgtcctccggatttgattctagtactgtattctataggagtcaagcataaaaaacaaggatacagtaataaggagtggccaatcagtggaggagcttggaaccttggagcacaaacatatccagaaattattattactggtcatgcagatggatcaataaaattttgggatgcttctgcaataactctgcagatgctgtacaagctaaaaacttcaaaagtgtttgaaaaacagaaggtaggagaaggaaaacaaacatgtgaaattgtagaggaagacccatttgccattcagatgatttactggtgtccagagagcagaatattctgtgtatcaggagtctctgcatatgtcataatttataaattcagcagacatgaaattacaacagaaatagtgtcattagaggtacgacttcagtatgatgttgaagatattattacccctgaaccagaaacaagtcctccgtttccagatctctcagcccagcttccttcttcaaggagtctttctgggagcactaacactgttgctagtgaaggagtaacaaaggacagtattccatgcctcaatgtgaagacacggccagtgcgaatgcctccaggatatcaagcagaacttgttattcaattggtgtgggtagatggtgaacctccacaacagattactagtcttgctgtaagctcagcatatggaatagttgcatttgggaactgcaatgggttggctgtggtggattttatacagaagacagtactgttaagcatggggaccattgacctatatagatcaagtgacttataccagcgacaaccacggtctcctcgaaaaaacaaacagttcattgcagacaacttttgcatgcgtggcctgtctaacttttatcctgatttaacgaaacggatccgtacttcctatcagagtttaactgaactgaatgacagtccagttcccctagaacttgagcgctgcaagtctcctacctcagaccatgtaaatggacactgcacaagtccaacttctcagagttgcagttctggaaaacgtctttctagtgccgatgtttcaaaagtaaatcgctggggtcctggaagaccaccatttcgaaaggcccagtcagcagcctgcatggagatttctttaccagttacaacagaagaaaaccgagaaaattcctataatcgttctagaagctctagtatctccagtattgacaaagattctaaagaagcaattacagcactatacttcatggactcctttgcacggaaaaatgactctaccatctctccttgtctgttcgttggaaccagtctgggaatggtgttaatcatctccttaaacctaccattagcagatgaacaaaggtttacagagccagtcatggtattgccaagtggtacattcctctcattgaaaggagctgtgctaacattctcctgtatggaccgaatgggtggattaatgcaaccgccatatgaagtttggagggatccaaacaacatagatgaaaatgaaaaatcttggagaaggaaagtggtaatgaactcatcttctgcatcccaagaaataggagatcatcagtatacaataatctgctcagaaaaacaagccaaagtcttctcactgccttctcagacttgcctttatgttcataacatcacggagacatcttttatactgcaagcaaatgtggtggtcatgtgtagcagtgcctgcttggcatgcttttgtgctaacggacatatcatgataatgagcctacctagtcttcgcccaatgttggatgttaattatttgccactgacagacatgaggatagcacgaacattttgttttaccaatgaaggacaggcattatacctcgtctctcctactgaaattcagcggttaacatacagccaagaaatgtgtgataatctacaggacatgctaggagatttgtttactcccatagagacaccagaagctcaaaacagaggctttctcaagggactgtttggtggaagcggacaaacatttgacagagaagagctctttggggaagcttcggcaggaaaagcatcccgcagccttgcgcaacacattcctggaccaggtagtatagaagggatgaaaggcgctgctggaggggtgatgggagagctgacccgtgcacggattgcacttgatgaaagaggacagaggctaggagagctggaagagaaaactgcaggcatgatgaccagtgcagaagcattttccaaacatgcacatgagttaatgctgaaatacaaggataagaaatggtaccaattctgacttctaaagaagctgtgactgctttgagaaaccatattcagggaaaccaaatttattcccagcatcactactcaactgctagaagccagtttcttctacaaaatgttccatttacagtcaatctgaaattttcataaaagagatgtatcagagacactgtgcaacccaaaggctggagccctggttaaaatcccaaaatacggctgaatttgccttttcccatgtggaatggagctatcatcttggcatgtcattcgataaggatttatatttagtaactacggggagtcctcttgatttgaaaattcctgtacaaacaaaagcattaatgcacttaatgaaaaaaaatctttgcatgataaattaacatcttaaggggaaaagaaaaaaaagcatgttgtgatagaagaaaaaaagattcatggtaaactatttctatcaattgggccacactcaacaatttaaaaaatctgcatttgaagatgtcagtgcatttcaaatatatttgccatacccaactgaaacggaaaacaaaacaaaacaagaacccagagttttctcctcatctgtaactttcattgtactagaaccttattgaattcttatggcaagagtctgattaatgttctctctccatgttttacatcattcacagttgtgtcaaaatcaaatattgccagtatagtaaattattcccaacacaatcagtttcatttctatcaccttcagaatgggttgctgtttttagcacaaaccatgcagggttgggtcacctcaaagcattttcttcagcctggcttgtactctataggggagttggtagtaggtgtggggaatctataggaacaatagagttagctatgagaactgacttcacaaaaagggaaatttcacacaccccaatttcagcttctaaagtgatatattttaaaagcttcatttgtatccttgtctgccagttacacagtatattactgttcaaacccagtagggtctgcaatcgaaaggtgctcttgcagcctgacattcacaaaccaaactggtcattctctttagtgtgattcagtaaaatctcagttaatgttttgggaaagggattctgatttatgacatttctgatttacaagggctttccttagaaaatacctttcggtttgatacttaccactggaaattggttcgatacttaccactggaaatctttataaaatatagtgatctgtttgctatcttggtctcagtcatcattatagacaatagaaatacataaagagtttaatgatacaaaatcaatgcttttgtccctaggtcaaataatataagccactagattatgtcaatagatgccaaacacttgtcccttattaaagactcttttaaagctggaataaagaatatccttaacatgatacaaggtatctataactcaccagaaaagcaccagagtcaaaaccaaatagagacacctactaccatttaacatgattctggaagtcaaaagttataggaatgtatatatacacattccaggacccatcctgtaatatgttgtttcgtcaagaaaagttttaattatggttttggcttattgaatttttgtttatcaaggtctcattggatttacatttgtgtttcttaagacttcacaattttcctggatttcaggttattttattagccaaaaaatcgtatttttatttcctttttagtctaattttttgctagaagttgtactttctagcaaatgtttctagtggtacaatgttctcagtaattttgaggagaacaaagatgagtgaaagagttagataatgtacactaggatagcatttctcagagtccttgaatcctcttgttaagaaagcctctctgaatctcccagactcctgtgaacagccttacggtaacagaatctggcttggaaacacagacattacatgactgtataatttatagaattataaaattatatggtaaaaatattaaagaaacttaagagtaggatctagaaaatactagtggccaaattgcaatgtattctttgtaccatctgtttcaaagacttagttttctgattttcagaacaaatactttatcgtttctgtattttaaaaaaaactaaaagagtaaaatattagtttattttagaaataatgaaattcagtccaaagtagcagtacatttgatgagtatttctgaagccttcaataagatttaacttgttttaacttgatctacatcgagatttctcaaaagcagcactattagctgaaagtctttgttgtggggaactgtcctgtgtattgtaggatgttagcaacatccctggcctctgtctactagatgccagtaagaacctcctagtaatgacaatcaaaatgtctccagtcattgccaaaatttctcccagttcacagccactattctacatcatacaaagaggtagattgtgtgaatatgtaatatatgttgttgtataaaactgtacaataagtatacaatgtcttagcaagataaattattatacccaaaattacatgtgtggttcatatgcaataagatacaattttgaagaaagcttataggaatcagtgaaaaataacaactacagaatattttaaggcacacagagaaaatatcaaaaaggacattatagcatttcactgtagaagtgcttaaaaccttggcctcagtgaatagatcaaaagtttataattagcacaccaattggaagtaaacaggtgcttctcaaatgcttgaaaagaaaaggctctttgaagtagttaaaacgtgtctttcaaaattgcttttataagcccttccttaacgtaagggtaacttcatctcacaaactcctggttagtggaatccaaattaatgaggttttactgtatcaaaattatttttataattcaaagagatgatagcaataagaagaatctaatgtggatgtgatttttctctttgaacaattctgttctgttgcactgaccttagcacgcacgcacacacacacacaccatcgccaccactaccatcatcatcttatcctcatctttggaaaataagtactgttgatccatgtaatcctttgcatagtctcatctttactatctttcttctatttcggaacataagaaaaatactcctaataacttggacaatgatacagaaagtgactctgagccttagttaccatcaaaattacattctatctgctaaagcgacatcagaagataaggcttgcaaaccacagtcccaacaagttgaccttgtctccctatgatttccttggaagataaggcctttttagtgttacagtagaaaatgggccttttcatttattcatctgtgagaagctagaggtatttgtttccctgataataacgtgagcaatagtccctaccttgaaatcatccattagtcttggagtttggagggaggaatgattgattcctcatttgttttaatcacctacaaaagcagtactactgactttgcttcttacacttcactgagccccagactttagggccccaatcattgtcaagatcattgtctaactggaactctgaaaggacagtgacagaactgaatgagatgttttccagtgattcagtcacaaagacaattttctcagatcttttgaaagtgattctcaaataaataaatcaaaatccaactcctttccctcaaagtttctagggatctgaaggaaaaggtttactgttggagtccctttttatgtgacccatgtaccagttttaaaggcatcatctatactttatctacatgaagggatcaccatgactttgagagaaaaaagaatcagattaggcctaacattggttgaagaagattaaaatagattcttatattcaagcagaagggaaaaatgaagccaatctagaaaagtaagctaaaaatcctctccttggcttaggatcattgggtcaaactgggagtatatctgtgtgattacaacctgctgctatgagaaaaaagaattgtaacttgaccatgttggctcacacagggcaatgcaaaagaagtcaaaacattcatatcaggtcttggtatctgtgtcaggagaaacgtggtggctttcacagcttcttcacctctgtcctctgtcatgcaactccatttttggctaggtactatttcacatgcacactgtcctgggtgccagaaatacttgtggtgtacttggtttgagcagtacctctagtatgcaccattccagggaacatggttgtcaacataacaagtttagtgtgtgtatttgcagacaacatagccctgaaagcatgaaatgtagaataggtaaggtctgtcttagaaaaggaggaggaagtaccaatttggtgcaagaagatcgtggtgaggaaggacatgggagccacagtgaagtgaaagaggctttaaggaatcagatgcacagatggatgctttgatttacacatttatctagaggagtgattctcaaccttgactgtacataagaatcacctcaggaaatttttaaattcccaattatattaaaatcatttggagtgggaaccagacaccaatatttgcgaaagcctccaaggcggttctaatgtccagccaaagttgattatcactgctttatggccaactaaggaaaccttgtttgtctgccttggctggtgctccagccccagttctgagtggtcagggaaggcaagatgtaagatatagtaatggtatttattctgtatgtctcacagaacaaaagcatttgagaatttctgaccaggcagtgctccatcaactcttaataatcatctttgtgatattctcctatgtgacttgtccatcaattattccaattcaaaggtctaggttttttttcaattgtcttacacatgtgacatcacaagataccagaagtagcacagtaaattcaagagcatataaagctaagtggaaaactaattcttcatatttagacagtggaaattctcaaaacaatcatttgctaaattaggtccaaatttattattcattcttcttctggaggagacatgggtaccaggtacctgttctgctgtaggtatatttcactggacttggtcttagcaaaaaggaagaacaaatcttcctttttgattgttatctcaatcaaaagctcccagggccacttggatttattttcttagtctttggacatgtgtttaaaggaaaagaatacctgtaacttcctatatgacatccagtgccctgaaagggtgcttacaccttcaaaaaaggagagtccagcctatcaaaggcagtaacacataatgagaagaaactcagagttattgcctttcatactgctttccctctgctgttggcccacccttcttgactgcaaagccagaaaataaactagatggtggttttggacaattgtacacaggaacagaatctctaataacctataatttttagtacttaattatgtgatgttttattctaggaaataagaaacagatgacatcattgatgtatctttctttcatcttcagaatttttgcatcttttcagaaaatgacaaattactatttttctgttgcactcagcaattgtgactatacttaacaaaattcttgtagtctgtagagatatcaataaaattgtatatgtttgtacataaaaaaaaaaaaaaaaaa

SEQ ID NO: 33 - RNA, 9310 nt, Homo sapiens
  source 1..9310: mol_type = mRNA
ctgactgctcggttaggacctcggagagcgccaggcgccgcgaccagagggcccagagaagcggccggagcccgcctacctcggccccctcagcttcccgggctggcaggcggctagaggcgtctgaggaagtgtttaaaatgaagaagtttaatttccgaaaagttttggatggcttaactgcctcctcccctggcagtggtagcagcagtggcagtaacagtggtggtggggctggaagtggttccgtacatccggcggggactgcaggggttctcagagaggaaattcaggaaactttgacttcggagtatttccagatttgcaagacagttcggcatggttttcctcatcagcccacagcattagcctttgatccagttcagaaaatcttggctattgggacgagaacaggtgctatacgaatactcgggagacctggtgttgattgctattgccaacatgaaagtggtgcagctgtcctacagctccaatttttgatcaatgagggtgccttggtcagtgcaagttcagatgatacacttcatttgtggaaccttagacaaaaaaggccagccatactccattctcttaaatttaaccgggaacgaattacttactgtcatctacctttccagagtaaatggctttatgttggaacagaaagaggaaatacacatattgtaaatattgaatctttcattctttctggatatgttatcatgtggaacaaggcaattgaactatccactaagactcatccaggtccagttgtacatttaagcgatagcccaagagatgaaggcaaactgctaataggttatgaaaatggtactgtagtattctgggacttgaaatctaaaagagcagaactgagagtttattatgatgaggctattcattcaattgattggcatcatgagggcaaacagttcatgtgcagccattcagatggtagtttgactttatggaacctgaaaagcccaagtcgccctttccagaccacaattccacatggaaaaagtcaaagagaaggaagaaaatctgaatcttgtaaaccaattcttaaagtagaatacaagacctgcaaaaacagcgaaccattcataatattctctggtgggctgtcctatgacaaagcttgtagaagaccaagtttaaccatcatgcatggaaaagcaattacagtacttgaaatggatcatcctattgttgaatttctaactttatgtgaaacgccctatccaaatgaatttcaagaaccctatgctgtcgtggtacttctggagaaagatctcattgtagttgatctgacacaaagcaattttccaatctttgaaaatccatatcccatggacattcatgaatcaccagttacatgcacagcatactttgcagattgtcctccggatttgattctagtactgtattctataggagtcaagcataaaaaacaaggatacagtaataaggagtggccaatcagtggaggagcttggaaccttggagcacaaacatatccagaaattattattactggtcatgcagatggatcaataaaattttgggatgcttctgcaataactctgcagatgctgtacaagctaaaaacttcaaaagtgtttgaaaaacagaaggtaggagaaggaaaacaaacatgtgaaattgtagaggaagacccatttgccattcagatgatttactggtgtccagagagcagaatattctgtgtatcaggagtctctgcatatgtcataatttataaattcagcagacatgaaattacaacagaaatagtgtcattagaggtacgacttcagtatgatgttgaagatattattacccctgaaccagaaacaagtcctccgtttccagatctctcagcccagcttccttcttcaaggagtctttctgggagcactaacactgttgctagtgaaggagtaacaaaggacagtattccatgcctcaatgtgaagacacggccagtgcgaatgcctccaggatatcaagcagaacttgttattcaattggtgtgggtagatggtgaacctccacaacagattactagtcttgctgtaagctcagcatatggaatagttgcatttgggaactgcaatgggttggctgtggtggattttatacagaagacagtactgttaagcatggggaccattgacctatatagatcaagtgacttataccagcgacaaccacggtctcctcgaaaaaacaaacagttcattgcaggtttaactgaactgaatgacagtccagttcccctagaacttgagcgctgcaagtctcctacctcagaccatgtaaatggacactgcacaagtccaacttctcagagttgcagttctggaaaacgtctttctagtgccgatgtttcaaaagtaaatcgctggggtcctggaagaccaccatttcgaaaggcccagtcagcagcctgcatggagatttctttaccagttacaacagaagaaaaccgagaaaattcctataatcgttctagaagctctagtatctccagtattgacaaagattctaaagaagcaattacagcactatacttcatggactcctttgcacggaaaaatgactctaccatctctccttgtctgttcgttggaaccagtctgggaatggtgttaatcatctccttaaacctaccattagcagatgaacaaaggtttacagagccagtcatggtattgccaagtggtacattcctctcattgaaaggagctgtgctaacattctcctgtatggaccgaatgggtggattaatgcaaccgccatatgaagtttggagggatccaaacaacatagatgaaaatgaaaaatcttggagaaggaaagtggtaatgaactcatcttctgcatcccaagaaataggagatcatcagtatacaataatctgctcagaaaaacaagccaaagtcttctcactgccttctcagacttgcctttatgttcataacatcacggagacatcttttatactgcaagcaaatgtggtggtcatgtgtagcagtgcctgcttggcatgcttttgtgctaacggacatatcatgataatgagcctacctagtcttcgcccaatgttggatgttaattatttgccactgacagacatgaggatagcacgaacattttgttttaccaatgaaggacaggcattatacctcgtctctcctactgaaattcagcggttaacatacagccaagaaatgtgtgataatctacaggacatgctaggagatttgtttactcccatagagacaccagaagctcaaaacagaggctttctcaagggactgtttggtggaagcggacaaacatttgacagagaagagctctttggggaagcttcggcaggaaaagcatcccgcagccttgcgcaacacattcctggaccaggtagtatagaagggatgaaaggcgctgctggaggggtgatgggagagctgacccgtgcacggattgcacttgatgaaagaggacagaggctaggagagctggaagagaaaactgcaggcatgatgaccagtgcagaagcattttccaaacatgcacatgagttaatgctgaaatacaaggataagaaatggtaccaattctgacttctaaagaagctgtgactgctttgagaaaccatattcagggaaaccaaatttattcccagcatcactactcaactgctagaagccagtttcttctacaaaatgttccatttacagtcaatctgaaattttcataaaagagatgtatcagagacactgtgcaacccaaaggctggagccctggttaaaatcccaaaatacggctgaatttgccttttcccatgtggaatggagctatcatcttggcatgtcattcgataaggatttatatttagtaactacggggagtcctcttgatttgaaaattcctgtacaaacaaaagcattaatgcacttaatgaaaaaaaatctttgcatgataaattaacatcttaaggggaaaagaaaaaaaagcatgttgtgatagaagaaaaaaagattcatggtaaactatttctatcaattgggccacactcaacaatttaaaaaatctgcatttgaagatgtcagtgcatttcaaatatatttgccatacccaactgaaacggaaaacaaaacaaaacaagaacccagagttttctcctcatctgtaactttcattgtactagaaccttattgaattcttatggcaagagtctgattaatgttctctctccatgttttacatcattcacagttgtgtcaaaatcaaatattgccagtatagtaaattattcccaacacaatcagtttcatttctatcaccttcagaatgggttgctgtttttagcacaaaccatgcagggttgggtcacctcaaagcattttcttcagcctggcttgtactctataggggagttggtagtaggtgtggggaatctataggaacaatagagttagctatgagaactgacttcacaaaaagggaaatttcacacaccccaatttcagcttctaaagtgatatattttaaaagcttcatttgtatccttgtctgccagttacacagtatattactgttcaaacccagtagggtctgcaatcgaaaggtgctcttgcagcctgacattcacaaaccaaactggtcattctctttagtgtgattcagtaaaatctcagttaatgttttgggaaagggattctgatttatgacatttctgatttacaagggctttccttagaaaatacctttcggtttgatacttaccactggaaattggttcgatacttaccactggaaatctttataaaatatagtgatctgtttgctatcttggtctcagtcatcattatagacaatagaaatacataaagagtttaatgatacaaaatcaatgcttttgtccctaggtcaaataatataagccactagattatgtcaatagatgccaaacacttgtcccttattaaagactcttttaaagctggaataaagaatatccttaacatgatacaaggtatctataactcaccagaaaagcaccagagtcaaaaccaaatagagacacctactaccatttaacatgattctggaagtcaaaagttataggaatgtatatatacacattccaggacccatcctgtaatatgttgtttcgtcaagaaaagttttaattatggttttggcttattgaatttttgtttatcaaggtctcattggatttacatttgtgtttcttaagacttcacaattttcctggatttcaggttattttattagccaaaaaatcgtatttttatttcctttttagtctaattttttgctagaagttgtactttctagcaaatgtttctagtggtacaatgttctcagtaattttgaggagaacaaagatgagtgaaagagttagataatgtacactaggatagcatttctcagagtccttgaatcctcttgttaagaaagcctctctgaatctcccagactcctgtgaacagccttacggtaacagaatctggcttggaaacacagacattacatgactgtataatttatagaattataaaattatatggtaaaaatattaaagaaacttaagagtaggatctagaaaatactagtggccaaattgcaatgtattctttgtaccatctgtttcaaagacttagttttctgattttcagaacaaatactttatcgtttctgtattttaaaaaaaactaaaagagtaaaatattagtttattttagaaataatgaaattcagtccaaagtagcagtacatttgatgagtatttctgaagccttcaataagatttaacttgttttaacttgatctacatcgagatttctcaaaagcagcactattagctgaaagtctttgttgtggggaactgtcctgtgtattgtaggatgttagcaacatccctggcctctgtctactagatgccagtaagaacctcctagtaatgacaatcaaaatgtctccagtcattgccaaaatttctcccagttcacagccactattctacatcatacaaagaggtagattgtgtgaatatgtaatatatgttgttgtataaaactgtacaataagtatacaatgtcttagcaagataaattattatacccaaaattacatgtgtggttcatatgcaataagatacaattttgaagaaagcttataggaatcagtgaaaaataacaactacagaatattttaaggcacacagagaaaatatcaaaaaggacattatagcatttcactgtagaagtgcttaaaaccttggcctcagtgaatagatcaaaagtttataattagcacaccaattggaagtaaacaggtgcttctcaaatgcttgaaaagaaaaggctctttgaagtagttaaaacgtgtctttcaaaattgcttttataagcccttccttaacgtaagggtaacttcatctcacaaactcctggttagtggaatccaaattaatgaggttttactgtatcaaaattatttttataattcaaagagatgatagcaataagaagaatctaatgtggatgtgatttttctctttgaacaattctgttctgttgcactgaccttagcacgcacgcacacacacacacaccatcgccaccactaccatcatcatcttatcctcatctttggaaaataagtactgttgatccatgtaatcctttgcatagtctcatctttactatctttcttctatttcggaacataagaaaaatactcctaataacttggacaatgatacagaaagtgactctgagccttagttaccatcaaaattacattctatctgctaaagcgacatcagaagataaggcttgcaaaccacagtcccaacaagttgaccttgtctccctatgatttccttggaagataaggcctttttagtgttacagtagaaaatgggccttttcatttattcatctgtgagaagctagaggtatttgtttccctgataataacgtgagcaatagtccctaccttgaaatcatccattagtcttggagtttggagggaggaatgattgattcctcatttgttttaatcacctacaaaagcagtactactgactttgcttcttacacttcactgagccccagactttagggccccaatcattgtcaagatcattgtctaactggaactctgaaaggacagtgacagaactgaatgagatgttttccagtgattcagtcacaaagacaattttctcagatcttttgaaagtgattctcaaataaataaatcaaaatccaactcctttccctcaaagtttctagggatctgaaggaaaaggtttactgttggagtccctttttatgtgacccatgtaccagttttaaaggcatcatctatactttatctacatgaagggatcaccatgactttgagagaaaaaagaatcagattaggcctaacattggttgaagaagattaaaatagattcttatattcaagcagaagggaaaaatgaagccaatctagaaaagtaagctaaaaatcctctccttggcttaggatcattgggtcaaactgggagtatatctgtgtgattacaacctgctgctatgagaaaaaagaattgtaacttgaccatgttggctcacacagggcaatgcaaaagaagtcaaaacattcatatcaggtcttggtatctgtgtcaggagaaacgtggtggctttcacagcttcttcacctctgtcctctgtcatgcaactccatttttggctaggtactatttcacatgcacactgtcctgggtgccagaaatacttgtggtgtacttggtttgagcagtacctctagtatgcaccattccagggaacatggttgtcaacataacaagtttagtgtgtgtatttgcagacaacatagccctgaaagcatgaaatgtagaataggtaaggtctgtcttagaaaaggaggaggaagtaccaatttggtgcaagaagatcgtggtgaggaaggacatgggagccacagtgaagtgaaagaggctttaaggaatcagatgcacagatggatgctttgatttacacatttatctagaggagtgattctcaaccttgactgtacataagaatcacctcaggaaatttttaaattcccaattatattaaaatcatttggagtgggaaccagacaccaatatttgcgaaagcctccaaggcggttctaatgtccagccaaagttgattatcactgctttatggccaactaaggaaaccttgtttgtctgccttggctggtgctccagccccagttctgagtggtcagggaaggcaagatgtaagatatagtaatggtatttattctgtatgtctcacagaacaaaagcatttgagaatttctgaccaggcagtgctccatcaactcttaataatcatctttgtgatattctcctatgtgacttgtccatcaattattccaattcaaaggtctaggttttttttcaattgtcttacacatgtgacatcacaagataccagaagtagcacagtaaattcaagagcatataaagctaagtggaaaactaattcttcatatttagacagtggaaattctcaaaacaatcatttgctaaattaggtccaaatttattattcattcttcttctggaggagacatgggtaccaggtacctgttctgctgtaggtatatttcactggacttggtcttagcaaaaaggaagaacaaatcttcctttttgattgttatctcaatcaaaagctcccagggccacttggatttattttcttagtctttggacatgtgtttaaaggaaaagaatacctgtaacttcctatatgacatccagtgccctgaaagggtgcttacaccttcaaaaaaggagagtccagcctatcaaaggcagtaacacataatgagaagaaactcagagttattgcctttcatactgctttccctctgctgttggcccacccttcttgactgcaaagccagaaaataaactagatggtggttttggacaattgtacacaggaacagaatctctaataacctataatttttagtacttaattatgtgatgttttattctaggaaataagaaacagatgacatcattgatgtatctttctttcatcttcagaatttttgcatcttttcagaaaatgacaaattactatttttctgttgcactcagcaattgtgactatacttaacaaaattcttgtagtctgtagagatatcaataaaattgtatatgtttgtacataaaaaaaaaaaaaaaaaa

SEQ ID NO: 34 - RNA, 9302 nt, Homo sapiens
  source 1..9302: mol_type = mRNA
gtgcagcggggagagcggacggcgggcgggcgaacaggcgggagagcgcggcggcggctgcgggcagagtgtttaaaatgaagaagtttaatttccgaaaagttttggatggcttaactgcctcctcccctggcagtggtagcagcagtggcagtaacagtggtggtggggctggaagtggttccgtacatccggcggggactgcaggggttctcagagaggaaattcaggaaactttgacttcggagtatttccagatttgcaagacagttcggcatggttttcctcatcagcccacagcattagcctttgatccagttcagaaaatcttggctattgggacgagaacaggtgctatacgaatactcgggagacctggtgttgattgctattgccaacatgaaagtggtgcagctgtcctacagctccaatttttgatcaatgagggtgccttggtcagtgcaagttcagatgatacacttcatttgtggaaccttagacaaaaaaggccagccatactccattctcttaaatttaaccgggaacgaattacttactgtcatctacctttccagagtaaatggctttatgttggaacagaaagaggaaatacacatattgtaaatattgaatctttcattctttctggatatgttatcatgtggaacaaggcaattgaactatccactaagactcatccaggtccagttgtacatttaagcgatagcccaagagatgaaggcaaactgctaataggttatgaaaatggtactgtagtattctgggacttgaaatctaaaagagcagaactgagagtttattatgatgaggctattcattcaattgattggcatcatgagggcaaacagttcatgtgcagccattcagatggtagtttgactttatggaacctgaaaagcccaagtcgccctttccagaccacaattccacatggaaaaagtcaaagagaaggaagaaaatctgaatcttgtaaaccaattcttaaagtagaatacaagacctgcaaaaacagcgaaccattcataatattctctggtgggctgtcctatgacaaagcttgtagaagaccaagtttaaccatcatgcatggaaaagcaattacagtacttgaaatggatcatcctattgttgaatttctaactttatgtgaaacgccctatccaaatgaatttcaagaaccctatgctgtcgtggtacttctggagaaagatctcattgtagttgatctgacacaaagcaattttccaatctttgaaaatccatatcccatggacattcatgaatcaccagttacatgcacagcatactttgcagattgtcctccggatttgattctagtactgtattctataggagtcaagcataaaaaacaaggatacagtaataaggagtggccaatcagtggaggagcttggaaccttggagcacaaacatatccagaaattattattactggtcatgcagatggatcaataaaattttgggatgcttctgcaataactctgcagatgctgtacaagctaaaaacttcaaaagtgtttgaaaaacagaaggtaggagaaggaaaacaaacatgtgaaattgtagaggaagacccatttgccattcagatgatttactggtgtccagagagcagaatattctgtgtatcaggagtctctgcatatgtcataatttataaattcagcagacatgaaattacaacagaaatagtgtcattagaggtacgacttcagtatgatgttgaagatattattacccctgaaccagaaacaagtcctccgtttccagatctctcagcccagcttccttcttcaaggagtctttctgggagcactaacactgttgctagtgaaggagtaacaaaggacagtattccatgcctcaatgtgaagacacggccagtgcgaatgcctccaggatatcaagcagaacttgttattcaattggtgtgggtagatggtgaacctccacaacagattactagtcttgctgtaagctcagcatatggaatagttgcatttgggaactgcaatgggttggctgtggtggattttatacagaagacagtactgttaagcatggggaccattgacctatatagatcaagtgacttataccagcgacaaccacggtctcctcgaaaaaacaaacagttcattgcagacaacttttgcatgcgtggcctgtctaacttttatcctgatttaacgaaacggatccgtacttcctatcagagtttaactgaactgaatgacagtccagttcccctagaacttgagcgctgcaagtctcctacctcagaccatgtaaatggacactgcacaagtccaacttctcagagttgcagttctggaaaacgtctttctagtgccgatgtttcaaaagtaaatcgctggggtcctggaagaccaccatttcgaaaggcccagtcagcagcctgcatggagatttctttaccagttacaacagaagaaaaccgagaaaattcctataatcgttctagaagctctagtatctccagtattgacaaagattctaaagaagcaattacagcactatacttcatggactcctttgcacggaaaaatgactctaccatctctccttgtctgttcgttggaaccagtctgggaatggtgttaatcatctccttaaacctaccattagcagatgaacaaaggtttacagagccagtcatggtattgccaagtggtacattcctctcattgaaaggagctgtgctaacattctcctgtatggaccgaatgggtggattaatgcaaccgccatatgaagtttggagggatccaaacaacatagatgaaaatgaaaaatcttggagaaggaaagtggtaatgaactcatcttctgcatcccaagaaataggagatcatcagtatacaataatctgctcagaaaaacaagccaaagtcttctcactgccttctcagacttgcctttatgttcataacatcacggagacatcttttatactgcaagcaaatgtggtggtcatgtgtagcagtgcctgcttggcatgcttttgtgctaacggacatatcatgataatgagcctacctagtcttcgcccaatgttggatgttaattatttgccactgacagacatgaggatagcacgaacattttgttttaccaatgaaggacaggcattatacctcgtctctcctactgaaattcagcggttaacatacagccaagaaatgtgtgataatctacaggacatgctaggagatttgtttactcccatagagacaccagaagctcaaaacagaggctttctcaagggactgtttggtggaagcggacaaacatttgacagagaagagctctttggggaagcttcggcaggaaaagcatcccgcagccttgcgcaacacattcctggaccaggtagtatagaagggatgaaaggcgctgctggaggggtgatgggagagctgacccgtgcacggattgcacttgatgaaagaggacagaggctaggagagctggaagagaaaactgcaggcatgatgaccagtgcagaagcattttccaaacatgcacatgagttaatgctgaaatacaaggataagaaatggtaccaattctgacttctaaagaagctgtgactgctttgagaaaccatattcagggaaaccaaatttattcccagcatcactactcaactgctagaagccagtttcttctacaaaatgttccatttacagtcaatctgaaattttcataaaagagatgtatcagagacactgtgcaacccaaaggctggagccctggttaaaatcccaaaatacggctgaatttgccttttcccatgtggaatggagctatcatcttggcatgtcattcgataaggatttatatttagtaactacggggagtcctcttgatttgaaaattcctgtacaaacaaaagcattaatgcacttaatgaaaaaaaatctttgcatgataaattaacatcttaaggggaaaagaaaaaaaagcatgttgtgatagaagaaaaaaagattcatggtaaactatttctatcaattgggccacactcaacaatttaaaaaatctgcatttgaagatgtcagtgcatttcaaatatatttgccatacccaactgaaacggaaaacaaaacaaaacaagaacccagagttttctcctcatctgtaactttcattgtactagaaccttattgaattcttatggcaagagtctgattaatgttctctctccatgttttacatcattcacagttgtgtcaaaatcaaatattgccagtatagtaaattattcccaacacaatcagtttcatttctatcaccttcagaatgggttgctgtttttagcacaaaccatgcagggttgggtcacctcaaagcattttcttcagcctggcttgtactctataggggagttggtagtaggtgtggggaatctataggaacaatagagttagctatgagaactgacttcacaaaaagggaaatttcacacaccccaatttcagcttctaaagtgatatattttaaaagcttcatttgtatccttgtctgccagttacacagtatattactgttcaaacccagtagggtctgcaatcgaaaggtgctcttgcagcctgacattcacaaaccaaactggtcattctctttagtgtgattcagtaaaatctcagttaatgttttgggaaagggattctgatttatgacatttctgatttacaagggctttccttagaaaatacctttcggtttgatacttaccactggaaattggttcgatacttaccactggaaatctttataaaatatagtgatctgtttgctatcttggtctcagtcatcattatagacaatagaaatacataaagagtttaatgatacaaaatcaatgcttttgtccctaggtcaaataatataagccactagattatgtcaatagatgccaaacacttgtcccttattaaagactcttttaaagctggaataaagaatatccttaacatgatacaaggtatctataactcaccagaaaagcaccagagtcaaaaccaaatagagacacctactaccatttaacatgattctggaagtcaaaagttataggaatgtatatatacacattccaggacccatcctgtaatatgttgtttcgtcaagaaaagttttaattatggttttggcttattgaatttttgtttatcaaggtctcattggatttacatttgtgtttcttaagacttcacaattttcctggatttcaggttattttattagccaaaaaatcgtatttttatttcctttttagtctaattttttgctagaagttgtactttctagcaaatgtttctagtggtacaatgttctcagtaattttgaggagaacaaagatgagtgaaagagttagataatgtacactaggatagcatttctcagagtccttgaatcctcttgttaagaaagcctctctgaatctcccagactcctgtgaacagccttacggtaacagaatctggcttggaaacacagacattacatgactgtataatttatagaattataaaattatatggtaaaaatattaaagaaacttaagagtaggatctagaaaatactagtggccaaattgcaatgtattctttgtaccatctgtttcaaagacttagttttctgattttcagaacaaatactttatcgtttctgtattttaaaaaaaactaaaagagtaaaatattagtttattttagaaataatgaaattcagtccaaagtagcagtacatttgatgagtatttctgaagccttcaataagatttaacttgttttaacttgatctacatcgagatttctcaaaagcagcactattagctgaaagtctttgttgtggggaactgtcctgtgtattgtaggatgttagcaacatccctggcctctgtctactagatgccagtaagaacctcctagtaatgacaatcaaaatgtctccagtcattgccaaaatttctcccagttcacagccactattctacatcatacaaagaggtagattgtgtgaatatgtaatatatgttgttgtataaaactgtacaataagtatacaatgtcttagcaagataaattattatacccaaaattacatgtgtggttcatatgcaataagatacaattttgaagaaagcttataggaatcagtgaaaaataacaactacagaatattttaaggcacacagagaaaatatcaaaaaggacattatagcatttcactgtagaagtgcttaaaaccttggcctcagtgaatagatcaaaagtttataattagcacaccaattggaagtaaacaggtgcttctcaaatgcttgaaaagaaaaggctctttgaagtagttaaaacgtgtctttcaaaattgcttttataagcccttccttaacgtaagggtaacttcatctcacaaactcctggttagtggaatccaaattaatgaggttttactgtatcaaaattatttttataattcaaagagatgatagcaataagaagaatctaatgtggatgtgatttttctctttgaacaattctgttctgttgcactgaccttagcacgcacgcacacacacacacaccatcgccaccactaccatcatcatcttatcctcatctttggaaaataagtactgttgatccatgtaatcctttgcatagtctcatctttactatctttcttctatttcggaacataagaaaaatactcctaataacttggacaatgatacagaaagtgactctgagccttagttaccatcaaaattacattctatctgctaaagcgacatcagaagataaggcttgcaaaccacagtcccaacaagttgaccttgtctccctatgatttccttggaagataaggcctttttagtgttacagtagaaaatgggccttttcatttattcatctgtgagaagctagaggtatttgtttccctgataataacgtgagcaatagtccctaccttgaaatcatccattagtcttggagtttggagggaggaatgattgattcctcatttgttttaatcacctacaaaagcagtactactgactttgcttcttacacttcactgagccccagactttagggccccaatcattgtcaagatcattgtctaactggaactctgaaaggacagtgacagaactgaatgagatgttttccagtgattcagtcacaaagacaattttctcagatcttttgaaagtgattctcaaataaataaatcaaaatccaactcctttccctcaaagtttctagggatctgaaggaaaaggtttactgttggagtccctttttatgtgacccatgtaccagttttaaaggcatcatctatactttatctacatgaagggatcaccatgactttgagagaaaaaagaatcagattaggcctaacattggttgaagaagattaaaatagattcttatattcaagcagaagggaaaaatgaagccaatctagaaaagtaagctaaaaatcctctccttggcttaggatcattgggtcaaactgggagtatatctgtgtgattacaacctgctgctatgagaaaaaagaattgtaacttgaccatgttggctcacacagggcaatgcaaaagaagtcaaaacattcatatcaggtcttggtatctgtgtcaggagaaacgtggtggctttcacagcttcttcacctctgtcctctgtcatgcaactccatttttggctaggtactatttcacatgcacactgtcctgggtgccagaaatacttgtggtgtacttggtttgagcagtacctctagtatgcaccattccagggaacatggttgtcaacataacaagtttagtgtgtgtatttgcagacaacatagccctgaaagcatgaaatgtagaataggtaaggtctgtcttagaaaaggaggaggaagtaccaatttggtgcaagaagatcgtggtgaggaaggacatgggagccacagtgaagtgaaagaggctttaaggaatcagatgcacagatggatgctttgatttacacatttatctagaggagtgattctcaaccttgactgtacataagaatcacctcaggaaatttttaaattcccaattatattaaaatcatttggagtgggaaccagacaccaatatttgcgaaagcctccaaggcggttctaatgtccagccaaagttgattatcactgctttatggccaactaaggaaaccttgtttgtctgccttggctggtgctccagccccagttctgagtggtcagggaaggcaagatgtaagatatagtaatggtatttattctgtatgtctcacagaacaaaagcatttgagaatttctgaccaggcagtgctccatcaactcttaataatcatctttgtgatattctcctatgtgacttgtccatcaattattccaattcaaaggtctaggttttttttcaattgtcttacacatgtgacatcacaagataccagaagtagcacagtaaattcaagagcatataaagctaagtggaaaactaattcttcatatttagacagtggaaattctcaaaacaatcatttgctaaattaggtccaaatttattattcattcttcttctggaggagacatgggtaccaggtacctgttctgctgtaggtatatttcactggacttggtcttagcaaaaaggaagaacaaatcttcctttttgattgttatctcaatcaaaagctcccagggccacttggatttattttcttagtctttggacatgtgtttaaaggaaaagaatacctgtaacttcctatatgacatccagtgccctgaaagggtgcttacaccttcaaaaaaggagagtccagcctatcaaaggcagtaacacataatgagaagaaactcagagttattgcctttcatactgctttccctctgctgttggcccacccttcttgactgcaaagccagaaaataaactagatggtggttttggacaattgtacacaggaacagaatctctaataacctataatttttagtacttaattatgtgatgttttattctaggaaataagaaacagatgacatcattgatgtatctttctttcatcttcagaatttttgcatcttttcagaaaatgacaaattactatttttctgttgcactcagcaattgtgactatacttaacaaaattcttgtagtctgtagagatatcaataaaattgtatatgtttgtacata

SEQ ID NO: 35 - RNA, 9230 nt, Homo sapiens
  source 1..9230: mol_type = mRNA
gtgcagcggggagagcggacggcgggcgggcgaacaggcgggagagcgcggcggcggctgcgggcagagtgtttaaaatgaagaagtttaatttccgaaaagttttggatggcttaactgcctcctcccctggcagtggtagcagcagtggcagtaacagtggtggtggggctggaagtggttccgtacatccggcggggactgcaggggttctcagagaggaaattcaggaaactttgacttcggagtatttccagatttgcaagacagttcggcatggttttcctcatcagcccacagcattagcctttgatccagttcagaaaatcttggctattgggacgagaacaggtgctatacgaatactcgggagacctggtgttgattgctattgccaacatgaaagtggtgcagctgtcctacagctccaatttttgatcaatgagggtgccttggtcagtgcaagttcagatgatacacttcatttgtggaaccttagacaaaaaaggccagccatactccattctcttaaatttaaccgggaacgaattacttactgtcatctacctttccagagtaaatggctttatgttggaacagaaagaggaaatacacatattgtaaatattgaatctttcattctttctggatatgttatcatgtggaacaaggcaattgaactatccactaagactcatccaggtccagttgtacatttaagcgatagcccaagagatgaaggcaaactgctaataggttatgaaaatggtactgtagtattctgggacttgaaatctaaaagagcagaactgagagtttattatgatgaggctattcattcaattgattggcatcatgagggcaaacagttcatgtgcagccattcagatggtagtttgactttatggaacctgaaaagcccaagtcgccctttccagaccacaattccacatggaaaaagtcaaagagaaggaagaaaatctgaatcttgtaaaccaattcttaaagtagaatacaagacctgcaaaaacagcgaaccattcataatattctctggtgggctgtcctatgacaaagcttgtagaagaccaagtttaaccatcatgcatggaaaagcaattacagtacttgaaatggatcatcctattgttgaatttctaactttatgtgaaacgccctatccaaatgaatttcaagaaccctatgctgtcgtggtacttctggagaaagatctcattgtagttgatctgacacaaagcaattttccaatctttgaaaatccatatcccatggacattcatgaatcaccagttacatgcacagcatactttgcagattgtcctccggatttgattctagtactgtattctataggagtcaagcataaaaaacaaggatacagtaataaggagtggccaatcagtggaggagcttggaaccttggagcacaaacatatccagaaattattattactggtcatgcagatggatcaataaaattttgggatgcttctgcaataactctgcagatgctgtacaagctaaaaacttcaaaagtgtttgaaaaacagaaggtaggagaaggaaaacaaacatgtgaaattgtagaggaagacccatttgccattcagatgatttactggtgtccagagagcagaatattctgtgtatcaggagtctctgcatatgtcataatttataaattcagcagacatgaaattacaacagaaatagtgtcattagaggtacgacttcagtatgatgttgaagatattattacccctgaaccagaaacaagtcctccgtttccagatctctcagcccagcttccttcttcaaggagtctttctgggagcactaacactgttgctagtgaaggagtaacaaaggacagtattccatgcctcaatgtgaagacacggccagtgcgaatgcctccaggatatcaagcagaacttgttattcaattggtgtgggtagatggtgaacctccacaacagattactagtcttgctgtaagctcagcatatggaatagttgcatttgggaactgcaatgggttggctgtggtggattttatacagaagacagtactgttaagcatggggaccattgacctatatagatcaagtgacttataccagcgacaaccacggtctcctcgaaaaaacaaacagttcattgcaggtttaactgaactgaatgacagtccagttcccctagaacttgagcgctgcaagtctcctacctcagaccatgtaaatggacactgcacaagtccaacttctcagagttgcagttctggaaaacgtctttctagtgccgatgtttcaaaagtaaatcgctggggtcctggaagaccaccatttcgaaaggcccagtcagcagcctgcatggagatttctttaccagttacaacagaagaaaaccgagaaaattcctataatcgttctagaagctctagtatctccagtattgacaaagattctaaagaagcaattacagcactatacttcatggactcctttgcacggaaaaatgactctaccatctctccttgtctgttcgttggaaccagtctgggaatggtgttaatcatctccttaaacctaccattagcagatgaacaaaggtttacagagccagtcatggtattgccaagtggtacattcctctcattgaaaggagctgtgctaacattctcctgtatggaccgaatgggtggattaatgcaaccgccatatgaagtttggagggatccaaacaacatagatgaaaatgaaaaatcttggagaaggaaagtggtaatgaactcatcttctgcatcccaagaaataggagatcatcagtatacaataatctgctcagaaaaacaagccaaagtcttctcactgccttctcagacttgcctttatgttcataacatcacggagacatcttttatactgcaagcaaatgtggtggtcatgtgtagcagtgcctgcttggcatgcttttgtgctaacggacatatcatgataatgagcctacctagtcttcgcccaatgttggatgttaattatttgccactgacagacatgaggatagcacgaacattttgttttaccaatgaaggacaggcattatacctcgtctctcctactgaaattcagcggttaacatacagccaagaaatgtgtgataatctacaggacatgctaggagatttgtttactcccatagagacaccagaagctcaaaacagaggctttctcaagggactgtttggtggaagcggacaaacatttgacagagaagagctctttggggaagcttcggcaggaaaagcatcccgcagccttgcgcaacacattcctggaccaggtagtatagaagggatgaaaggcgctgctggaggggtgatgggagagctgacccgtgcacggattgcacttgatgaaagaggacagaggctaggagagctggaagagaaaactgcaggcatgatgaccagtgcagaagcattttccaaacatgcacatgagttaatgctgaaatacaaggataagaaatggtaccaattctgacttctaaagaagctgtgactgctttgagaaaccatattcagggaaaccaaatttattcccagcatcactactcaactgctagaagccagtttcttctacaaaatgttccatttacagtcaatctgaaattttcataaaagagatgtatcagagacactgtgcaacccaaaggctggagccctggttaaaatcccaaaatacggctgaatttgccttttcccatgtggaatggagctatcatcttggcatgtcattcgataaggatttatatttagtaactacggggagtcctcttgatttgaaaattcctgtacaaacaaaagcattaatgcacttaatgaaaaaaaatctttgcatgataaattaacatcttaaggggaaaagaaaaaaaagcatgttgtgatagaagaaaaaaagattcatggtaaactatttctatcaattgggccacactcaacaatttaaaaaatctgcatttgaagatgtcagtgcatttcaaatatatttgccatacccaactgaaacggaaaacaaaacaaaacaagaacccagagttttctcctcatctgtaactttcattgtactagaaccttattgaattcttatggcaagagtctgattaatgttctctctccatgttttacatcattcacagttgtgtcaaaatcaaatattgccagtatagtaaattattcccaacacaatcagtttcatttctatcaccttcagaatgggttgctgtttttagcacaaaccatgcagggttgggtcacctcaaagcattttcttcagcctggcttgtactctataggggagttggtagtaggtgtggggaatctataggaacaatagagttagctatgagaactgacttcacaaaaagggaaatttcacacaccccaatttcagcttctaaagtgatatattttaaaagcttcatttgtatccttgtctgccagttacacagtatattactgttcaaacccagtagggtctgcaatcgaaaggtgctcttgcagcctgacattcacaaaccaaactggtcattctctttagtgtgattcagtaaaatctcagttaatgttttgggaaagggattctgatttatgacatttctgatttacaagggctttccttagaaaatacctttcggtttgatacttaccactggaaattggttcgatacttaccactggaaatctttataaaatatagtgatctgtttgctatcttggtctcagtcatcattatagacaatagaaatacataaagagtttaatgatacaaaatcaatgcttttgtccctaggtcaaataatataagccactagattatgtcaatagatgccaaacacttgtcccttattaaagactcttttaaagctggaataaagaatatccttaacatgatacaaggtatctataactcaccagaaaagcaccagagtcaaaaccaaatagagacacctactaccatttaacatgattctggaagtcaaaagttataggaatgtatatatacacattccaggacccatcctgtaatatgttgtttcgtcaagaaaagttttaattatggttttggcttattgaatttttgtttatcaaggtctcattggatttacatttgtgtttcttaagacttcacaattttcctggatttcaggttattttattagccaaaaaatcgtatttttatttcctttttagtctaattttttgctagaagttgtactttctagcaaatgtttctagtggtacaatgttctcagtaattttgaggagaacaaagatgagtgaaagagttagataatgtacactaggatagcatttctcagagtccttgaatcctcttgttaagaaagcctctctgaatctcccagactcctgtgaacagccttacggtaacagaatctggcttggaaacacagacattacatgactgtataatttatagaattataaaattatatggtaaaaatattaaagaaacttaagagtaggatctagaaaatactagtggccaaattgcaatgtattctttgtaccatctgtttcaaagacttagttttctgattttcagaacaaatactttatcgtttctgtattttaaaaaaaactaaaagagtaaaatattagtttattttagaaataatgaaattcagtccaaagtagcagtacatttgatgagtatttctgaagccttcaataagatttaacttgttttaacttgatctacatcgagatttctcaaaagcagcactattagctgaaagtctttgttgtggggaactgtcctgtgtattgtaggatgttagcaacatccctggcctctgtctactagatgccagtaagaacctcctagtaatgacaatcaaaatgtctccagtcattgccaaaatttctcccagttcacagccactattctacatcatacaaagaggtagattgtgtgaatatgtaatatatgttgttgtataaaactgtacaataagtatacaatgtcttagcaagataaattattatacccaaaattacatgtgtggttcatatgcaataagatacaattttgaagaaagcttataggaatcagtgaaaaataacaactacagaatattttaaggcacacagagaaaatatcaaaaaggacattatagcatttcactgtagaagtgcttaaaaccttggcctcagtgaatagatcaaaagtttataattagcacaccaattggaagtaaacaggtgcttctcaaatgcttgaaaagaaaaggctctttgaagtagttaaaacgtgtctttcaaaattgcttttataagcccttccttaacgtaagggtaacttcatctcacaaactcctggttagtggaatccaaattaatgaggttttactgtatcaaaattatttttataattcaaagagatgatagcaataagaagaatctaatgtggatgtgatttttctctttgaacaattctgttctgttgcactgaccttagcacgcacgcacacacacacacaccatcgccaccactaccatcatcatcttatcctcatctttggaaaataagtactgttgatccatgtaatcctttgcatagtctcatctttactatctttcttctatttcggaacataagaaaaatactcctaataacttggacaatgatacagaaagtgactctgagccttagttaccatcaaaattacattctatctgctaaagcgacatcagaagataaggcttgcaaaccacagtcccaacaagttgaccttgtctccctatgatttccttggaagataaggcctttttagtgttacagtagaaaatgggccttttcatttattcatctgtgagaagctagaggtatttgtttccctgataataacgtgagcaatagtccctaccttgaaatcatccattagtcttggagtttggagggaggaatgattgattcctcatttgttttaatcacctacaaaagcagtactactgactttgcttcttacacttcactgagccccagactttagggccccaatcattgtcaagatcattgtctaactggaactctgaaaggacagtgacagaactgaatgagatgttttccagtgattcagtcacaaagacaattttctcagatcttttgaaagtgattctcaaataaataaatcaaaatccaactcctttccctcaaagtttctagggatctgaaggaaaaggtttactgttggagtccctttttatgtgacccatgtaccagttttaaaggcatcatctatactttatctacatgaagggatcaccatgactttgagagaaaaaagaatcagattaggcctaacattggttgaagaagattaaaatagattcttatattcaagcagaagggaaaaatgaagccaatctagaaaagtaagctaaaaatcctctccttggcttaggatcattgggtcaaactgggagtatatctgtgtgattacaacctgctgctatgagaaaaaagaattgtaacttgaccatgttggctcacacagggcaatgcaaaagaagtcaaaacattcatatcaggtcttggtatctgtgtcaggagaaacgtggtggctttcacagcttcttcacctctgtcctctgtcatgcaactccatttttggctaggtactatttcacatgcacactgtcctgggtgccagaaatacttgtggtgtacttggtttgagcagtacctctagtatgcaccattccagggaacatggttgtcaacataacaagtttagtgtgtgtatttgcagacaacatagccctgaaagcatgaaatgtagaataggtaaggtctgtcttagaaaaggaggaggaagtaccaatttggtgcaagaagatcgtggtgaggaaggacatgggagccacagtgaagtgaaagaggctttaaggaatcagatgcacagatggatgctttgatttacacatttatctagaggagtgattctcaaccttgactgtacataagaatcacctcaggaaatttttaaattcccaattatattaaaatcatttggagtgggaaccagacaccaatatttgcgaaagcctccaaggcggttctaatgtccagccaaagttgattatcactgctttatggccaactaaggaaaccttgtttgtctgccttggctggtgctccagccccagttctgagtggtcagggaaggcaagatgtaagatatagtaatggtatttattctgtatgtctcacagaacaaaagcatttgagaatttctgaccaggcagtgctccatcaactcttaataatcatctttgtgatattctcctatgtgacttgtccatcaattattccaattcaaaggtctaggttttttttcaattgtcttacacatgtgacatcacaagataccagaagtagcacagtaaattcaagagcatataaagctaagtggaaaactaattcttcatatttagacagtggaaattctcaaaacaatcatttgctaaattaggtccaaatttattattcattcttcttctggaggagacatgggtaccaggtacctgttctgctgtaggtatatttcactggacttggtcttagcaaaaaggaagaacaaatcttcctttttgattgttatctcaatcaaaagctcccagggccacttggatttattttcttagtctttggacatgtgtttaaaggaaaagaatacctgtaacttcctatatgacatccagtgccctgaaagggtgcttacaccttcaaaaaaggagagtccagcctatcaaaggcagtaacacataatgagaagaaactcagagttattgcctttcatactgctttccctctgctgttggcccacccttcttgactgcaaagccagaaaataaactagatggtggttttggacaattgtacacaggaacagaatctctaataacctataatttttagtacttaattatgtgatgttttattctaggaaataagaaacagatgacatcattgatgtatctttctttcatcttcagaatttttgcatcttttcagaaaatgacaaattactatttttctgttgcactcagcaattgtgactatacttaacaaaattcttgtagtctgtagagatatcaataaaattgtatatgtttgtacata

SEQ ID NO: 36 - RNA, 9248 nt, Homo sapiens
  source 1..9248: mol_type = mRNA
ccaacgtcgtttttctgaaaataaaatactctgagccgaacgtttcgaagaaggaaagtccgcccttaagagagagacagagtcttgtgtttaaaatgaagaagtttaatttccgaaaagttttggatggcttaactgcctcctcccctggcagtggtagcagcagtggcagtaacagtggtggtggggctggaagtggttccgtacatccggcggggactgcaggggttctcagagaggaaattcaggaaactttgacttcggagtatttccagatttgcaagacagttcggcatggttttcctcatcagcccacagcattagcctttgatccagttcagaaaatcttggctattgggacgagaacaggtgctatacgaatactcgggagacctggtgttgattgctattgccaacatgaaagtggtgcagctgtcctacagctccaatttttgatcaatgagggtgccttggtcagtgcaagttcagatgatacacttcatttgtggaaccttagacaaaaaaggccagccatactccattctcttaaatttaaccgggaacgaattacttactgtcatctacctttccagagtaaatggctttatgttggaacagaaagaggaaatacacatattgtaaatattgaatctttcattctttctggatatgttatcatgtggaacaaggcaattgaactatccactaagactcatccaggtccagttgtacatttaagcgatagcccaagagatgaaggcaaactgctaataggttatgaaaatggtactgtagtattctgggacttgaaatctaaaagagcagaactgagagtttattatgatgaggctattcattcaattgattggcatcatgagggcaaacagttcatgtgcagccattcagatggtagtttgactttatggaacctgaaaagcccaagtcgccctttccagaccacaattccacatggaaaaagtcaaagagaaggaagaaaatctgaatcttgtaaaccaattcttaaagtagaatacaagacctgcaaaaacagcgaaccattcataatattctctggtgggctgtcctatgacaaagcttgtagaagaccaagtttaaccatcatgcatggaaaagcaattacagtacttgaaatggatcatcctattgttgaatttctaactttatgtgaaacgccctatccaaatgaatttcaagaaccctatgctgtcgtggtacttctggagaaagatctcattgtagttgatctgacacaaagcaattttccaatctttgaaaatccatatcccatggacattcatgaatcaccagttacatgcacagcatactttgcagattgtcctccggatttgattctagtactgtattctataggagtcaagcataaaaaacaaggatacagtaataaggagtggccaatcagtggaggagcttggaaccttggagcacaaacatatccagaaattattattactggtcatgcagatggatcaataaaattttgggatgcttctgcaataactctgcagatgctgtacaagctaaaaacttcaaaagtgtttgaaaaacagaaggtaggagaaggaaaacaaacatgtgaaattgtagaggaagacccatttgccattcagatgatttactggtgtccagagagcagaatattctgtgtatcaggagtctctgcatatgtcataatttataaattcagcagacatgaaattacaacagaaatagtgtcattagaggtacgacttcagtatgatgttgaagatattattacccctgaaccagaaacaagtcctccgtttccagatctctcagcccagcttccttcttcaaggagtctttctgggagcactaacactgttgctagtgaaggagtaacaaaggacagtattccatgcctcaatgtgaagacacggccagtgcgaatgcctccaggatatcaagcagaacttgttattcaattggtgtgggtagatggtgaacctccacaacagattactagtcttgctgtaagctcagcatatggaatagttgcatttgggaactgcaatgggttggctgtggtggattttatacagaagacagtactgttaagcatggggaccattgacctatatagatcaagtgacttataccagcgacaaccacggtctcctcgaaaaaacaaacagttcattgcaggtttaactgaactgaatgacagtccagttcccctagaacttgagcgctgcaagtctcctacctcagaccatgtaaatggacactgcacaagtccaacttctcagagttgcagttctggaaaacgtctttctagtgccgatgtttcaaaagtaaatcgctggggtcctggaagaccaccatttcgaaaggcccagtcagcagcctgcatggagatttctttaccagttacaacagaagaaaaccgagaaaattcctataatcgttctagaagctctagtatctccagtattgacaaagattctaaagaagcaattacagcactatacttcatggactcctttgcacggaaaaatgactctaccatctctccttgtctgttcgttggaaccagtctgggaatggtgttaatcatctccttaaacctaccattagcagatgaacaaaggtttacagagccagtcatggtattgccaagtggtacattcctctcattgaaaggagctgtgctaacattctcctgtatggaccgaatgggtggattaatgcaaccgccatatgaagtttggagggatccaaacaacatagatgaaaatgaaaaatcttggagaaggaaagtggtaatgaactcatcttctgcatcccaagaaataggagatcatcagtatacaataatctgctcagaaaaacaagccaaagtcttctcactgccttctcagacttgcctttatgttcataacatcacggagacatcttttatactgcaagcaaatgtggtggtcatgtgtagcagtgcctgcttggcatgcttttgtgctaacggacatatcatgataatgagcctacctagtcttcgcccaatgttggatgttaattatttgccactgacagacatgaggatagcacgaacattttgttttaccaatgaaggacaggcattatacctcgtctctcctactgaaattcagcggttaacatacagccaagaaatgtgtgataatctacaggacatgctaggagatttgtttactcccatagagacaccagaagctcaaaacagaggctttctcaagggactgtttggtggaagcggacaaacatttgacagagaagagctctttggggaagcttcggcaggaaaagcatcccgcagccttgcgcaacacattcctggaccaggtagtatagaagggatgaaaggcgctgctggaggggtgatgggagagctgacccgtgcacggattgcacttgatgaaagaggacagaggctaggagagctggaagagaaaactgcaggcatgatgaccagtgcagaagcattttccaaacatgcacatgagttaatgctgaaatacaaggataagaaatggtaccaattctgacttctaaagaagctgtgactgctttgagaaaccatattcagggaaaccaaatttattcccagcatcactactcaactgctagaagccagtttcttctacaaaatgttccatttacagtcaatctgaaattttcataaaagagatgtatcagagacactgtgcaacccaaaggctggagccctggttaaaatcccaaaatacggctgaatttgccttttcccatgtggaatggagctatcatcttggcatgtcattcgataaggatttatatttagtaactacggggagtcctcttgatttgaaaattcctgtacaaacaaaagcattaatgcacttaatgaaaaaaaatctttgcatgataaattaacatcttaaggggaaaagaaaaaaaagcatgttgtgatagaagaaaaaaagattcatggtaaactatttctatcaattgggccacactcaacaatttaaaaaatctgcatttgaagatgtcagtgcatttcaaatatatttgccatacccaactgaaacggaaaacaaaacaaaacaagaacccagagttttctcctcatctgtaactttcattgtactagaaccttattgaattcttatggcaagagtctgattaatgttctctctccatgttttacatcattcacagttgtgtcaaaatcaaatattgccagtatagtaaattattcccaacacaatcagtttcatttctatcaccttcagaatgggttgctgtttttagcacaaaccatgcagggttgggtcacctcaaagcattttcttcagcctggcttgtactctataggggagttggtagtaggtgtggggaatctataggaacaatagagttagctatgagaactgacttcacaaaaagggaaatttcacacaccccaatttcagcttctaaagtgatatattttaaaagcttcatttgtatccttgtctgccagttacacagtatattactgttcaaacccagtagggtctgcaatcgaaaggtgctcttgcagcctgacattcacaaaccaaactggtcattctctttagtgtgattcagtaaaatctcagttaatgttttgggaaagggattctgatttatgacatttctgatttacaagggctttccttagaaaatacctttcggtttgatacttaccactggaaattggttcgatacttaccactggaaatctttataaaatatagtgatctgtttgctatcttggtctcagtcatcattatagacaatagaaatacataaagagtttaatgatacaaaatcaatgcttttgtccctaggtcaaataatataagccactagattatgtcaatagatgccaaacacttgtcccttattaaagactcttttaaagctggaataaagaatatccttaacatgatacaaggtatctataactcaccagaaaagcaccagagtcaaaaccaaatagagacacctactaccatttaacatgattctggaagtcaaaagttataggaatgtatatatacacattccaggacccatcctgtaatatgttgtttcgtcaagaaaagttttaattatggttttggcttattgaatttttgtttatcaaggtctcattggatttacatttgtgtttcttaagacttcacaattttcctggatttcaggttattttattagccaaaaaatcgtatttttatttcctttttagtctaattttttgctagaagttgtactttctagcaaatgtttctagtggtacaatgttctcagtaattttgaggagaacaaagatgagtgaaagagttagataatgtacactaggatagcatttctcagagtccttgaatcctcttgttaagaaagcctctctgaatctcccagactcctgtgaacagccttacggtaacagaatctggcttggaaacacagacattacatgactgtataatttatagaattataaaattatatggtaaaaatattaaagaaacttaagagtaggatctagaaaatactagtggccaaattgcaatgtattctttgtaccatctgtttcaaagacttagttttctgattttcagaacaaatactttatcgtttctgtattttaaaaaaaactaaaagagtaaaatattagtttattttagaaataatgaaattcagtccaaagtagcagtacatttgatgagtatttctgaagccttcaataagatttaacttgttttaacttgatctacatcgagatttctcaaaagcagcactattagctgaaagtctttgttgtggggaactgtcctgtgtattgtaggatgttagcaacatccctggcctctgtctactagatgccagtaagaacctcctagtaatgacaatcaaaatgtctccagtcattgccaaaatttctcccagttcacagccactattctacatcatacaaagaggtagattgtgtgaatatgtaatatatgttgttgtataaaactgtacaataagtatacaatgtcttagcaagataaattattatacccaaaattacatgtgtggttcatatgcaataagatacaattttgaagaaagcttataggaatcagtgaaaaataacaactacagaatattttaaggcacacagagaaaatatcaaaaaggacattatagcatttcactgtagaagtgcttaaaaccttggcctcagtgaatagatcaaaagtttataattagcacaccaattggaagtaaacaggtgcttctcaaatgcttgaaaagaaaaggctctttgaagtagttaaaacgtgtctttcaaaattgcttttataagcccttccttaacgtaagggtaacttcatctcacaaactcctggttagtggaatccaaattaatgaggttttactgtatcaaaattatttttataattcaaagagatgatagcaataagaagaatctaatgtggatgtgatttttctctttgaacaattctgttctgttgcactgaccttagcacgcacgcacacacacacacaccatcgccaccactaccatcatcatcttatcctcatctttggaaaataagtactgttgatccatgtaatcctttgcatagtctcatctttactatctttcttctatttcggaacataagaaaaatactcctaataacttggacaatgatacagaaagtgactctgagccttagttaccatcaaaattacattctatctgctaaagcgacatcagaagataaggcttgcaaaccacagtcccaacaagttgaccttgtctccctatgatttccttggaagataaggcctttttagtgttacagtagaaaatgggccttttcatttattcatctgtgagaagctagaggtatttgtttccctgataataacgtgagcaatagtccctaccttgaaatcatccattagtcttggagtttggagggaggaatgattgattcctcatttgttttaatcacctacaaaagcagtactactgactttgcttcttacacttcactgagccccagactttagggccccaatcattgtcaagatcattgtctaactggaactctgaaaggacagtgacagaactgaatgagatgttttccagtgattcagtcacaaagacaattttctcagatcttttgaaagtgattctcaaataaataaatcaaaatccaactcctttccctcaaagtttctagggatctgaaggaaaaggtttactgttggagtccctttttatgtgacccatgtaccagttttaaaggcatcatctatactttatctacatgaagggatcaccatgactttgagagaaaaaagaatcagattaggcctaacattggttgaagaagattaaaatagattcttatattcaagcagaagggaaaaatgaagccaatctagaaaagtaagctaaaaatcctctccttggcttaggatcattgggtcaaactgggagtatatctgtgtgattacaacctgctgctatgagaaaaaagaattgtaacttgaccatgttggctcacacagggcaatgcaaaagaagtcaaaacattcatatcaggtcttggtatctgtgtcaggagaaacgtggtggctttcacagcttcttcacctctgtcctctgtcatgcaactccatttttggctaggtactatttcacatgcacactgtcctgggtgccagaaatacttgtggtgtacttggtttgagcagtacctctagtatgcaccattccagggaacatggttgtcaacataacaagtttagtgtgtgtatttgcagacaacatagccctgaaagcatgaaatgtagaataggtaaggtctgtcttagaaaaggaggaggaagtaccaatttggtgcaagaagatcgtggtgaggaaggacatgggagccacagtgaagtgaaagaggctttaaggaatcagatgcacagatggatgctttgatttacacatttatctagaggagtgattctcaaccttgactgtacataagaatcacctcaggaaatttttaaattcccaattatattaaaatcatttggagtgggaaccagacaccaatatttgcgaaagcctccaaggcggttctaatgtccagccaaagttgattatcactgctttatggccaactaaggaaaccttgtttgtctgccttggctggtgctccagccccagttctgagtggtcagggaaggcaagatgtaagatatagtaatggtatttattctgtatgtctcacagaacaaaagcatttgagaatttctgaccaggcagtgctccatcaactcttaataatcatctttgtgatattctcctatgtgacttgtccatcaattattccaattcaaaggtctaggttttttttcaattgtcttacacatgtgacatcacaagataccagaagtagcacagtaaattcaagagcatataaagctaagtggaaaactaattcttcatatttagacagtggaaattctcaaaacaatcatttgctaaattaggtccaaatttattattcattcttcttctggaggagacatgggtaccaggtacctgttctgctgtaggtatatttcactggacttggtcttagcaaaaaggaagaacaaatcttcctttttgattgttatctcaatcaaaagctcccagggccacttggatttattttcttagtctttggacatgtgtttaaaggaaaagaatacctgtaacttcctatatgacatccagtgccctgaaagggtgcttacaccttcaaaaaaggagagtccagcctatcaaaggcagtaacacataatgagaagaaactcagagttattgcctttcatactgctttccctctgctgttggcccacccttcttgactgcaaagccagaaaataaactagatggtggttttggacaattgtacacaggaacagaatctctaataacctataatttttagtacttaattatgtgatgttttattctaggaaataagaaacagatgacatcattgatgtatctttctttcatcttcagaatttttgcatcttttcagaaaatgacaaattactatttttctgttgcactcagcaattgtgactatacttaacaaaattcttgtagtctgtagagatatcaataaaattgtatatgtttgtacata

SEQ ID NO: 37 - protein, 530 aa, Homo sapiens
MTRDFKPGDLIFAKMKGYPHWPARVDEVPDGAVKPPTNKLPIFFFGTHETAFLGPKDIFPYSENKEKYGKPNKRKGFNEGLWEIDNNPKVKFSSQQAATKQSNASSDVEVEEKETSVSKEDTDHEEKASNEDVTKAVDITTPKAARRGRKRKAEKQVETEEAGVVTTATASVNLKVSPKRGRPAATEVKIPKPRGRPKMVKQPCPSESDIITEEDKSKKKGQEEKQPKKQPKKDEEGQKEEDKPRKEPDKKEGKKEVESKRKNLAKTGVTSTSDSEEEGDDQEGEKKRKGGRNFQTAHRRNMLKGQHEKEAADRKRKQEEQMETEQQNKDEGKKPEVKKVEKKRETSMDSRLQRIHAEIKNSLKIDNLDVNRCIEALDELASLQVTMQQAQKHTEMITTLKKIRRFKVSQVIMEKSTMLYNKFKNMFLVGEGDSVITQVLNKSLAEQRQHEEANKTKDQGKKGPNKKLEKEQTGSKTLNGGSDAQDGNQPQHNGESNEDSKDNHEASTKKKPSSEERETEISLKDSTLDN

SEQ ID NO: 38 - protein, 333 aa, Homo sapiens
MTRDFKPGDLIFAKMKGYPHWPARVDEVPDGAVKPPTNKLPIFFFGTHETAFLGPKDIFPYSENKEKYGKPNKRKGFNEGLWEIDNNPKVKFSSQQAATKQSNASSDVEVEEKETSVSKEDTDHEEKASNEDVTKAVDITTPKAARRGRKRKAEKQVETEEAGVVTTATASVNLKVSPKRGRPAATEVKIPKPRGRPKMVKQPCPSESDIITEEDKSKKKGQEEKQPKKQPKKDEEGQKEEDKPRKEPDKKEGKKEVESKRKNLAKTGVTSTSDSEEEGDDQEGEKKRKGGRNFQTAHRRNMLKGQHEKEAADRKRKQEEQMETEHQTTCNLQ

SEQ ID NO: 39 - protein, 329 aa, Homo sapiens
MTRDFKPGDLIFAKMKGYPHWPARVDEVPDGAVKPPTNKLPIFFFGTHETAFLGPKDIFPYSENKEKYGKPNKRKGFNEGLWEIDNNPKVKFSSQQAATKQSNASSDVEVEEKETSVSKEDTDHEEKASNEDVTKAVDITTPKAARRGRKRKAEKQVETEEAGVVTTATASVNLKVSPKRGRPAATEVKIPKPRGRPKMVKQPCPSESDIITEEDKSKKKGQEEKQPKKQPKKDEEGQKEEDKPRKEPDKKEGKKEVESKRKNLAKTGVTSTSDSEEEGDDQEGEKKRKGGRNFQTAHRRNMLKGQHEKEAADRKRKQEEQMETEHFAL

SEQ ID NO: 40 - RNA, 1690 nt, Homo sapiens
  source 1..1690: mol_type = mRNA
cgggcccggtagctgggcccgcgtccgccgcccgcatccccgcgccgccgcatctcctcgccgcctcccgggcttcggacccccggtctcgcccccgaaacatgactcgcgatttcaaacctggagacctcatcttcgccaagatgaaaggttatccccattggccagctcgagtagacgaagttcctgatggagctgtaaagccacccacaaacaaactacccattttcttttttggaactcatgagactgcttttttaggaccaaaggatatatttccttactcagaaaataaggaaaagtatggcaaaccaaataaaagaaaaggttttaatgaaggtttatgggagatagataacaatccaaaagtgaaattttcaagtcaacaggcagcaactaaacaatcaaatgcatcatctgatgttgaagttgaagaaaaggaaactagtgtttcaaaggaagataccgaccatgaagaaaaagccagcaatgaggatgtgactaaagcagttgacataactactccaaaagctgccagaagggggagaaagagaaaggcagaaaaacaagtagaaactgaggaggcaggagtagtgacaacagcaacagcatctgttaatctaaaagtgagtcctaaaagaggacgacctgcagctacagaagtcaagattccaaaaccaagaggcagacccaaaatggtaaaacagccctgtccttcagagagtgacatcattactgaagaggacaaaagtaagaaaaaggggcaagaggaaaaacaacctaaaaagcagcctaagaaggatgaagagggccagaaggaagaagataagccaagaaaagagccggataaaaaagaggggaagaaagaagttgaatcaaaaaggaaaaatttagctaaaacaggggttacttcaacctccgattctgaagaagaaggagatgatcaagaaggtgaaaagaagagaaaaggtgggaggaactttcagactgctcacagaaggaatatgctgaaaggccaacatgagaaagaagcagcagatcgaaaacgcaagcaagaggaacaaatggaaactgagcaccaaacaacatgtaatctacagtaataaaaaatatatctcattttgggctcaaagcattaatccagttactgaaaagagaatacaagtggagcaaacaagagatgaagatcttgatacagactcattggactgaatttcccccttccccccattgatggaagaatgttccagattctaaattgaggacttcattattaatggcattactgtgttatgattaacaaatttcctgtaaggtacacactacatactaaggtcggccatcattcctgttttttttttttttttttttttttaaccaagcttaaaatgaagctttgtgtttgaaagtaataacaagctcagacgaagatggtggttgtacattattcatctagaaaatataaaaattcattttgttttgaagctagttattaaactggaatagcagttatatccctgagaatggggcccttctcttgacattcctttgttgtttaattctttagaatcttaataaatgtttttttaatcctgagagattaaacagtagtagacttgttaagaatgaaactgtaaccaaaattttaaaataaagttttttttaaaaaaaaaaaaaaaaaaaaaaaaaa

SEQ ID NO: 41 - RNA, 3410 nt, Homo sapiens
  source 1..3410: mol_type = mRNA
agttggtcgcgccccagtgctagcgggcgccgagcgggagccgcgcgggagcagcgcagctacggcggcggcagcggcggcgcggttgcgattccgagccgttgagacgcctctgcggcagctggtggcgcaggtggcttgcgtggacgcgggtagaggcgaccggccagcaaccgcagcgtcggcgcccgcggccccggcagcaggcgcgtcgggacgccccgaggcatcctcccccgcccgcgggcccggtagctgggcccgcgtccgccgcccgcatccccgcgccgccgcatctcctcgccgcctcccgggcttcggacccccggtctcgcccccgaaacatgactcgcgatttcaaacctggagacctcatcttcgccaagatgaaaggttatccccattggccagctcgagtagacgaagttcctgatggagctgtaaagccacccacaaacaaactacccattttcttttttggaactcatgagactgcttttttaggaccaaaggatatatttccttactcagaaaataaggaaaagtatggcaaaccaaataaaagaaaaggttttaatgaaggtttatgggagatagataacaatccaaaagtgaaattttcaagtcaacaggcagcaactaaacaatcaaatgcatcatctgatgttgaagttgaagaaaaggaaactagtgtttcaaaggaagataccgaccatgaagaaaaagccagcaatgaggatgtgactaaagcagttgacataactactccaaaagctgccagaagggggagaaagagaaaggcagaaaaacaagtagaaactgaggaggcaggagtagtgacaacagcaacagcatctgttaatctaaaagtgagtcctaaaagaggacgacctgcagctacagaagtcaagattccaaaaccaagaggcagacccaaaatggtaaaacagccctgtccttcagagagtgacatcattactgaagaggacaaaagtaagaaaaaggggcaagaggaaaaacaacctaaaaagcagcctaagaaggatgaagagggccagaaggaagaagataagccaagaaaagagccggataaaaaagaggggaagaaagaagttgaatcaaaaaggaaaaatttagctaaaacaggggttacttcaacctccgattctgaagaagaaggagatgatcaagaaggtgaaaagaagagaaaaggtgggaggaactttcagactgctcacagaaggaatatgctgaaaggccaacatgagaaagaagcagcagatcgaaaacgcaagcaagaggaacaaatggaaactgagcagcagaataaagatgaaggaaagaagccagaagttaagaaagtggagaagaagcgagaaacatcaatggattctcgacttcaaaggatacatgctgagattaaaaattcactcaaaattgataatcttgatgtgaacagatgcattgaggccttggatgaacttgcttcacttcaggtcacaatgcaacaagctcagaaacacacagagatgattactacactgaaaaaaatacggcgattcaaagttagtcaggtaatcatggaaaagtctacaatgttgtataacaagtttaagaacatgttcttggttggtgaaggagattccgtgatcacccaagtgctgaataaatctcttgctgaacaaagacagcatgaggaagcgaataaaaccaaagatcaagggaagaaagggccaaacaaaaagctagagaaggaacaaacagggtcaaagactctaaatggaggatctgatgctcaagatggtaatcagccacaacataacggggagagcaatgaagacagcaaagacaaccatgaagccagcacgaagaaaaagccatccagtgaagagagagagactgaaatatctctgaaggattctacactagataactaggttgacatacctggaatatagagaacacttgagaagtttgtaatggttttcatttgaaatagactgctgaaagttttaaatttttataagcataggtttgatgttgaaaacttgttttgagggagaaaatccctttgttttaaagtaaagtaaacattatcgctaagtgtacttgtgcagtattaacagctacattatacagtaaatgtgggataaaatccatttagaaaatgttaaactgcttttccagacatggttgtagcatattttcaattagtgtgtgtatgttaatgtgtaattgatagtagaacaaagttacatttttaaaactgctacttgtataaaccttgcctcttttcccaaatactgtgggttttgtgcatagtttttacaaaccttggatttaccagactgtcttttcactgtttgtgggttttgtagaagttacacatttttatggtagataaaatgttacttctatacaagtactcactccctttttatcaaaagttaattttaatctcacagtctacattgtgctacattatccagcttctttggaacaatgtgtgctctgtatggttttttttggtatgacaactaattaagcaactgacatggaactgagaattctacaaactataaaacattaatttttgaaggtaatttagttttgtggctgggcattcagtgaagtcttaggacttctttgcagacaactgactgggtatatataggaatgaatctggctttagggttaaatcatttaaggtccttttataggcaggcactagtaactaaaactgaaaactaagtaagtttatttttgaggaatgttgttaaaaatgtctttaggaagtcactaaaacttaattggaagaaaaaatcatgatgcttatacaataaatatgaataaatgttatataaggaaactcacctatttgaaatcatggctatattgtttttattttctagattccaaaaatacaaacactagttgttccagcattgtactttgataagtctgtacattgacgtgtatggactaaatccagggtaaaatcaatgttacaaaatttaagggtatgttaactaaaggatagcatttctaagatattttgaatattagggtcatttggcacttctcagcaagtaggatacttctcatgttttgaaattatatgaatatggaaaaaaatggcttaagaccagcgtctctgtatgacattgtgtggttgaccctctgagataactgttttcatctacagaattgcatttttgcttttaaagaggtcttataatggaactaggaatcaccgttttgagagaacctgcatatataccagtcattatctgtttggtccttatacagttttaacttacttagatttattctagttaagccataagttcaacgtgtaaacttgttttcattaaagaatttttctatcaaaaaaaaaaaaaaaaaaaaaa

SEQ ID NO: 42 - RNA, 3407 nt, Homo sapiens
  source 1..3407: mol_type = mRNA
agttggtcgcgccccagtgctagcgggcgccgagcgggagccgcgcgggagcagcgcagctacggcggcggcagcggcggcgcggttgcgattccgagccgttgagacgcctctgcggcagctggtggcgcaggtggcttgcgtggacgcgggtagaggcgaccggccagcaaccgcagcgtcggcgcccgcggccccggcaggcgcgtcgggacgccccgaggcatcctcccccgcccgcgggcccggtagctgggcccgcgtccgccgcccgcatccccgcgccgccgcatctcctcgccgcctcccgggcttcggacccccggtctcgcccccgaaacatgactcgcgatttcaaacctggagacctcatcttcgccaagatgaaaggttatccccattggccagctcgagtagacgaagttcctgatggagctgtaaagccacccacaaacaaactacccattttcttttttggaactcatgagactgcttttttaggaccaaaggatatatttccttactcagaaaataaggaaaagtatggcaaaccaaataaaagaaaaggttttaatgaaggtttatgggagatagataacaatccaaaagtgaaattttcaagtcaacaggcagcaactaaacaatcaaatgcatcatctgatgttgaagttgaagaaaaggaaactagtgtttcaaaggaagataccgaccatgaagaaaaagccagcaatgaggatgtgactaaagcagttgacataactactccaaaagctgccagaagggggagaaagagaaaggcagaaaaacaagtagaaactgaggaggcaggagtagtgacaacagcaacagcatctgttaatctaaaagtgagtcctaaaagaggacgacctgcagctacagaagtcaagattccaaaaccaagaggcagacccaaaatggtaaaacagccctgtccttcagagagtgacatcattactgaagaggacaaaagtaagaaaaaggggcaagaggaaaaacaacctaaaaagcagcctaagaaggatgaagagggccagaaggaagaagataagccaagaaaagagccggataaaaaagaggggaagaaagaagttgaatcaaaaaggaaaaatttagctaaaacaggggttacttcaacctccgattctgaagaagaaggagatgatcaagaaggtgaaaagaagagaaaaggtgggaggaactttcagactgctcacagaaggaatatgctgaaaggccaacatgagaaagaagcagcagatcgaaaacgcaagcaagaggaacaaatggaaactgagcagcagaataaagatgaaggaaagaagccagaagttaagaaagtggagaagaagcgagaaacatcaatggattctcgacttcaaaggatacatgctgagattaaaaattcactcaaaattgataatcttgatgtgaacagatgcattgaggccttggatgaacttgcttcacttcaggtcacaatgcaacaagctcagaaacacacagagatgattactacactgaaaaaaatacggcgattcaaagttagtcaggtaatcatggaaaagtctacaatgttgtataacaagtttaagaacatgttcttggttggtgaaggagattccgtgatcacccaagtgctgaataaatctcttgctgaacaaagacagcatgaggaagcgaataaaaccaaagatcaagggaagaaagggccaaacaaaaagctagagaaggaacaaacagggtcaaagactctaaatggaggatctgatgctcaagatggtaatcagccacaacataacggggagagcaatgaagacagcaaagacaaccatgaagccagcacgaagaaaaagccatccagtgaagagagagagactgaaatatctctgaaggattctacactagataactaggttgacatacctggaatatagagaacacttgagaagtttgtaatggttttcatttgaaatagactgctgaaagttttaaatttttataagcataggtttgatgttgaaaacttgttttgagggagaaaatccctttgttttaaagtaaagtaaacattatcgctaagtgtacttgtgcagtattaacagctacattatacagtaaatgtgggataaaatccatttagaaaatgttaaactgcttttccagacatggttgtagcatattttcaattagtgtgtgtatgttaatgtgtaattgatagtagaacaaagttacatttttaaaactgctacttgtataaaccttgcctcttttcccaaatactgtgggttttgtgcatagtttttacaaaccttggatttaccagactgtcttttcactgtttgtgggttttgtagaagttacacatttttatggtagataaaatgttacttctatacaagtactcactccctttttatcaaaagttaattttaatctcacagtctacattgtgctacattatccagcttctttggaacaatgtgtgctctgtatggttttttttggtatgacaactaattaagcaactgacatggaactgagaattctacaaactataaaacattaatttttgaaggtaatttagttttgtggctgggcattcagtgaagtcttaggacttctttgcagacaactgactgggtatatataggaatgaatctggctttagggttaaatcatttaaggtccttttataggcaggcactagtaactaaaactgaaaactaagtaagtttatttttgaggaatgttgttaaaaatgtctttaggaagtcactaaaacttaattggaagaaaaaatcatgatgcttatacaataaatatgaataaatgttatataaggaaactcacctatttgaaatcatggctatattgtttttattttctagattccaaaaatacaaacactagttgttccagcattgtactttgataagtctgtacattgacgtgtatggactaaatccagggtaaaatcaatgttacaaaatttaagggtatgttaactaaaggatagcatttctaagatattttgaatattagggtcatttggcacttctcagcaagtaggatacttctcatgttttgaaattatatgaatatggaaaaaaatggcttaagaccagcgtctctgtatgacattgtgtggttgaccctctgagataactgttttcatctacagaattgcatttttgcttttaaagaggtcttataatggaactaggaatcaccgttttgagagaacctgcatatataccagtcattatctgtttggtccttatacagttttaacttacttagatttattctagttaagccataagttcaacgtgtaaacttgttttcattaaagaatttttctatcaaaaaaaaaaaaaaaaaaaaaa

SEQ ID NO: 43 - RNA, 2014 nt, Homo sapiens
  source 1..2014: mol_type = mRNA
agttggtcgcgccccagtgctagcgggcgccgagcgggagccgcgcgggagcagcgcagctacggcggcggcagcggcggcgcggttgcgattccgagccgttgagacgcctctgcggcagctggtggcgcaggtggcttgcgtggacgcgggtagaggcgaccggccagcaaccgcagcgtcggcgcccgcggccccggcaggcgcgtcgggacgccccgaggcatcctcccccgcccgcgggcccggtagctgggcccgcgtccgccgcccgcatccccgcgccgccgcatctcctcgccgcctcccgggcttcggacccccggtctcgcccccgaaacatgactcgcgatttcaaacctggagacctcatcttcgccaagatgaaaggttatccccattggccagctcgagtagacgaagttcctgatggagctgtaaagccacccacaaacaaactacccattttcttttttggaactcatgagactgcttttttaggaccaaaggatatatttccttactcagaaaataaggaaaagtatggcaaaccaaataaaagaaaaggttttaatgaaggtttatgggagatagataacaatccaaaagtgaaattttcaagtcaacaggcagcaactaaacaatcaaatgcatcatctgatgttgaagttgaagaaaaggaaactagtgtttcaaaggaagataccgaccatgaagaaaaagccagcaatgaggatgtgactaaagcagttgacataactactccaaaagctgccagaagggggagaaagagaaaggcagaaaaacaagtagaaactgaggaggcaggagtagtgacaacagcaacagcatctgttaatctaaaagtgagtcctaaaagaggacgacctgcagctacagaagtcaagattccaaaaccaagaggcagacccaaaatggtaaaacagccctgtccttcagagagtgacatcattactgaagaggacaaaagtaagaaaaaggggcaagaggaaaaacaacctaaaaagcagcctaagaaggatgaagagggccagaaggaagaagataagccaagaaaagagccggataaaaaagaggggaagaaagaagttgaatcaaaaaggaaaaatttagctaaaacaggggttacttcaacctccgattctgaagaagaaggagatgatcaagaaggtgaaaagaagagaaaaggtgggaggaactttcagactgctcacagaaggaatatgctgaaaggccaacatgagaaagaagcagcagatcgaaaacgcaagcaagaggaacaaatggaaactgagcattttgctctgtaaagcatttcagatgcagcttgtgtgaaatgcattatgcaaaataaagtttattgtattgtattcccagccaaacaacatgtaatctacagtaataaaaaatatatctcattttgggctcaaagcattaatccagttactgaaaagagaatacaagtggagcaaacaagagatgaagatcttgatacagactcattggactgaatttcccccttccccccattgatggaagaatgttccagattctaaattgaggacttcattattaatggcattactgtgttatgattaacaaatttcctgtaaggtacacactacatactaaggtcggccatcattcctgttttttttttttttttttttttttaaccaagcttaaaatgaagctttgtgtttgaaagtaataacaagctcagacgaagatggtggttgtacattattcatctagaaaatataaaaattcattttgttttgaagctagttattaaactggaatagcagttatatccctgagaatggggcccttctcttgacattcctttgttgtttaattctttagaatcttaataaatgtttttttaatcctgagagattaaacagtagtagacttgttaagaatgaaactgtaaccaaaattttaaaataaagttttttttaaaaaaaaaaaaaaaaaaaaaaaaaaaaaa

SEQ ID NO: 44 - RNA, 1903 nt, Homo sapiens
  source 1..1903: mol_type = mRNA
agttggtcgcgccccagtgctagcgggcgccgagcgggagccgcgcgggagcagcgcagctacggcggcggcagcggcggcgcggttgcgattccgagccgttgagacgcctctgcggcagctggtggcgcaggtggcttgcgtggacgcgggtagaggcgaccggccagcaaccgcagcgtcggcgcccgcggccccggcaggcgcgtcgggacgccccgaggcatcctcccccgcccgcgggcccggtagctgggcccgcgtccgccgcccgcatccccgcgccgccgcatctcctcgccgcctcccgggcttcggacccccggtctcgcccccgaaacatgactcgcgatttcaaacctggagacctcatcttcgccaagatgaaaggttatccccattggccagctcgagtagacgaagttcctgatggagctgtaaagccacccacaaacaaactacccattttcttttttggaactcatgagactgcttttttaggaccaaaggatatatttccttactcagaaaataaggaaaagtatggcaaaccaaataaaagaaaaggttttaatgaaggtttatgggagatagataacaatccaaaagtgaaattttcaagtcaacaggcagcaactaaacaatcaaatgcatcatctgatgttgaagttgaagaaaaggaaactagtgtttcaaaggaagataccgaccatgaagaaaaagccagcaatgaggatgtgactaaagcagttgacataactactccaaaagctgccagaagggggagaaagagaaaggcaggagtagtgacaacagcaacagcatctgttaatctaaaagtgagtcctaaaagaggacgacctgcagctacagaagtcaagattccaaaaccaagaggcagacccaaaatggtaaaacagccctgtccttcagagagtgacatcattactgaagaggacaaaagtaagaaaaaggggcaagaggaaaaacaacctaaaaagcagcctaagaaggatgaagagggccagaaggaagaagataagccaagaaaagagccggataaaaaagaggggaagaaagaagttgaatcaaaaaggaaaaatttagctaaaacaggggttacttcaacctccgattctgaagaagaaggagatgatcaagaaggtgaaaagaagagaaaaggtgggaggaactttcagactgctcacagaaggaatatgctgaaaggccaacatgagaaagaagcagcagatcgaaaacgcaagcaagaggaacaaatggaaactgagcaccaaacaacatgtaatctacagtaataaaaaatatatctcattttgggctcaaagcattaatccagttactgaaaagagaatacaagtggagcaaacaagagatgaagatcttgatacagactcattggactgaatttcccccttccccccattgatggaagaatgttccagattctaaattgaggacttcattattaatggcattactgtgttatgattaacaaatttcctgtaaggtacacactacatactaaggtcggccatcattcctgttttttttttttttttttttttttaaccaagcttaaaatgaagctttgtgtttgaaagtaataacaagctcagacgaagatggtggttgtacattattcatctagaaaatataaaaattcattttgttttgaagctagttattaaactggaatagcagttatatccctgagaatggggcccttctcttgacattcctttgttgtttaattctttagaatcttaataaatgtttttttaatcctgagagattaaacagtagtagacttgttaagaatgaaactgtaaccaaaattttaaaataaagttttttttaaaaaaaaaaaaaaaaaaaaaaaaaa

SEQ ID NO: 45 - protein, 653 aa, Homo sapiens
MISSKMMSSNPEEDPLDTFLQYIEDMGMKAYDGLVIQNASDIARENDRLRNETNLAYLKEKNEKRRRQEEAIKRIGGEVGRGHEGSYVGKHFRMGFMTMPAPQDRLPHPCSSGFSVRSQSLHSVGGTDDDSSCGSRRQPPPKPKRDPSTKLSTSSETVSSTAASKSGKTPERTEASAKPRPHSDEYSKKIPPPKPKRNPNTQLSTSFDETYIKKHGPRRTSLPRDSSLSQMGSPAGDPEEEEPVYIEMVGNILRDFRKEDDDQSEAVYEEMKYPIFDDLGQDAKCDFDHHSCSSQCATPTVPDLDFAKASVPCPPKGLLCDIPPPFPNLLSHRPPLLVFPPAPVHCSPNSDESPLTPLEVTKLPVLENVSYMKQPAGASPSTLPSHVPGHAKLEKEQAAALGPASATPALSSSPPPPSTLYRTQSPHGYPKSHSTSPSPVSMGRSLTPLSLKRPPPYDAVHSGSLSRSSPSVPHSTPRPVSQDGAKMVNAAVNTYGAAPGGSRSRTPTSPLEELTSLFSSGRSLLRKSSSGRRSKEPAEKSTEELKVRSHSTEPLPKLDNKERGHHGASSSREPVKAQEWDGTPGTPVVTSRLGRCSVSPTLLAGNHSSEPKVSCKLGRSASTSGVPPPSVTPLRQSSDLQQSQVPSSLANRD

SEQ ID NO: 46 - protein, 145 aa, Homo sapiens
MISSKMMSSNPEEDPLDTFLQYIEDMGMKAYDGLVIQNASDIARENDRLRNETNLAYLKEKNEKRRRQEEAIKRINRGTESPKPQHGAITKVGQQGKRPPWGVFLQRACQSSGMGWNTRATCGHQSTRKMLCEPHLVSGKPQFRA

SEQ ID NO: 47 - protein, 159 aa, Homo sapiens
MVNAAVNTYGAAPGGSRSRTPTSPLEELTSLFSSGRSLLRKSSSGRRSKEPAEKSTEELKVRSHSTEPLPKLDNKERGHHGASSSREPVKAQEWDGTPGTPVVTSRLGRCSVSPTLLAGNHSSEPKVSCKLGRSASTSGVPPPSVTPLRQSSDLQQSQI

SEQ ID NO: 48 - RNA, 4590 nt, Homo sapiens
  source 1..4590: mol_type = mRNA
taattgaagaaacactgagctgaactacaagtctatttcttatggtgctggattactcctacagaactgccctgagatcaaccgtgagagagggctctgacagacacaagtcaccttctggttattgcacttagctctccctggggacttaaattttggcagtgttcctctttacatgatatcctccaagatgatgagttctaatcctgaggaagaccctttggacacatttctccagtacattgaggatatggggatgaaggcctatgatggcttggttattcagaatgcgtcagatattgctcgagagaatgatcgcttgagaaatgaaactaacctagcctatttgaaagagaagaatgaaaaacgccgaagacaagaagaagcaataaagcgcataggtggagaagtagggcgaggccacgaaggaagttacgtgggcaaacatttccgcatgggattcatgacaatgcctgctcctcaggacagacttccccatccttgctccagtggcttttctgtgagatcacagtccctgcactcggttgggggcacagacgatgacagcagctgtggctcacggagacaaccaccacccaaacccaagagggaccccagcaccaagctgagcacctcatcagagacagtcagcagcactgcagccagtaagagcgggaaaacccctgagaggactgaagcgtcagctaaaccaagaccccacagcgatgaatattccaagaagattcctcctcccaaaccgaagcgaaatccgaacactcagctgagcacatctttcgatgaaacgtacatcaaaaagcatgggccccggaggacgtcgctgccgcgggactcctccttgtcccagatgggcagccccgcgggagaccccgaggaagaggagcccgtgtacatcgagatggtggggaacattctcagagacttcaggaaggaggacgatgaccagagcgaggccgtctacgaggaaatgaagtaccctatctttgacgacttgggccaagacgccaaatgtgacttcgaccatcacagctgttcttcgcagtgtgctactcccacggtgcctgacttggacttcgccaaggcctcagtgccatgcccccccaaggggctgctttgcgacatccctccgcccttccccaacctgctttctcacagacccccgctgctggtatttccccccgcccccgtgcattgctcccccaactccgacgagtccccgcttacccctctggaggtcacgaagcttcccgtgctggaaaacgtgtcttacatgaaacagccagccggggcgtcgccctccacgctgccgtcccacgtccccggccatgcgaaactggagaaagagcaggccgcggccctgggacctgcctctgccacccctgcgctctcctcgtcgcccccacccccgtctacgctgtaccgaacccagtctccccatggctaccctaaaagtcactccacctctccctcccccgtcagcatggggaggtccctgactcccctgagcctcaaaaggcctcccccttacgacgctgtgcattcgggcagcctctcaaggagctctccttcagtgcctcactcgacccccagacccgtgtcgcaagatggggccaagatggtcaacgccgcggtgaacacctacggggcagccccgggtggctcccggtcccggacacccacgagcccgctggaggagctgaccagcctcttctcctccggccgcagcctgctgcgcaagtcgtccagtggccggcgctccaaagagcctgcagagaaatcaacagaggaactgaaagtccgaagccacagcacggagccattaccaaagttggacaacaaggaaagaggccaccatggggcgtcttcctccagagagcctgtcaaagctcaggaatgggatggaacaccagggacacctgtggtcaccagtcgactaggaagatgctctgtgagccccaccttgttagcgggaaaccacagttcagagcctaaagtaagctgcaaattaggccggtctgcgtcgacgtcaggtgtgcctcctccatcagtcactcccctcaggcaaagcagtgacctgcaacagagccaggtaccatcatcgttagccaatcgtgattgacttcctgtgatacaacttgccaaatgcttcccacctctgtctgtcctgttgctgtagacaactttcgcatttgcttttatttttctatgtgtgtatgggttaggggatgcgggggatgagttctggcagtctgtgttttcatttgaaaaagaatatctttcttccttgtgattggtggtgaaactttctttgctgtttgttaccaaatcgtttttgtctctggtttccatcattctgtaatataaatgtagtaaacttgtactatatgtattggcttagtggttcttttttaaattctttctctctttcatgttttgtgtacttttatactgtctctgaaaatttatcaatatttgataaatttatctactttgttttatgtagatttctttttaaatgttttgtccagaacactcgcacagatgttgtcaatgaatttgtacatatttcttagctcttatcctattatactgtaatatttctggtggttttatttttatttagcttggagcatgactgtaagacactgttgaatattgatgtccttataaatattcatatcccgattcatttggattgagtatggcagctagtctttcttctttcttaggctattgactggcctaagacaatttgactggccagacaaattgactggccagataatctagatatttaacaaaaactgcagattaataaggcaacctttaaatgaatgacttttctctcttataccaacaatatcagaaatgttctcagaaagggaatgtaagtgttcatgcatggtaaatgagatctcaattatcacttggagaaaagagacaagaaataaaggcataaactgaaatatcatttaatcctttacagcataatatgttgctctgatgttcgtttgggtacgtggttgtggatggggaattagtatggggaaaaatcactacacataaatgtcctatctttagctcacccaataggaattcaatacattgacttaatttgtgaggcttaattgtcgttactgttaagtattataggtgttaagtagggtggtgtcattctggaatgttttctctctgcttcctagcttcaatctttgcattcatgaaactcttctgaaatagcaacttataaaacactgatgatacctccaagggaactgcccattactgatgagaaaattacatattcatctattattttaaatgtcaggctattttaaaaacataactaagtagaataattgcgttttcttctaatgagagacattgtgcctcttagtgtttttgtctgacttaaatatgcaaaatagttgatttataaatatatgaggtatctgcaaatacaagaaatgagaggcttctctcaagggtatctcaagtaccatttagaatttcttgtgtcttaatttaaaatttaaatgcctttatataaatgttaaatgcctttataactaaatgtaccaactcaaacactttttggatataaaagaagtagaaacagtaagacactgaataaaataaataagataaactgccaacttagctaattaaagctattccaaaaatattgtacttaccaacatttaaagcttaaaaacattgggtactgaaagaagagaagtttagctaattggcagaggattgcactaatacaatcaagttttcaagtttatgacccttgctagtatattaccttcaatatctcagagatgttttgtattatttgttttgttttgcttttttcctagttgtctttatagctgtttcaccctaagccccttcaaactctcaatgaaagcaggttcttgggataaacttccagaatagagacaaggtataccctttgtgcctttgcattatcaactctttgttcacctgatgggaagttcttcgtttttcaaaatgtagcaagggagaaagcccaggacgcctttatatgctgttagtttccttacctgctgatagagattctgacacacagtcaaatcatacatgggctgtcagagctataaattagaaggctggcctctaggcttctcctctgtggcttatagccagttgtaatatacatgcattcctatactctagagatgaagtggtaagcatagctcatatgaacactgctctgaactcctctgacttagcattcaacttaagtcaagaaatacttattggctgggcgtggtggctcacgcctgtaatcccagcactctgggaggcagaggtgggtggatcacaaggtcaggagattgagaccatcctggctaacacggtgagaccccatctctactaaaaatacaaaaaattagccaggtgtggtggcgggcgcctgtagtcccagctacttgggaggctgaggcaggagaatgtggtgaacctgggaggtggagcttgcagtgagctgagatcgcaccactgcactccagcctgggtgacagagcgagactccatctc

SEQ ID NO: 49 - protein, 1225 aa, Homo sapiens
MFARKPPGAAPLGAMPVPDQPSSASEKTSSLSPGLNTSNGDGSETETTSAILASVKEQELQFERLTRELEAERQIVASQLERCKLGSETGSMSSMSSAEEQFQWQSQDGQKDIEDELTTGLELVDSCIRSLQESGILDPQDYSTGERPSLLSQSALQLNSKPEGSFQYPASYHSNQTLALGETTPSQLPARGTQARATGQSFSQGTTSRAGHLAGPEPAPPPPPPPREPFAPSLGSAFHLPDAPPAAAAAALYYSSSTLPAPPRGGSPLAAPQGGSPTKLQRGGSAPEGATYAAPRGSSPKQSPSRLAKSYSTSSPINIVVSSAGLSPIRVTSPPTVQSTISSSPIHQLSSTIGTYATLSPTKRLVHASEQYSKHSQELYATATLQRPGSLAAGSRASYSSQHGHLGPELRALQSPEHHIDPIYEDRVYQKPPMRSLSQSQGDPLPPAHTGTYRTSTAPSSPGVDSVPLQRTGSQHGPQNAAAATFQRASYAAGPASNYADPYRQLQYCPSVESPYSKSGPALPPEGTLARSPSIDSIQKDPREFGWRDPELPEVIQMLQHQFPSVQSNAAAYLQHLCFGDNKIKAEIRRQGGIQLLVDLLDHRMTEVHRSACGALRNLVYGKANDDNKIALKNCGGIPALVRLLRKTTDLEIRELVTGVLWNLSSCDALKMPIIQDALAVLTNAVIIPHSGWENSPLQDDRKIQLHSSQVLRNATGCLRNVSSAGEEARRRMRECDGLTDALLYVIQSALGSSEIDSKTVENCVCILRNLSYRLAAETSQGQHMGTDELDGLLCGEANGKDAESSGCWGKKKKKKKSQDQWDGVGPLPDCAEPPKGIQMLWHPSIVKPYLTLLSECSNPDTLEGAAGALQNLAAGSWKWSVYIRAAVRKEKGLPILVELLRIDNDRVVCAVATALRNMALDVRNKELIGKYAMRDLVHRLPGGNNSNNTASKAMSDDTVTAVCCTLHEVITKNMENAKALRDAGGIEKLVGISKSKGDKHSPKVVKAASQVLNSMWQYRDLRSLYKKDGWSQYHFVASSSTIERDRQRPYSSSRTPSISPVRVSPNNRSASAPASPREMISLKERKTDYECTGSNATYHGAKGEHTSRKDAMTAQNTGISTLYRNSYGAPAEDIKHNQVSAQPVPQEPSRKDYETYQPFQNSTRNYDESFFEDQVHHRPPASEYTMHLGLKSTGNYVDFYSAARPYSELNYETSHYPASPDSWV

SEQ ID NO: 50 - protein, 1167 aa, Homo sapiens
MFARKPPGAAPLGAMPVPDQPSSASEKTSSLSPGLNTSNGDGSETETTSAILASVKEQELQFERLTRELEAERQIVASQLERCKLGSETGSMSSMSSAEEQFQWQSQDGQKDIEDELTTGLELVDSCIRSLQESGILDPQDYSTGERPSLLSQSALQLNSKPEGSFQYPASYHSNQTLALGETTPSQLPARGTQARATGQSFSQGTTSRAGHLAGPEPAPPPPPPPREPFAPSLGSAFHLPDAPPAAAAAALYYSSSTLPAPPRGGSPLAAPQGGSPTKLQRGGSAPEGATYAAPRGSSPKQSPSRLAKSYSTSSPINIVVSSAGLSPIRVTSPPTVQSTISSSPIHQLSSTIGTYATLSPTKRLVHASEQYSKHSQELYATATLQRPGSLAAGSRASYSSQHGHLGPELRALQSPEHHIDPIYEDRVYQKPPMRSLSQSQGDPLPPAHTGTYRTSTAPSSPGVDSVPLQRTGSQHGPQNAAAATFQRASYAAGPASNYADPYRQLQYCPSVESPYSKSGPALPPEGTLARSPSIDSIQKDPREFGWRDPELPEVIQMLQHQFPSVQSNAAAYLQHLCFGDNKIKAEIRRQGGIQLLVDLLDHRMTEVHRSACGALRNLVYGKANDDNKIALKNCGGIPALVRLLRKTTDLEIRELVTGVLWNLSSCDALKMPIIQDALAVLTNAVIIPHSGWENSPLQDDRKIQLHSSQVLRNATGCLRNVSSAGEEARRRMRECDGLTDALLYVIQSALGSSEIDSKTVENCVCILRNLSYRLAAETSQGQHMGTDELDGLLCGEANGKDAESSGCWGKKKKKKKSQDQWSVYIRAAVRKEKGLPILVELLRIDNDRVVCAVATALRNMALDVRNKELIGKYAMRDLVHRLPGGNNSNNTASKAMSDDTVTAVCCTLHEVITKNMENAKALRDAGGIEKLVGISKSKGDKHSPKVVKAASQVLNSMWQYRDLRSLYKKDGWSQYHFVASSSTIERDRQRPYSSSRTPSISPVRVSPNNRSASAPASPREMISLKERKTDYECTGSNATYHGAKGEHTSRKDAMTAQNTGISTLYRNSYGAPAEDIKHNQVSAQPVPQEPSRKDYETYQPFQNSTRNYDESFFEDQVHHRPPASEYTMHLGLKSTGNYVDFYSAARPYSELNYETSHYPASPDSWV

SEQ ID NO: 51 - RNA, 5481 nt, Homo sapiens
  source 1..5481: mol_type = mRNA
gcgtcgggagccgcctctcgcccgcggcgctcgcccctgccgcccgccagcatcccttgtcccgcggccgcgctcagacaacaaaagcggaagatgctgcagttgggcaaggtcaggaccttgccctgaagccgggcggcgccgcgcacgcctcttcccggactgaggagctgtcgccggcggagggtgcatgtttgcgaggaagccgccgggcgccgcgcctttgggagctatgcctgttccagaccagccttcatcagcctcagagaagacgagttccctgagccccggcttaaacacctccaacggggatggctctgaaacagaaaccacctctgccatcctcgcctcagtcaaagaacaggaattacagtttgaaaggctgacccgagagctggaggctgaacggcagatcgtagccagccagctggagcgatgcaagctcggatccgagactggcagcatgagcagcatgagttcagcagaagagcagtttcagtggcagtcacaagatggtcaaaaagatatcgaagatgagcttacaacaggtctcgagctggtggactcctgtattaggtcactacaggaatcaggaatacttgacccacaggattattctacaggtgaaaggcccagcctgctctcccagagtgcacttcagctcaattccaaacctgaagggtctttccagtatccggccagctaccatagcaaccagaccctggccctgggggaaaccaccccttcacagctcccggcccgaggcacacaagcccgagctacgggccagagcttcagccagggcacgaccagccgcgccggccacctggcggggcccgagcccgcgccgccgccgccgccgccgccgcgggagccgttcgcgcccagcctgggcagcgccttccacctgcccgacgcgccgcccgccgccgccgccgccgcgctctactactccagctccacgctgcccgcgccgccgcgcgggggctccccgctggccgcgccccagggcggttcgcccaccaagctgcagcgcggcggctcggcccccgagggcgccacctacgccgcgccgcgcggctcctcgcccaagcagtcgcccagccgcctggccaagtcctacagcaccagctcgcccatcaacatcgtcgtgtcctcggccggcctgtccccgatccgcgtgacctcgccccccaccgtgcagtccaccatctcctcctcgcccatccaccagctgagctccaccatcggcacgtacgccaccctgtcgcccaccaagcgcctggtccacgcgtccgagcagtacagcaagcactcgcaggagctgtatgccacggccaccctccagaggccgggcagcctggcagctggttcccgagcctcatacagcagccagcatgggcacctgggcccagagttgcgggccctgcagtccccagaacaccacatagatcccatctatgaagaccgcgtctatcagaagccccctatgaggagtctcagccagagccagggggaccctctgccgccagcacacaccggcacctaccgcacgagcacagccccatcttcccctggtgtcgactccgtccccttgcagcgcacaggcagccagcacggcccacagaatgccgccgcggccaccttccagagggccagctatgccgccggcccagcctccaattacgcggacccctaccgacagctgcagtattgtccctctgttgagtctccatacagcaaatccggccctgctctcccgcctgaaggcaccttggccaggtccccgtccattgatagcattcagaaagatcccagagaatttggatggagagacccggaactgccggaagtgattcagatgttgcagcaccagtttccctcggtccagtctaacgcggcagcctacttgcaacacctctgttttggagacaacaaaattaaagccgagataaggagacaaggaggcatccagctcctggtggacctgttggatcatcggatgaccgaagtccaccgtagtgcctgtggagctctgagaaacctggtgtatgggaaggccaacgatgataacaaaattgccctgaaaaactgtggtggcatcccagcactggtgaggttactccgcaagacgactgacctggagatccgggagctggtcacaggagtcctttggaacctctcctcatgcgatgcactcaaaatgccaatcatccaggatgccctagcagtactgaccaacgcggtgattatcccccactcaggctgggaaaattcgcctcttcaggatgatcggaaaatacagctgcattcatcacaggtgctgcgtaacgccaccgggtgcctaaggaatgttagttcggccggagaggaggcccgcagaaggatgagagagtgtgatgggcttacggatgccttgctgtacgtgatccagtctgcgctggggagcagtgagatcgatagcaagaccgttgaaaactgtgtgtgcattttaaggaacctctcgtaccggctggcggcagaaacgtctcagggacagcacatgggcacggacgagctggacgggctactctgtggcgaggccaatggcaaggatgctgagagctctgggtgctggggcaagaagaagaagaaaaagaaatcccaagatcagtgggatggagtaggacctcttccagactgtgctgaaccaccaaaagggatccagatgctgtggcacccatcaatagtcaaaccctacctcacactgctctctgagtgctcaaatccagacacgctggaaggggcggcaggcgccctgcagaacttggctgcagggagctggaagtggtcagtatatatccgagccgctgtccgaaaagagaaaggcctgcccatcctcgtggagctgctccgaatagacaatgaccgtgtggtgtgcgcggtggccactgcgctgcggaacatggccttggacgtcagaaataaggagctcatcggcaaatacgccatgcgagacctagtccacaggcttccaggagggaacaacagcaacaacactgcaagcaaggccatgtcggatgacacagtgacagctgtctgctgcacactgcacgaagtgattaccaagaacatggagaacgccaaggccttacgggatgccggtggcatcgagaagttggtcggcatctccaaaagcaaaggagataaacactctccaaaagtggtcaaggctgcatctcaggtcctcaacagcatgtggcagtaccgagatctgaggagtctctacaaaaaggatggatggtcacaataccactttgtagcctcgtcttcaaccatcgagagggaccggcaaaggccctactcctcctcccgcacgccctccatctcccctgtgcgcgtgtctcccaacaaccgctcagcaagtgccccagcttcacctcgggaaatgatcagcctcaaagaaaggaaaacagactacgagtgcaccggcagcaacgccacctaccacggagctaaaggcgaacacacttccaggaaagatgccatgacagctcaaaacactggaatttcaactttgtataggaattcttatggtgcgcccgctgaagacatcaaacacaaccaggtttcagcacagccagtcccacaggagcccagcagaaaagattacgagacctaccagccatttcagaattccacaagaaattacgatgagtccttcttcgaggaccaggtccaccatcgccctcccgccagcgagtacaccatgcacctgggtctcaagtccaccggcaactacgttgacttctactcagctgcccgtccctacagtgaactgaactatgaaacgagccactacccggcctcccccgactcctgggtgtgaggagcagggcacaggcgctccgggaacagtgcatgtgcatgcataccacaagacatttctttctgttttgtttttttctcctgcaaatttagtttgttaaagcctgttccataggaaggctgtgataaccagtaaggaaatattaagagctattttagaaagctaaatgaatcgcaagttaacttggaaatcagtagaaagctaaagtgatcctaaatatgacagtgggcagcacctttctagcgtgagctgtagagtaacgagaagtgctttatactgaacgtggttgatgggaggagagacgaggcattcgggccggtggggcgtaagggttatcgttaagcacaagacacagaatagtttacacactgtgtgggggacggcttctcacgctttgtttactctcttcatccgttgtgactctaggcttcaggttgcattggggttcctctgtacagcaagatgtttcttgccttttgttaatgcattgttgtaaagtatttgatgtacattacagattaaagaagaaaagcgcgttgtgtatattacaccaatgccgccgtgtttcctcatctatggttctaaatattgcttcaatttcaaacttttgaaagatgtatggatttccagtttttctttactttctcccagtatgttttaacaaaaaaaaaaaaaagcaggaaaaaaggaatatttagcagtattgttcgttctgatatgtgaatttgtttgtgacaactaaacaaggcattcagcagtttctgacaattaacatacatcattccacactccttgtcaacaaagtgctttttcactgcctaaaattttagatgtagatatttgaaatagattttttcatttataccagttttctttatgatgatacagtgttaaaagaaaataaattacaattgatctgtcatccatatttgctaagaatgtctatttccaagaacctatatcttacaaaatacacattcttgcttgtgtgtctgtgtgtgtgggtgtatgtatgtccacgtactagaaaaattacctgtgtgagattttattttgacagaagctatttcatttgctgttcatcttgtacaaactttgtttttggttttttagtataaatgtacatcagtttgttccttttgtactgtatctattcttctgaccatctagtgactcaggatattaggccagttgaagtggagttataggattttcacacattcacgcatacttggatatcaaccctctctacaggtccgtttccttacacattttatcccctcagaacacgataaaccatggccaattcagtttcactttggggccaattacttgaagtatccacagaaaatgtaaactgctcgccttattcccccaaactttttgttcatgtggcagggagcagtacacaactatggaatagattattaaaactgaacttgaagctaacgttagaatagtggttaacagagctaagaaataaggctaaccatcgaaaagaacatgggccgcgggtaaactagctttgctctttagatgcaagtggctgaggccaataggtgcctagtaaatgttaactgttcttggaaaaaataaaaacatcagtaacaaaa

SEQ ID NO: 52 - RNA, 5289 nt, Homo sapiens
  source 1..5289: mol_type = mRNA
gttccttttagccgtggtgcagggagggaggagggaggtgggtaggatgccaggaaccgcctgctccacagcctggggaaggagggaagagtaacccttcatctttgggactagtcgtcttgtttgcctagactacagttttcaagtatttaaggaccatttatttcaaaaggaattacagtttgaaaggctgacccgagagctggaggctgaacggcagatcgtagccagccagctggagcgatgcaagctcggatccgagactggcagcatgagcagcatgagttcagcagaagagcagtttcagtggcagtcacaagatggtcaaaaagatatcgaagatgagcttacaacaggtctcgagctggtggactcctgtattaggtcactacaggaatcaggaatacttgacccacaggattattctacaggtgaaaggcccagcctgctctcccagagtgcacttcagctcaattccaaacctgaagggtctttccagtatccggccagctaccatagcaaccagaccctggccctgggggaaaccaccccttcacagctcccggcccgaggcacacaagcccgagctacgggccagagcttcagccagggcacgaccagccgcgccggccacctggcggggcccgagcccgcgccgccgccgccgccgccgccgcgggagccgttcgcgcccagcctgggcagcgccttccacctgcccgacgcgccgcccgccgccgccgccgccgcgctctactactccagctccacgctgcccgcgccgccgcgcgggggctccccgctggccgcgccccagggcggttcgcccaccaagctgcagcgcggcggctcggcccccgagggcgccacctacgccgcgccgcgcggctcctcgcccaagcagtcgcccagccgcctggccaagtcctacagcaccagctcgcccatcaacatcgtcgtgtcctcggccggcctgtccccgatccgcgtgacctcgccccccaccgtgcagtccaccatctcctcctcgcccatccaccagctgagctccaccatcggcacgtacgccaccctgtcgcccaccaagcgcctggtccacgcgtccgagcagtacagcaagcactcgcaggagctgtatgccacggccaccctccagaggccgggcagcctggcagctggttcccgagcctcatacagcagccagcatgggcacctgggcccagagttgcgggccctgcagtccccagaacaccacatagatcccatctatgaagaccgcgtctatcagaagccccctatgaggagtctcagccagagccagggggaccctctgccgccagcacacaccggcacctaccgcacgagcacagccccatcttcccctggtgtcgactccgtccccttgcagcgcacaggcagccagcacggcccacagaatgccgccgcggccaccttccagagggccagctatgccgccggcccagcctccaattacgcggacccctaccgacagctgcagtattgtccctctgttgagtctccatacagcaaatccggccctgctctcccgcctgaaggcaccttggccaggtccccgtccattgatagcattcagaaagatcccagagaatttggatggagagacccggaactgccggaagtgattcagatgttgcagcaccagtttccctcggtccagtctaacgcggcagcctacttgcaacacctctgttttggagacaacaaaattaaagccgagataaggagacaaggaggcatccagctcctggtggacctgttggatcatcggatgaccgaagtccaccgtagtgcctgtggagctctgagaaacctggtgtatgggaaggccaacgatgataacaaaattgccctgaaaaactgtggtggcatcccagcactggtgaggttactccgcaagacgactgacctggagatccgggagctggtcacaggagtcctttggaacctctcctcatgcgatgcactcaaaatgccaatcatccaggatgccctagcagtactgaccaacgcggtgattatcccccactcaggctgggaaaattcgcctcttcaggatgatcggaaaatacagctgcattcatcacaggtgctgcgtaacgccaccgggtgcctaaggaatgttagttcggccggagaggaggcccgcagaaggatgagagagtgtgatgggcttacggatgccttgctgtacgtgatccagtctgcgctggggagcagtgagatcgatagcaagaccgttgaaaactgtgtgtgcattttaaggaacctctcgtaccggctggcggcagaaacgtctcagggacagcacatgggcacggacgagctggacgggctactctgtggcgaggccaatggcaaggatgctgagagctctgggtgctggggcaagaagaagaagaaaaagaaatcccaagatcagtgggatggagtaggacctcttccagactgtgctgaaccaccaaaagggatccagatgctgtggcacccatcaatagtcaaaccctacctcacactgctctctgagtgctcaaatccagacacgctggaaggggcggcaggcgccctgcagaacttggctgcagggagctggaagtggtcagtatatatccgagccgctgtccgaaaagagaaaggcctgcccatcctcgtggagctgctccgaatagacaatgaccgtgtggtgtgcgcggtggccactgcgctgcggaacatggccttggacgtcagaaataaggagctcatcggcaaatacgccatgcgagacctagtccacaggcttccaggagggaacaacagcaacaacactgcaagcaaggccatgtcggatgacacagtgacagctgtctgctgcacactgcacgaagtgattaccaagaacatggagaacgccaaggccttacgggatgccggtggcatcgagaagttggtcggcatctccaaaagcaaaggagataaacactctccaaaagtggtcaaggctgcatctcaggtcctcaacagcatgtggcagtaccgagatctgaggagtctctacaaaaaggatggatggtcacaataccactttgtagcctcgtcttcaaccatcgagagggaccggcaaaggccctactcctcctcccgcacgccctccatctcccctgtgcgcgtgtctcccaacaaccgctcagcaagtgccccagcttcacctcgggaaatgatcagcctcaaagaaaggaaaacagactacgagtgcaccggcagcaacgccacctaccacggagctaaaggcgaacacacttccaggaaagatgccatgacagctcaaaacactggaatttcaactttgtataggaattcttatggtgcgcccgctgaagacatcaaacacaaccaggtttcagcacagccagtcccacaggagcccagcagaaaagattacgagacctaccagccatttcagaattccacaagaaattacgatgagtccttcttcgaggaccaggtccaccatcgccctcccgccagcgagtacaccatgcacctgggtctcaagtccaccggcaactacgttgacttctactcagctgcccgtccctacagtgaactgaactatgaaacgagccactacccggcctcccccgactcctgggtgtgaggagcagggcacaggcgctccgggaacagtgcatgtgcatgcataccacaagacatttctttctgttttgtttttttctcctgcaaatttagtttgttaaagcctgttccataggaaggctgtgataaccagtaaggaaatattaagagctattttagaaagctaaatgaatcgcaagttaacttggaaatcagtagaaagctaaagtgatcctaaatatgacagtgggcagcacctttctagcgtgagctgtagagtaacgagaagtgctttatactgaacgtggttgatgggaggagagacgaggcattcgggccggtggggcgtaagggttatcgttaagcacaagacacagaatagtttacacactgtgtgggggacggcttctcacgctttgtttactctcttcatccgttgtgactctaggcttcaggttgcattggggttcctctgtacagcaagatgtttcttgccttttgttaatgcattgttgtaaagtatttgatgtacattacagattaaagaagaaaagcgcgttgtgtatattacaccaatgccgccgtgtttcctcatctatggttctaaatattgcttcaatttcaaacttttgaaagatgtatggatttccagtttttctttactttctcccagtatgttttaacaaaaaaaaaaaaaagcaggaaaaaaggaatatttagcagtattgttcgttctgatatgtgaatttgtttgtgacaactaaacaaggcattcagcagtttctgacaattaacatacatcattccacactccttgtcaacaaagtgctttttcactgcctaaaattttagatgtagatatttgaaatagattttttcatttataccagttttctttatgatgatacagtgttaaaagaaaataaattacaattgatctgtcatccatatttgctaagaatgtctatttccaagaacctatatcttacaaaatacacattcttgcttgtgtgtctgtgtgtgtgggtgtatgtatgtccacgtactagaaaaattacctgtgtgagattttattttgacagaagctatttcatttgctgttcatcttgtacaaactttgtttttggttttttagtataaatgtacatcagtttgttccttttgtactgtatctattcttctgaccatctagtgactcaggatattaggccagttgaagtggagttataggattttcacacattcacgcatacttggatatcaaccctctctacaggtccgtttccttacacattttatcccctcagaacacgataaaccatggccaattcagtttcactttggggccaattacttgaagtatccacagaaaatgtaaactgctcgccttattcccccaaactttttgttcatgtggcagggagcagtacacaactatggaatagattattaaaactgaacttgaagctaacgttagaatagtggttaacagagctaagaaataaggctaaccatcgaaaagaacatgggccgcgggtaaactagctttgctctttagatgcaagtggctgaggccaataggtgcctagtaaatgttaactgttcttggaaaaaataaaaacatcagtaacaaaa

SEQ ID NO: 53 - RNA, 4551 nt, Homo sapiens
  source 1..4551: mol_type = mRNA
gttccttttagccgtggtgcagggagggaggagggaggtgggtaggatgccaggaaccgcctgctccacagcctggggaaggagggaagagtaacccttcatctttgggactagtcgtcttgtttgcctagactacagttttcaagtatttaaggaccatttatttcaaaaggaattacagtttgaaaggctgacccgagagctggaggctgaacggcagatcgtagccagccagctggagcgatgcaagctcggatccgagactggcagcatgagcagcatgagttcagcagaagagcagtttcagtggcagtcacaagatggtcaaaaagatatcgaagatgagcttacaacaggtctcgagctggtggactcctgtattaggtcactacaggaatcaggaatacttgacccacaggattattctacaggtgaaactggttcccgagcctcatacagcagccagcatgggcacctgggcccagagttgcgggccctgcagtccccagaacaccacatagatcccatctatgaagaccgcgtctatcagaagccccctatgaggagtctcagccagagccagggggaccctctgccgccagcacacaccggcacctaccgcacgagcacagccccatcttcccctggtgtcgactccgtccccttgcagcgcacaggcagccagcacggcccacagaatgccgccgcggccaccttccagagggccagctatgccgccggcccagcctccaattacgcggacccctaccgacagctgcagtattgtccctctgttgagtctccatacagcaaatccggccctgctctcccgcctgaaggcaccttggccaggtccccgtccattgatagcattcagaaagatcccagagaatttggatggagagacccggaactgccggaagtgattcagatgttgcagcaccagtttccctcggtccagtctaacgcggcagcctacttgcaacacctctgttttggagacaacaaaattaaagccgagataaggagacaaggaggcatccagctcctggtggacctgttggatcatcggatgaccgaagtccaccgtagtgcctgtggagctctgagaaacctggtgtatgggaaggccaacgatgataacaaaattgccctgaaaaactgtggtggcatcccagcactggtgaggttactccgcaagacgactgacctggagatccgggagctggtcacaggagtcctttggaacctctcctcatgcgatgcactcaaaatgccaatcatccaggatgccctagcagtactgaccaacgcggtgattatcccccactcaggctgggaaaattcgcctcttcaggatgatcggaaaatacagctgcattcatcacaggtgctgcgtaacgccaccgggtgcctaaggaatgttagttcggccggagaggaggcccgcagaaggatgagagagtgtgatgggcttacggatgccttgctgtacgtgatccagtctgcgctggggagcagtgagatcgatagcaagaccgttgaaaactgtgtgtgcattttaaggaacctctcgtaccggctggcggcagaaacgtctcagggacagcacatgggcacggacgagctggacgggctactctgtggcgaggccaatggcaaggatgctgagagctctgggtgctggggcaagaagaagaagaaaaagaaatcccaagatcagtgggatggagtaggacctcttccagactgtgctgaaccaccaaaagggatccagatgctgtggcacccatcaatagtcaaaccctacctcacactgctctctgagtgctcaaatccagacacgctggaaggggcggcaggcgccctgcagaacttggctgcagggagctggaagtggtcagtatatatccgagccgctgtccgaaaagagaaaggcctgcccatcctcgtggagctgctccgaatagacaatgaccgtgtggtgtgcgcggtggccactgcgctgcggaacatggccttggacgtcagaaataaggagctcatcggcaaatacgccatgcgagacctagtccacaggcttccaggagggaacaacagcaacaacactgcaagcaaggccatgtcggatgacacagtgacagctgtctgctgcacactgcacgaagtgattaccaagaacatggagaacgccaaggccttacgggatgccggtggcatcgagaagttggtcggcatctccaaaagcaaaggagataaacactctccaaaagtggtcaaggctgcatctcaggtcctcaacagcatgtggcagtaccgagatctgaggagtctctacaaaaaggatggatggtcacaataccactttgtagcctcgtcttcaaccatcgagagggaccggcaaaggccctactcctcctcccgcacgccctccatctcccctgtgcgcgtgtctcccaacaaccgctcagcaagtgccccagcttcacctcgggaaatgatcagcctcaaagaaaggaaaacagactacgagtgcaccggcagcaacgccacctaccacggagctaaaggcgaacacacttccaggaaagatgccatgacagctcaaaacactggaatttcaactttgtataggaattcttatggtgcgcccgctgaagacatcaaacacaaccaggtttcagcacagccagtcccacaggagcccagcagaaaagattacgagacctaccagccatttcagaattccacaagaaattacgatgagtccttcttcgaggaccaggtccaccatcgccctcccgccagcgagtacaccatgcacctgggtctcaagtccaccggcaactacgttgacttctactcagctgcccgtccctacagtgaactgaactatgaaacgagccactacccggcctcccccgactcctgggtgtgaggagcagggcacaggcgctccgggaacagtgcatgtgcatgcataccacaagacatttctttctgttttgtttttttctcctgcaaatttagtttgttaaagcctgttccataggaaggctgtgataaccagtaaggaaatattaagagctattttagaaagctaaatgaatcgcaagttaacttggaaatcagtagaaagctaaagtgatcctaaatatgacagtgggcagcacctttctagcgtgagctgtagagtaacgagaagtgctttatactgaacgtggttgatgggaggagagacgaggcattcgggccggtggggcgtaagggttatcgttaagcacaagacacagaatagtttacacactgtgtgggggacggcttctcacgctttgtttactctcttcatccgttgtgactctaggcttcaggttgcattggggttcctctgtacagcaagatgtttcttgccttttgttaatgcattgttgtaaagtatttgatgtacattacagattaaagaagaaaagcgcgttgtgtatattacaccaatgccgccgtgtttcctcatctatggttctaaatattgcttcaatttcaaacttttgaaagatgtatggatttccagtttttctttactttctcccagtatgttttaacaaaaaaaaaaaaaagcaggaaaaaaggaatatttagcagtattgttcgttctgatatgtgaatttgtttgtgacaactaaacaaggcattcagcagtttctgacaattaacatacatcattccacactccttgtcaacaaagtgctttttcactgcctaaaattttagatgtagatatttgaaatagattttttcatttataccagttttctttatgatgatacagtgttaaaagaaaataaattacaattgatctgtcatccatatttgctaagaatgtctatttccaagaacctatatcttacaaaatacacattcttgcttgtgtgtctgtgtgtgtgggtgtatgtatgtccacgtactagaaaaattacctgtgtgagattttattttgacagaagctatttcatttgctgttcatcttgtacaaactttgtttttggttttttagtataaatgtacatcagtttgttccttttgtactgtatctattcttctgaccatctagtgactcaggatattaggccagttgaagtggagttataggattttcacacattcacgcatacttggatatcaaccctctctacaggtccgtttccttacacattttatcccctcagaacacgataaaccatggccaattcagtttcactttggggccaattacttgaagtatccacagaaaatgtaaactgctcgccttattcccccaaactttttgttcatgtggcagggagcagtacacaactatggaatagattattaaaactgaacttgaagctaacgttagaatagtggttaacagagctaagaaataaggctaaccatcgaaaagaacatgggccgcgggtaaactagctttgctctttagatgcaagtggctgaggccaataggtgcctagtaaatgttaactgttcttggaaaaaataaaaacatcagtaacaaaa

SEQ ID NO: 54 - RNA, 4916 nt, Homo sapiens
  source 1..4916: mol_type = mRNA
gcgtcgggagccgcctctcgcccgcggcgctcgcccctgccgcccgccagcatcccttgtcccgcggccgcgctcagacaacaaaagcggaagatgctgcagttgggcaaggtcaggaccttgccctgaagccgggcggcgccgcgcacgcctcttcccggactgaggagctgtcgccggcggagggtgcatgtttgcgaggaagccgccgggcgccgcgcctttgggagctatgcctgttccagaccagccttcatcagcctcagagaagacgagttccctgagccccggcttaaacacctccaacggggatggctctgaaacagaaaccacctctgccatcctcgcctcagtcaaagaacaggaattacagtttgaaaggctgacccgagagctggaggctgaacggcagatcgtagccagccagctggagcgatgcaagctcggatccgagactggcagcatgagcagcatgagttcagcagaagagcagtttcagtggcagtcacaagatggtcaaaaagatatcgaagatgagcttacaacaggtctcgagctggtggactcctgtattaggtcactacaggaatcaggaatacttgacccacaggattattctacaggtgaaaggcccagcctgctctcccagagtgcacttcagctcaattccaaacctgaagggtctttccagtatccggccagctaccatagcaaccagaccctggccctgggggaaaccaccccttcacagctcccggcccgaggcacacaagcccgagctacgggccagagcttcagccagctggttcccgagcctcatacagcagccagcatgggcacctgggcccagagttgcgggccctgcagtccccagaacaccacatagatcccatctatgaagaccgcgtctatcagaagccccctatgaggagtctcagccagagccagggggaccctctgccgccagcacacaccggcacctaccgcacgagcacagccccatcttcccctggtgtcgactccgtccccttgcagcgcacaggcagccagcacggcccacagaatgccgccgcggccaccttccagagggccagctatgccgccggcccagcctccaattacgcggacccctaccgacagctgcagtattgtccctctgttgagtctccatacagcaaatccggccctgctctcccgcctgaaggcaccttggccaggtccccgtccattgatagcattcagaaagatcccagagaatttggatggagagacccggaactgccggaagtgattcagatgttgcagcaccagtttccctcggtccagtctaacgcggcagcctacttgcaacacctctgttttggagacaacaaaattaaagccgagataaggagacaaggaggcatccagctcctggtggacctgttggatcatcggatgaccgaagtccaccgtagtgcctgtggagctctgagaaacctggtgtatgggaaggccaacgatgataacaaaattgccctgaaaaactgtggtggcatcccagcactggtgaggttactccgcaagacgactgacctggagatccgggagctggtcacaggagtcctttggaacctctcctcatgcgatgcactcaaaatgccaatcatccaggatgccctagcagtactgaccaacgcggtgattatcccccactcaggctgggaaaattcgcctcttcaggatgatcggaaaatacagctgcattcatcacaggtgctgcgtaacgccaccgggtgcctaaggaatgttagttcggccggagaggaggcccgcagaaggatgagagagtgtgatgggcttacggatgccttgctgtacgtgatccagtctgcgctggggagcagtgagatcgatagcaagaccgttgaaaactgtgtgtgcattttaaggaacctctcgtaccggctggcggcagaaacgtctcagggacagcacatgggcacggacgagctggacgggctactctgtggcgaggccaatggcaaggatgctgagagctctgggtgctggggcaagaagaagaagaaaaagaaatcccaagatcagtgggatggagtaggacctcttccagactgtgctgaaccaccaaaagggatccagatgctgtggcacccatcaatagtcaaaccctacctcacactgctctctgagtgctcaaatccagacacgctggaaggggcggcaggcgccctgcagaacttggctgcagggagctggaagtggtcagtatatatccgagccgctgtccgaaaagagaaaggcctgcccatcctcgtggagctgctccgaatagacaatgaccgtgtggtgtgcgcggtggccactgcgctgcggaacatggccttggacgtcagaaataaggagctcatcggcaaatacgccatgcgagacctagtccacaggcttccaggagggaacaacagcaacaacactgcaagcaaggccatgtcggatgacacagtgacagctgtctgctgcacactgcacgaagtgattaccaagaacatggagaacgccaaggccttacgggatgccggtggcatcgagaagttggtcggcatctccaaaagcaaaggagataaacactctccaaaagtggtcaaggctgcatctcaggtcctcaacagcatgtggcagtaccgagatctgaggagtctctacaaaaaggatggatggtcacaataccactttgtagcctcgtcttcaaccatcgagagggaccggcaaaggccctactcctcctcccgcacgccctccatctcccctgtgcgcgtgtctcccaacaaccgctcagcaagtgccccagcttcacctcgggaaatgatcagcctcaaagaaaggaaaacagactacgagtgcaccggcagcaacgccacctaccacggagctaaaggcgaacacacttccaggaaagatgccatgacagctcaaaacactggaatttcaactttgtataggaattcttatggtgcgcccgctgaagacatcaaacacaaccaggtttcagcacagccagtcccacaggagcccagcagaaaagattacgagacctaccagccatttcagaattccacaagaaattacgatgagtccttcttcgaggaccaggtccaccatcgccctcccgccagcgagtacaccatgcacctgggtctcaagtccaccggcaactacgttgacttctactcagctgcccgtccctacagtgaactgaactatgaaacgagccactacccggcctcccccgactcctgggtgtgaggagcagggcacaggcgctccgggaacagtgcatgtgcatgcataccacaagacatttctttctgttttgtttttttctcctgcaaatttagtttgttaaagcctgttccataggaaggctgtgataaccagtaaggaaatattaagagctattttagaaagctaaatgaatcgcaagttaacttggaaatcagtagaaagctaaagtgatcctaaatatgacagtgggcagcacctttctagcgtgagctgtagagtaacgagaagtgctttatactgaacgtggttgatgggaggagagacgaggcattcgggccggtggggcgtaagggttatcgttaagcacaagacacagaatagtttacacactgtgtgggggacggcttctcacgctttgtttactctcttcatccgttgtgactctaggcttcaggttgcattggggttcctctgtacagcaagatgtttcttgccttttgttaatgcattgttgtaaagtatttgatgtacattacagattaaagaagaaaagcgcgttgtgtatattacaccaatgccgccgtgtttcctcatctatggttctaaatattgcttcaatttcaaacttttgaaagatgtatggatttccagtttttctttactttctcccagtatgttttaacaaaaaaaaaaaaaagcaggaaaaaaggaatatttagcagtattgttcgttctgatatgtgaatttgtttgtgacaactaaacaaggcattcagcagtttctgacaattaacatacatcattccacactccttgtcaacaaagtgctttttcactgcctaaaattttagatgtagatatttgaaatagattttttcatttataccagttttctttatgatgatacagtgttaaaagaaaataaattacaattgatctgtcatccatatttgctaagaatgtctatttccaagaacctatatcttacaaaatacacattcttgcttgtgtgtctgtgtgtgtgggtgtatgtatgtccacgtactagaaaaattacctgtgtgagattttattttgacagaagctatttcatttgctgttcatcttgtacaaactttgtttttggttttttagtataaatgtacatcagtttgttccttttgtactgtatctattcttctgaccatctagtgactcaggatattaggccagttgaagtggagttataggattttcacacattcacgcatacttggatatcaaccctctctacaggtccgtttccttacacattttatcccctcagaacacgataaaccatggccaattcagtttcactttggggccaattacttgaagtatccacagaaaatgtaaactgctcgccttattcccccaaactttttgttcatgtggcagggagcagtacacaactatggaatagattattaaaactgaacttgaagctaacgttagaatagtggttaacagagctaagaaataaggctaaccatcgaaaagaacatgggccgcgggtaaactagctttgctctttagatgcaagtggctgaggccaataggtgcctagtaaatgttaactgttcttggaaaaaataaaaacatcagtaacaaaa

SEQ ID NO: 55 - protein, 1322 aa, Homo sapiens
MDVFSFVKIAKLSSHRTKSSGWPPPSGTWGLSQVPPYGWEMTANRDGRDYFINHMTQAIPFDDPRLESCQIIPPAPRKVEMRRDPVLGFGFVAGSEKPVVVRSVTPGGPSEGKLIPGDQIVMINDEPVSAAPRERVIDLVRSCKESILLTVIQPYPSPKSAFISAAKKARLKSNPVKVRFSEEVIINGQVSETVKDNSLLFMPNVLKVYLENGQTKSFRFDCSTSIKDVILTLQEKLSIKGIEHFSLMLEQRTEGAGTKLLLLHEQETLTQVTQRPSSHKMRCLFRISFVPKDPIDLLRRDPVAFEYLYVQSCNDVVQERFGPELKYDIALRLAALQMYIATVTTKQTQKISLKYIEKEWGLETFLPSAVLQSMKEKNIKKALSHLVKANQNLVPPGKKLSALQAKVHYLKFLSDLRLYGGRVFKATLVQAEKRSEVTLLVGPRYGISHVINTKTNLVALLADFSHVNRIEMFSEEESLVRVELHVLDVKPITLLMESSDAMNLACLTAGYYRLLVDSRRSIFNMANKKNTATQETGPENKGKHNLLGPDWNCIPQMTTFIGEGEQEAQITYIDSKQKTVEITDSTMCPKEHRHLYIDNAYSSDGLNQQLSQPGEAPCEADYRSLAQRSLLTLSGPETLKKAQESPRGAKVSFIFGDFALDDGISPPTLGYETLLDEGPEMLEKQRNLYIGSANDMKGLDLTPEAEGIQFVENSVYANIGDVKSFQAAEGIEEPLLHDICYAENTDDAEDEDEVSCEEDLVVGEMNQPAILNLSGSSDDIIDLTSLPPPEGDDNEDDFLLRSLNMAIAAPPPGFRDSSDEEDSQSQAASFPEDKEKGSSLQNDEIPVSLIDAVPTSAEGKCEKGLDNAVVSTLGALEALSVSEEQQTSDNSGVAILRAYSPESSSDSGNETNSSEMTESSELATAQKQSENLSRMFLATHEGYHPLAEEQTEFPASKTPAGGLPPKSSHALAARPATDLPPKVVPSKQLLHSDHMEMEPETMETKSVTDYFSKLHMGSVAYSCTSKRKSKLADGEGKAPPNGNTTGKKQQGTKTAEMEEEASGKFGTVSSRDSQHLSTFNLERTAFRKDSQRWYVATEGGMAEKSGLEAATGKTFPRASGLGAREAEGKEEGAPDGETSDGSGLGQGDRFLTDVTCASSAKDLDNPEDADSSTCDHPSKLPEADESVARLCDYHLAKRMSSLQSEGHFSLQSSQGSSVDAGCGTGSSGSACATPVESPLCPSLGKHLIPDASGKGVNYIPSEERAPGLPNHGATFKELHPQTEGMCPRMTVPALHTAINTEPLFGTLRDGCHRLPKIKETTV

SEQ ID NO: 56 - RNA, 8477 nt, Homo sapiens
  source 1..8477: mol_type = mRNA
gggaggcagctgcagtgctgcgaggggtgcgtgcgcgtgtgcccagctcgcctgccgtctcccggctccgtctgcgctcctcggtgcgtggggcacgagggtccgagggccgggaagccagagcagcgcctctcgcccaggcctcgctttctctggacgcccggcagtccccggggctagagcgcacggggcggggcgcgagacccgggccgcgctccccgcccccgcctcttgcgccctgcctggctccctctccattgagttttcctgcctcgggtgcctatcaatggtcctgctcggggatgcacacgcagctcgcggccggaggggggtagcagccgccgcctccaggtgcaggttctctccggccgccgccgccacccgctgtcgccgcgactcgagccccgggcgcactgaggtcttggccatggggctgcggaggctgctgttgctggcgtgagaaggggcgacggagttgtcgcgctcgggggtccccagctgcctgcatggatgtcttcagctttgtgaagattgcaaagctttcgagccacaggacgaagtcttcaggctggccgcctccctcgggaacctggggcttgagccaggtgccgccctatggatgggagatgacggcaaaccgagatgggcgagactacttcatcaatcacatgacacaggcaatcccttttgacgaccctcggttagagagctgccaaatcatccctccggctcctcggaaggtggagatgagaagggaccccgtgctgggatttggttttgtggcaggcagtgaaaagccagtggtcgttcgctcagtaacaccaggtggcccctctgaaggcaagctgatcccgggagatcagattgtaatgattaatgatgaaccggtcagcgctgcacccagagagcgggtcatcgatctggtcagaagctgcaaagaatcgatactcctcactgtcattcagccttacccttctcccaaatcagcatttattagtgctgcaaaaaaggcaagattaaagtccaatcctgtcaaagtacgcttctctgaggaggtcatcatcaacggccaagtgtcggaaactgttaaggacaactcacttctttttatgccaaatgttttgaaagtctatctggaaaatgggcagaccaaatcatttcgttttgactgcagcacttccattaaggatgtcatcttaacccttcaagagaagctctccatcaaaggcattgaacacttctctctcatgctggagcagaggacagaaggggctggaacgaagctgctcttgcttcatgaacaggagactctaactcaggtgacacagaggcccagctcccataagatgagatgtcttttccgaattagcttcgtcccaaaagatccaattgaccttttaaggagagatccagttgctttcgagtatctctatgttcagagttgtaacgatgtggttcaggagcgatttgggccggagctgaaatatgacatagccctgcggctggccgcattacaaatgtacattgcaaccgttaccaccaagcaaacgcagaaaatctccctcaaatacatcgaaaaagaatggggattagagacttttcttccctctgctgtgctgcaaagcatgaaagagaagaacataaagaaagcactttcacaccttgtcaaagcaaatcaaaacttggtaccaccgggtaaaaagctctctgcactacaagccaaggtccattatctcaagttcctcagtgacctacgattgtatgggggccgtgtgttcaaggcaacattagtgcaggcagaaaagcgctcggaagtgactctcctggttgggccccggtatggcataagccatgtcatcaacaccaaaaccaatctggtggctcttttagccgactttagccacgtcaacaggatcgaaatgttttccgaggaggagagcttggtgcgggtagaactccacgtgctagatgtgaagcctatcacgcttctgatggaatcctcagatgccatgaacctggcctgcttgacggctggatactaccggctgcttgttgattccaggaggtcgatatttaacatggccaacaagaaaaacacagcgacccaggaaacaggacctgaaaacaaggggaagcataacctccttggcccagattggaactgtataccccaaatgaccacctttattggcgaaggggaacaagaagcccagataacatacatagattcaaagcagaagacggtggagatcacagacagcaccatgtgtccaaaagagcaccggcacttgtacatagacaatgcctatagttcagatggacttaaccagcagctgagccagcccggggaggccccctgtgaggcagactacagaagtctagctcagcggtccctattgaccctctcaggaccagaaactctgaagaaagcacaggaatctccgagaggagctaaagtgtcctttatttttggagacttcgccttggatgatggtattagtcccccaacccttggctatgaaacgctactagatgagggtcctgaaatgctggagaagcagagaaatctctacattggcagtgccaatgacatgaagggcctggatctcactccagaggcagagggcatccagtttgtggaaaattctgtttatgcaaacataggcgatgtgaagagcttccaggccgcggaggggatcgaggaacccctcttgcatgacatctgttatgcagaaaacactgatgacgcggaggacgaggacgaggtgagctgcgaggaggacctcgtggtgggggagatgaaccagccggccatcctcaacctgtctgggtcaagcgatgacatcattgacctcacatccctgccccctccagaaggtgatgacaatgaggatgacttcctgttgcgttccttgaacatggccattgccgcacccccacctggctttagagacagttcagatgaagaggactctcagagccaggcagcttccttccccgaggacaaggagaaaggcagcagcctgcaaaatgatgagatccccgtgtccctcattgacgctgtgcccaccagcgccgaaggcaagtgtgagaagggactggataatgccgtcgtctccacgctgggagctctagaggctctatccgtgtcagaagaacagcagaccagtgacaattcaggtgtagccatcttgcgggcttatagtcctgagtcttcgtcagactcgggcaatgaaactaactcttctgaaatgactgagagttctgaactggccacagcacaaaaacagtcagaaaacctctcccgcatgttcttggccactcacgaaggctaccacccccttgcagaagagcagaccgagttcccggcctccaagacccccgctgggggcttgcctccaaagtcctcgcacgccctggctgctaggccagcaaccgacctcccgcccaaagttgtgccttccaagcagttacttcactcagaccacatggagatggagcctgaaactatggagactaagtcggtcactgactattttagcaaactgcacatggggtcggtggcatactcctgcactagcaaaaggaaaagcaagctggccgatggtgaggggaaggcaccccctaatgggaacacaacaggaaaaaaacagcaggggaccaaaacggcagagatggaggaggaggccagtggtaaatttggtactgtgtcttcacgagacagtcaacacctgagcacttttaatctggagagaactgcctttcgcaaggacagtcaaagatggtatgtggccactgaaggtgggatggctgaaaaaagtggattagaagcagcaacagggaaaacctttccaagagcttctggtcttggggcaagggaggccgaagggaaggaagaaggagctcctgatggagaaaccagtgatggctcaggacttggtcaaggggaccgcttcttaactgacgtgacctgtgcatcttcagccaaagacttagataacccagaggacgctgactcgtccacctgcgaccatccttccaagcttcctgaggctgatgagagtgtggcccgcctttgtgactaccacttggccaagcggatgtcatcactgcaaagcgagggccatttttctctgcagagctcccaaggctcttcagtggatgcaggctgtggcacaggcagcagtggcagtgcctgtgccacacccgtggagtcgccgctctgcccctccctggggaagcacttgattcctgacgcttctgggaaaggcgtgaattacattccttcagaggagagagcccctgggcttcccaaccacggagccacctttaaggaactgcacccacagacagaagggatgtgtccacggatgacagtgcctgctctgcacacagccattaacaccgaacccctgtttggcacattgagagatggatgccatcggctccccaagattaaggaaaccacagtgtagctttgacagagcctgggaaggagagacgaggaggcatgccttcagcttggtctcaacatcctgaagctgatcccatcctgctaccatcaaacattcactcggaatcaaaggtgccaattccaaatcaagaccctaatgatttctcccaagcaaatcaggcatacggagaggctgtgagctggcggccaccggatctgagaggggggagcctcaggacacctcccagccagaaggctctgagacatagcagcagtatcctctccggatctgtcgatttggagaccttccgagagagaaccaagggtgcagtcagcttaaagtgtccaggcatcacagaagcacaggaggccagttctgaaaggcgagcagaactccccctggggaggaagctcaccaaaagtttttcccaaagctcaatgcacttgagctctgaggggaggtttcacaaaaggtccccagtggctcataaagactcaaagctgtataggacattacccttgcggaagctggagggcagcaattggagatgccggggacccttcagctattgcttcctgaaccgagggcaggatgaagatggtgaggaagaagaggagaggggagaggccaccgtccaggtctcttgcctctatagaccacagatgactcaagccatgccagaaccaagcagcccatgcctggctgtggcgattcagaagcaacgaggggagctatccagagggtcagtgctgaaggtctgggcagaagacctgcgagacccagatgacttggacttcagcaacctggcttttgatgcccggattgcaagaataaatgccctaaaggagagcacatatgcaatgcctgatgggttccttgcagcccaaaatgatgccaatgagctgctctgtctcgtcagggcaaccaaggagaagagggaggagtcacgccctgaagcgtacgaccttacactttctcagtacaagcaactgttatccattgagtccagacagttgggaagtgcctgtaggaaaatggcgatggctgagaaaagcccggaggagatgctcctagctatgacttccagctttcaagtgctctgttgcctaacagaagcttgcatgcgattagttaaagtcgtgaactcagaaacacagcggcaggaaattgtagggaagatcgatgaagtggtcataaattacatttgtctactgaaagctgccgaagcagccactggaaagaaccctggggaccctaatgttggactctcggcgcgacactcaaccaccatggccgctctcgtaagcacactgacacgttctctcaagaggcttttaaacaaataaatatggaagtcacgtcataatctacctttgcaaagccatacatgaacttttatttactttgtgtgtatgatgaacagatgtctcctttcttctctctgtatattttgttattttatataaaataggagataaaagtcacattgatgaaatgttgaaatgtactaatcagatgtattctgtttatattatacatatatatacacgtaaaagaaatatccaagaaagtgatgacatttggctatttttcatatagttaaaactccaggtatatgatgtgaaattttaaattctaccatgttagagcaaaacaatgaatcctatcccctttctttccaagtagctacttggaaaccatatcattcatatttagaagtaaaacacaaaacaaaaaagagagagaaaagaaaagaaatcacaatgtatataaaacagtacttatgttttaaaattatgatttttaagcattggaaatagcaaaaagacatttaaaattcaagaagctattatgaattactagagaatatatctgtaataaattaattttttgctcatagtatttggttactggatgctttcttccaagaatcccacatatttaatttgggtttttgctactggggctacaaattggtggggatggattctactgtgtcagcacaaatgctcttcacagtggttctagcatttaaaaaacttcccggggagaagaacagaggggatgatgggcagtttcctaggtaacacctagagttatagaatatctcattacataaaatgtatggaattaataataccaaaattaattatttgatggaaagatctgctttgactaaatgtcaaaaatctgcaaaccaaagacattatcttcccctcatcccaactcaactacgaaacttaaaattccctttagagtgataggacatttagtaaagtatttgcaaacttaaaaaaaggaacatttaatgatcatcaaaattaagtacagattcagtaatgtagaccagaccacacaccagcacctgtgagtctcatctcagatcacagctctcagcatagggcttcatgcatcaccgcctctacagaggctaaggctgccagtcaaatttggaattatagcgtagtactgggacaaaatctcaaatcttggatgttccagaaaatcagggagagatggctactgtaatcatgggagccatgagtaaatagttaagtatttattaaataaatacttaatctggattggctgataaaaatatgaaatctgaaaaaaaaaagaaagaaatggaagtggtatatttgaccagttcaagtgaaaccaatggaatgcaaagaactttccaggactgtcacatctctaaaagtaccctgcagtcataaaataaaatcgatatgtatatatgtatttcctgggtcattcagtgctcaagttacatgcactcctacttagacaggtggctccttaagaacatgatgggagtacaccaggtgcaaatatttctacttttgtagcctgctgagaaggagtcataacacagtccacaattgcaatctctctctagtcagccattccacagggactcaacaacaaaagccgcacgtggttatggatggcagcaaaggaaaggagtttaggtgtgtgttattataaataatgtttaactaaataataaaacattatttcattacaattataattataaatattggtgttttgatattgagagatattagtggtgtttactgtggaaaatcttagtaaatatcattctgtgtactaaaatcctaacctattaataggatgtgtgccctatgtcagacagtgtgctaagcatattaactatattatctcatttaatcatcacaacaatctgctggtttggacactattctctctggaggcaatatggatgagttcttacggatatggggtttggggtcagaaacatcttgattaaaattttgactctgccattttctagcccttttatgttgggaaagctactttttctagtctcaatttcctcataataaaatgaaaatcaattataagatcgatttccatagggttgtcatgagttttgagtaaaaatgtgtatgtaaagttcttaccacaatacctggcagagagtaagtattcaattaatgttagctattattatcatcataatcgttgtgttaaatatattgcccaagataatatgtgggggaatgtttgttttatatgcatattgtatcctgactgtgtgcagaacacattatgtgtattgcatatatgtaaaagaagtgtacaaggaagtggccatccttgttcaagttacgtatctagttagaacaacttcccagtccattggagttctttgagaagcctcagggaagtagctctgggtccttctaatcaacctcccattactgcgccagtaagtttctgtttcttataaataaactctttgctattcagaaaacctcaaggggcccccacattcactaagcatggggctcctaactggggtccaggtccatagagtgtaggaagaacatattagaacaatacttgtgcttatttttatctagcttttttatgtttgtgtatgttttataatggcataatagtacaatggtacatgtacataattttaaataaataaatgaatgaatgaataaataaaaaaaaaaaaaa

SEQ ID NO: 57 - protein, 886 aa, Homo sapiens
MRAEEPCAPGAPSALGAQRTPGPELRLSSQLLPELCTFVVRVLFYLGPVYLAGYLGLSITWLLLGALLWMWWRRNRRGKLGRLAAAFEFLDNEREFISRELRGQHLPAWIHFPDVERVEWANKIISQTWPYLSMIMESKFREKLEPKIREKSIHLRTFTFTKLYFGQKCPRVNGVKAHTNTCNRRRVTVDLQICYIGDCEISVELQKIQAGVNGIQLQGTLRVILEPLLVDKPFVGAVTVFFLQKPHLQINWTGLTNLLDAPGINDVSDSLLEDLIATHLVLPNRVTVPVKKGLDLTNLRFPLPCGVIRVHLLEAEQLAQKDNFLGLRGKSDPYAKVSIGLQHFRSRTIYRNLNPTWNEVFEFMVYEVPGQDLEVDLYDEDTDRDDFLGSLQICLGDVMTNRVVDEWFVLNDTTSGRLHLRLEWLSLLTDQEVLTEDHGGLSTAILVVFLESACNLPRNPFDYLNGEYRAKKLSRFARNKVSKDPSSYVKLSVGKKTHTSKTCPHNKDPVWSQVFSFFVHNVATERLHLKVLDDDQECALGMLEVPLCQILPYADLTLEQRFQLDHSGLDSLISMRLVLRFLQVEERELGSPYTGPEALKKGPLLIKKVATNQGPKAQPQEEGPTDLPCPPDPASDTKDVSRSTTTTTSATTVATEPTSQETGPEPKGKDSAKRFCEPIGEKKSPATIFLTVPGPHSPGPIKSPRPMKCPASPFAWPPKRLAPSMSSLNSLASSCFDLADISLNIEGGDLRRRQLGEIQLTVRYVCLRRCLSVLINGCRNLTPCTSSGADPYVRVYLLPERKWACRKKTSVKRKTLEPLFDETFEFFVPMEEVKKRSLDVAVKNSRPLGSHRRKELGKVLIDLSKEDLIKGFSQWYELTPNGQPRS

SEQ ID NO: 58 - protein, 501 aa, Homo sapiens
MRAEEPCAPGAPSALGAQRTPGPELRLSSQLLPELCTFVVRVLFYLGPVYLAGYLGLSITWLLLGALLWMWWRRNRRGKLGRLAAAFEFLDNEREFISRELRGQHLPAWIHFPDVERVEWANKIISQTWPYLSMIMESKFREKLEPKIREKSIHLRTFTFTKLYFGQKCPRVNGVKAHTNTCNRRRVTVDLQICYIGDCEISVELQKIQAGVNGIQLQGTLRVILEPLLVDKPFVGAVTVFFLQKPHLQINWTGLTNLLDAPGINDVSDSLLEDLIATHLVLPNRVTVPVKKGLDLTNLRFPLPCGVIRVHLLEAEQLAQKDNFLGLRGKSDPYAKVSIGLQHFRSRTIYRNLNPTWNEVFEFMVYEVPGQDLEVDLYDEDTDRDDFLGSLQICLGDVMTNRVVDEWFVLNDTTSGRLHLRLEWLSLLTDQEVLTEDHGGLSTAILVVFLESACNLPRNPFDYLNGEYRAKKLSRFARVKQGQQRPFFLCQTICRQEDTYK

SEQ ID NO: 59 - RNA, 5992 nt, Homo sapiens
  source 1..5992: mol_type = mRNA
actcactggagccgagaactggggcggcgcggcgcggcgcggtgcatttccaggcgctgctctccgtcgcagagaaccctgagctcggcgcgccgagagtcccagcagggcaagggggcgcggcgtcctggtcctcgagcttgggagacagatgcgcatgggcgtgggggcatgcggacctaagctcgggtgaagctctcgggaagggcaagactgcggcgacgagatgcgagcagaggagccctgcgcccccggggcccccagcgccctgggagcccagcgcacgccgggccccgagctgcgcctgtccagccagctgctgcccgagctctgtaccttcgtggtgcgcgtgctgttctacctggggcctgtctacctagctggctacctggggctcagcataacctggttgctgctcggcgccctgctgtggatgtggtggcgcaggaaccgccgcgggaagcttgggcgcctggccgccgccttcgaattccttgacaatgaacgcgagttcatcagccgcgagctgcggggccagcacctgccagcctggatccacttcccggacgtggagcgggtcgagtgggccaacaagatcatctctcagacctggccctacctaagcatgatcatggaaagcaagttccgggagaaacttgagcccaagatccgagagaagagcatccacctgaggacctttacctttaccaagctctactttggacagaagtgtcccagggtcaacggtgtcaaggcacacactaatacgtgcaaccgaagacgtgtgactgtggacctgcagatctgctacatcggggactgtgagatcagtgtggagctgcagaagattcaggctggtgtgaacgggatccagttgcagggcaccctgcgggtcatcctggagcccctcctagtggacaagccctttgtgggagccgtgactgtgttcttccttcagaagccgcacctacagatcaactggactggcctgaccaacctgctggatgcgccgggaatcaatgatgtgtcagacagcttactggaggacctcattgccacccacctggtgctgcccaaccgtgtgactgtgcctgtgaagaaggggctggatctgaccaacctgcgcttccctctgccctgtggggtgatcagagtgcacttgctggaggcagagcagctggcccagaaggacaactttctggggctccgaggcaagtcagatccctacgccaaggtgagcatcggcctacagcatttccggagtaggaccatctacaggaacctgaaccccacctggaacgaagtgtttgagttcatggtgtacgaagtccctggacaggacctggaggtagacctgtatgatgaggataccgacagggatgacttcctgggcagcctgcagatctgccttggagatgtcatgaccaacagagtggtggatgagtggtttgtcctgaatgacacaaccagcgggcggctgcacctgcggctggagtggctttcattgcttactgaccaagaagttctgactgaggaccatggtggcctttccactgccattctcgtggtcttcttggagagtgcctgcaacttgccgagaaacccttttgactacctgaatggtgaatatcgagccaaaaaactctccaggtttgccagaaacaaggtcagcaaagacccttcttcctatgtcaaactatctgtaggcaagaagacacatacaagtaagacctgtccccacaacaaggaccctgtgtggagccaggtgttctccttctttgtgcacaatgtggccactgagcggctccatctgaaggtgcttgatgatgaccaggagtgtgctctgggaatgctggaggtccccctgtgccagatcctcccctatgctgacctcactcttgagcagcgctttcagctggaccactcaggcctggacagcctcatctccatgaggctggtgcttcggttcctgcaagtggaggaacgagagctggggagcccatacacaggacctgaagccctaaagaaaggccctctgctcatcaagaaagtggctaccaaccagggtcccaaagcccaacctcaggaagaaggccctacagatttgccatgtcccccagaccctgcttctgatactaaggacgtatccaggagtaccacaaccaccaccagtgctaccaccgttgccactgagcccacatcccaagagacaggcccagagcctaaaggcaaggacagtgccaaaaggttctgtgagcccatcggggagaagaagagtccagccaccatcttcctgactgtcccaggtccccactctccagggcccatcaagtcacccagacccatgaaatgccctgcctccccattcgcatggccgcccaagaggctggctcccagcatgtcctcgctcaactccttggcctcttcttgctttgacctggcagatatcagcctcaacattgaaggtggggacctcaggcgacggcagctgggtgagattcagctcacagtgcgctatgtgtgtctgcggcgctgcctcagcgtgctaatcaatggctgcagaaacctaacaccatgtaccagcagtggagctgatccctacgtccgtgtctacttgttgccagaaaggaagtgggcatgtcgtaagaagacttcagtgaagcggaagaccttggaacccctgtttgatgagacatttgaattttttgttcccatggaagaagtaaagaagaggtcactagatgttgcagtgaaaaatagtaggccacttggctcacacagaagaaaggagttaggaaaagtactgattgacttatcaaaagaagatctgattaagggcttttcacaatggtatgagctgactccaaatggacagcccagaagctgatgatgagaattcttatcactcacctttatattaaaatgtatatatatgtatatattttttcctttggatcacttacatccaatatatgtatattttgtcatttaaatcagaacaaccacttgaaattatatacatacaattcttgtgtggaatttaactccatgactgaatagcataaggaagaggttatttaaaagcaagaactactttttttggttggatttttttgttcaagtccagaaagaaatgttatatttgtgcctactaaattatccaaacctcagtgtttatatacttaaacaagtgccactttttagtaggtaattatataccatctgatttaggacttacctgaatgtatgtaccagaaagtgtcctgcctctggcataggggctgggggaggtctgtttctggagccactaccagcattcctgggcagtgactggccaaagggaagtcacttttttatggaaatagaaagtgacccaactcaaaactgccaagagctaacactgccaaagcccttctggctgccacctgtggtacttgtatgcctggatatttgttcttttatttgacctggagctaaaaatgtatttccctactggcaaaaatgttatactgatatacttaaataccttgagttaaatactcttgtgtagtctaagggccaaactccagcgtgtagcattatttccataggaaaatgcaaaccaagttccaagcccaggtctatgtctgactctcatagcaaagcactggagactgctgaagagtgtcaccatcagagaaaaggaagctttcagataagtttaggctattcaacttttctaaagagatggttggttcacctaaataacatgttaaaagcaaagtattaaattatatgcttaaacaagcgcctcttttacatttcagactttacaagaccaaatatacttctcatcccctccaacattcctggacctcctcttctctcttaccaacaccaacactacctgccgtcagttttctgtctctgcctctgccttcactgccacttttctgaagcagggcaacattcgagaacaaagttttgtcatgttactcttattccagtttcctgccatctgattcacatgcagatgttctattccagagtagtccaaatactatgctctgctgactcaagtcatgtctcaaacctatttcctctattaagtaagtcagtcaatccatagtgaaatggactcttcctaccgcctgtagcatttactgttgatactgagtattttccattttaatagttcccagcctttataacactaagttttaagaaatgttgattaggcatctgctaaggttacatgctaagcagctacttatattgtatttggtatttaattttgtttattctccagttgaacagtagggaacaattcaagctacttgaattgtttttcaccctcaccatccaagaccgtgttaagtacatagaagatgcatggtgaaattcgtttctgctgaggtttctattttaaatggcaaattctcataataaaatggagcattgatgcctaccctgtctaccttatgatggcattctaattgccccctaaatagacaagtgccttgaaaatggagaagcaccagagaaataagggaatgtatcatatgtacatcgaaacattagcaaccctaaaacagctaatcaaaatggcagataagtgaaaacctacccctcttcttccaaacttaaaccacaaacatttattttaaacgtggtcaattgaaccgtttttacctgtgtcaggcaacacaggtaaatacctggtgatggtctgaagaggagttaaaatgttgaagggaaccagaattttagtacacagcagacaggaggcaaggttatataggcgctgtgtgaggggcagggagcctgaaaagttgttaataccttggctgccactgaggacaagaattggttttcagcagtgggtggaaacaatcagctaatatgcaggagcatagggtctgaagttaacatcatcttggtacagaaacccccaaacctaagacggaatgtgaatattggtttagaacctggaagcctgtgaagccttgatggaggcaaccataaaattggccccacagggttgccactcccatccagggcacatatgcgacaactgcagcagatggctgtcactaaagggaaactcacgggcaaaaataaattatgaaacaaaacaaaaacagactttaaaaaaaatacaaagtacacaggaatatcaaactgaaaaatagccatagataatatttcagccagaaggaaaatgtaccagtaaggcagaaatagcatgtgagaagcagtggaaagcaaagaaatccataaaatacattggcaaacctaagcaagttttgatgatgattgttcacaagatataaacaaataaccaaagatttttgcaagggttcagaaacatagtagaactaaaatgttagtactaacaactaagaaggggcagctaggctgattaagaaagtaagtattcaagaccatatcttatttaggaagctaaagatactcatcttaaaaatataactgtgtcagtcactaattcattacctctcagcttcaaattgacgtctgtctcctttgctgctttcccggcaggctgatgtttggctttgccaatagggggcgatggaaggacactctatagcaggaagaaggggcttttcttctgatgttttccatggctgctagctaattggcatacagagctgttctcaatcaatcacctaagtacccccacagtttacccttggctcatggccttcatgttttatcagcaggcaacaccttttggcaagtttcttagccacaagtgggttgcatggtcctatggctgccagcggaaatctaaatctcagcctggtagggaggcacttagtttctaacttcctttcttgttcactctcccttacccctgggggtaaggatctgcatcctgaagttgatattctgtatcccctagagtccacttctaccccgtttagtagtaaatacaagaattgctaactagtaaaaggtggttaagtttttcaaaaaaaaaaaaaaaaaa

SEQ ID NO: 60 - RNA, 5110 nt, Homo sapiens
  source 1..5110: mol_type = mRNA
actcactggagccgagaactggggcggcgcggcgcggcgcggtgcatttccaggcgctgctctccgtcgcagagaaccctgagctcggcgcgccgagagtcccagcagggcaagggggcgcggcgtcctggtcctcgagcttgggagacagatgcgcatgggcgtgggggcatgcggacctaagctcgggtgaagctctcgggaagggcaagactgcggcgacgagatgcgagcagaggagccctgcgcccccggggcccccagcgccctgggagcccagcgcacgccgggccccgagctgcgcctgtccagccagctgctgcccgagctctgtaccttcgtggtgcgcgtgctgttctacctggggcctgtctacctagctggctacctggggctcagcataacctggttgctgctcggcgccctgctgtggatgtggtggcgcaggaaccgccgcgggaagcttgggcgcctggccgccgccttcgaattccttgacaatgaacgcgagttcatcagccgcgagctgcggggccagcacctgccagcctggatccacttcccggacgtggagcgggtcgagtgggccaacaagatcatctctcagacctggccctacctaagcatgatcatggaaagcaagttccgggagaaacttgagcccaagatccgagagaagagcatccacctgaggacctttacctttaccaagctctactttggacagaagtgtcccagggtcaacggtgtcaaggcacacactaatacgtgcaaccgaagacgtgtgactgtggacctgcagatctgctacatcggggactgtgagatcagtgtggagctgcagaagattcaggctggtgtgaacgggatccagttgcagggcaccctgcgggtcatcctggagcccctcctagtggacaagccctttgtgggagccgtgactgtgttcttccttcagaagccgcacctacagatcaactggactggcctgaccaacctgctggatgcgccgggaatcaatgatgtgtcagacagcttactggaggacctcattgccacccacctggtgctgcccaaccgtgtgactgtgcctgtgaagaaggggctggatctgaccaacctgcgcttccctctgccctgtggggtgatcagagtgcacttgctggaggcagagcagctggcccagaaggacaactttctggggctccgaggcaagtcagatccctacgccaaggtgagcatcggcctacagcatttccggagtaggaccatctacaggaacctgaaccccacctggaacgaagtgtttgagttcatggtgtacgaagtccctggacaggacctggaggtagacctgtatgatgaggataccgacagggatgacttcctgggcagcctgcagatctgccttggagatgtcatgaccaacagagtggtggatgagtggtttgtcctgaatgacacaaccagcgggcggctgcacctgcggctggagtggctttcattgcttactgaccaagaagttctgactgaggaccatggtggcctttccactgccattctcgtggtcttcttggagagtgcctgcaacttgccgagaaacccttttgactacctgaatggtgaatatcgagccaaaaaactctccaggtttgccagaaacaaggtcagcaaagacccttcttcctatgtcaaactatctgtaggcaagaagacacatacaagtaagacctgtccccacaacaaggaccctgtgtggagccaggtgttctccttctttgtgcacaatgtggccactgagcggctccatctgaaggtgcttgatgatgaccaggagtgtgctctgggaatgctggaggtccccctgtgccagatcctcccctatgctgacctcactcttgagcagcgctttcagctggaccactcaggcctggacagcctcatctccatgaggctggtgcttcggttcctgcaagtggaggaacgagagctggggagcccatacacaggacctgaagccctaaagaaaggccctctgctcatcaagaaagtggctaccaaccagggtcccaaagcccaacctcaggaagaaggccctacagatttgccatgtcccccagaccctgcttctgatactaaggacgtatccaggagtaccacaaccaccaccagtgctaccaccgttgccactgagcccacatcccaagagacaggcccagagcctaaaggcaaggacagtgccaaaaggttctgtgagcccatcggggagaagaagagtccagccaccatcttcctgactgtcccaggtccccactctccagggcccatcaagtcacccagacccatgaaatgccctgcctccccattcgcatggccgcccaagaggctggctcccagcatgtcctcgctcaactccttggcctcttcttgctttgacctggcagatatcagcctcaacattgaaggtggggacctcaggcgacggcagctgggtgagattcagctcacagtgcgctatgtgtgtctgcggcgctgcctcagcgtgctaatcaatggctgcagaaacctaacaccatgtaccagcagtggagctgatccctacgtccgtgtctacttgttgccagaaaggaagtgggcatgtcgtaagaagacttcagtgaagcggaagaccttggaacccctgtttgatgagacatttgaattttttgttcccatggaagaagtaaagaagaggtcactagatgttgcagtgaaaaatagtaggccacttggctcacacagaagaaaggagttaggaaaagtactgattgacttatcaaaagaagatctgattaagggcttttcacaatggtatgagctgactccaaatggacagcccagaagctgatgatgagaattcttatcactcacctttatattaaaatactttacaagaccaaatatacttctcatcccctccaacattcctggacctcctcttctctcttaccaacaccaacactacctgccgtcagttttctgtctctgcctctgccttcactgccacttttctgaagcagggcaacattcgagaacaaagttttgtcatgttactcttattccagtttcctgccatctgattcacatgcagatgttctattccagagtagtccaaatactatgctctgctgactcaagtcatgtctcaaacctatttcctctattaagtaagtcagtcaatccatagtgaaatggactcttcctaccgcctgtagcatttactgttgatactgagtattttccattttaatagttcccagcctttataacactaagttttaagaaatgttgattaggcatctgctaaggttacatgctaagcagctacttatattgtatttggtatttaattttgtttattctccagttgaacagtagggaacaattcaagctacttgaattgtttttcaccctcaccatccaagaccgtgttaagtacatagaagatgcatggtgaaattcgtttctgctgaggtttctattttaaatggcaaattctcataataaaatggagcattgatgcctaccctgtctaccttatgatggcattctaattgccccctaaatagacaagtgccttgaaaatggagaagcaccagagaaataagggaatgtatcatatgtacatcgaaacattagcaaccctaaaacagctaatcaaaatggcagataagtgaaaacctacccctcttcttccaaacttaaaccacaaacatttattttaaacgtggtcaattgaaccgtttttacctgtgtcaggcaacacaggtaaatacctggtgatggtctgaagaggagttaaaatgttgaagggaaccagaattttagtacacagcagacaggaggcaaggttatataggcgctgtgtgaggggcagggagcctgaaaagttgttaataccttggctgccactgaggacaagaattggttttcagcagtgggtggaaacaatcagctaatatgcaggagcatagggtctgaagttaacatcatcttggtacagaaacccccaaacctaagacggaatgtgaatattggtttagaacctggaagcctgtgaagccttgatggaggcaaccataaaattggccccacagggttgccactcccatccagggcacatatgcgacaactgcagcagatggctgtcactaaagggaaactcacgggcaaaaataaattatgaaacaaaacaaaaacagactttaaaaaaaatacaaagtacacaggaatatcaaactgaaaaatagccatagataatatttcagccagaaggaaaatgtaccagtaaggcagaaatagcatgtgagaagcagtggaaagcaaagaaatccataaaatacattggcaaacctaagcaagttttgatgatgattgttcacaagatataaacaaataaccaaagatttttgcaagggttcagaaacatagtagaactaaaatgttagtactaacaactaagaaggggcagctaggctgattaagaaagtaagtattcaagaccatatcttatttaggaagctaaagatactcatcttaaaaatataactgtgtcagtcactaattcattacctctcagcttcaaattgacgtctgtctcctttgctgctttcccggcaggctgatgtttggctttgccaatagggggcgatggaaggacactctatagcaggaagaaggggcttttcttctgatgttttccatggctgctagctaattggcatacagagctgttctcaatcaatcacctaagtacccccacagtttacccttggctcatggccttcatgttttatcagcaggcaacaccttttggcaagtttcttagccacaagtgggttgcatggtcctatggctgccagcggaaatctaaatctcagcctggtagggaggcacttagtttctaacttcctttcttgttcactctcccttacccctgggggtaaggatctgcatcctgaagttgatattctgtatcccctagagtccacttctaccccgtttagtagtaaatacaagaattgctaactagtaaaaggtggttaagtttttcaaaaaaaaaaaaaaaaaa

SEQ ID NO: 61 - RNA, 5036 nt, Homo sapiens
  source 1..5036: mol_type = mRNA
actcactggagccgagaactggggcggcgcggcgcggcgcggtgcatttccaggcgctgctctccgtcgcagagaaccctgagctcggcgcgccgagagtcccagcagggcaagggggcgcggcgtcctggtcctcgagcttgggagacagatgcgcatgggcgtgggggcatgcggacctaagctcgggtgaagctctcgggaagggcaagactgcggcgacgagatgcgagcagaggagccctgcgcccccggggcccccagcgccctgggagcccagcgcacgccgggccccgagctgcgcctgtccagccagctgctgcccgagctctgtaccttcgtggtgcgcgtgctgttctacctggggcctgtctacctagctggctacctggggctcagcataacctggttgctgctcggcgccctgctgtggatgtggtggcgcaggaaccgccgcgggaagcttgggcgcctggccgccgccttcgaattccttgacaatgaacgcgagttcatcagccgcgagctgcggggccagcacctgccagcctggatccacttcccggacgtggagcgggtcgagtgggccaacaagatcatctctcagacctggccctacctaagcatgatcatggaaagcaagttccgggagaaacttgagcccaagatccgagagaagagcatccacctgaggacctttacctttaccaagctctactttggacagaagtgtcccagggtcaacggtgtcaaggcacacactaatacgtgcaaccgaagacgtgtgactgtggacctgcagatctgctacatcggggactgtgagatcagtgtggagctgcagaagattcaggctggtgtgaacgggatccagttgcagggcaccctgcgggtcatcctggagcccctcctagtggacaagccctttgtgggagccgtgactgtgttcttccttcagaagccgcacctacagatcaactggactggcctgaccaacctgctggatgcgccgggaatcaatgatgtgtcagacagcttactggaggacctcattgccacccacctggtgctgcccaaccgtgtgactgtgcctgtgaagaaggggctggatctgaccaacctgcgcttccctctgccctgtggggtgatcagagtgcacttgctggaggcagagcagctggcccagaaggacaactttctggggctccgaggcaagtcagatccctacgccaaggtgagcatcggcctacagcatttccggagtaggaccatctacaggaacctgaaccccacctggaacgaagtgtttgagttcatggtgtacgaagtccctggacaggacctggaggtagacctgtatgatgaggataccgacagggatgacttcctgggcagcctgcagatctgccttggagatgtcatgaccaacagagtggtggatgagtggtttgtcctgaatgacacaaccagcgggcggctgcacctgcggctggagtggctttcattgcttactgaccaagaagttctgactgaggaccatggtggcctttccactgccattctcgtggtcttcttggagagtgcctgcaacttgccgagaaacccttttgactacctgaatggtgaatatcgagccaaaaaactctccaggtttgccagaaacaaggtcagcaaagacccttcttcctatgtcaaactatctgtaggcaagaagacacatacaagtaagacctgtccccacaacaaggaccctgtgtggagccaggtgttctccttctttgtgcacaatgtggccactgagcggctccatctgaaggtgcttgatgatgaccaggagtgtgctctgggaatgctggaggtccccctgtgccagatcctcccctatgctgacctcactcttgagcagcgctttcagctggaccactcaggcctggacagcctcatctccatgaggctggtgcttcggttcctgcaagtggaggaacgagagctggggagcccatacacaggacctgaagccctaaagaaaggccctctgctcatcaagaaagtggctaccaaccagggtcccaaagcccaacctcaggaagaaggccctacagatttgccatgtcccccagaccctgcttctgatactaaggacgtatccaggagtaccacaaccaccaccagtgctaccaccgttgccactgagcccacatcccaagagacaggcccagagcctaaaggcaaggacagtgccaaaaggttctgtgagcccatcggggagaagaagagtccagccaccatcttcctgactgtcccaggtccccactctccagggcccatcaagtcacccagacccatgaaatgccctgcctccccattcgcatggccgcccaagaggctggctcccagcatgtcctcgctcaactccttggcctcttcttgctttgacctggcagatatcagcctcaacattgaaggtggggacctcaggcgacggcagctgggtgagattcagctcacagtgcgctatgtgtgtctgcggcgctgcctcagcgtgctaatcaatggctgcagaaacctaacaccatgtaccagcagtggagctgatccctacgtccgtgtctacttgttgccagaaaggaagtgggcatgtcgtaagaagacttcagtgaagcggaagaccttggaacccctgtttgatgagacatttgaattttttgttcccatggaagaagtaaagaagaggtcactagatgttgcagtgaaaaatagtaggccacttggctcacacagaagaaaggagttaggaaaagtactgattgacttatcaaaagaagatctgattaagggcttttcacaatgactttacaagaccaaatatacttctcatcccctccaacattcctggacctcctcttctctcttaccaacaccaacactacctgccgtcagttttctgtctctgcctctgccttcactgccacttttctgaagcagggcaacattcgagaacaaagttttgtcatgttactcttattccagtttcctgccatctgattcacatgcagatgttctattccagagtagtccaaatactatgctctgctgactcaagtcatgtctcaaacctatttcctctattaagtaagtcagtcaatccatagtgaaatggactcttcctaccgcctgtagcatttactgttgatactgagtattttccattttaatagttcccagcctttataacactaagttttaagaaatgttgattaggcatctgctaaggttacatgctaagcagctacttatattgtatttggtatttaattttgtttattctccagttgaacagtagggaacaattcaagctacttgaattgtttttcaccctcaccatccaagaccgtgttaagtacatagaagatgcatggtgaaattcgtttctgctgaggtttctattttaaatggcaaattctcataataaaatggagcattgatgcctaccctgtctaccttatgatggcattctaattgccccctaaatagacaagtgccttgaaaatggagaagcaccagagaaataagggaatgtatcatatgtacatcgaaacattagcaaccctaaaacagctaatcaaaatggcagataagtgaaaacctacccctcttcttccaaacttaaaccacaaacatttattttaaacgtggtcaattgaaccgtttttacctgtgtcaggcaacacaggtaaatacctggtgatggtctgaagaggagttaaaatgttgaagggaaccagaattttagtacacagcagacaggaggcaaggttatataggcgctgtgtgaggggcagggagcctgaaaagttgttaataccttggctgccactgaggacaagaattggttttcagcagtgggtggaaacaatcagctaatatgcaggagcatagggtctgaagttaacatcatcttggtacagaaacccccaaacctaagacggaatgtgaatattggtttagaacctggaagcctgtgaagccttgatggaggcaaccataaaattggccccacagggttgccactcccatccagggcacatatgcgacaactgcagcagatggctgtcactaaagggaaactcacgggcaaaaataaattatgaaacaaaacaaaaacagactttaaaaaaaatacaaagtacacaggaatatcaaactgaaaaatagccatagataatatttcagccagaaggaaaatgtaccagtaaggcagaaatagcatgtgagaagcagtggaaagcaaagaaatccataaaatacattggcaaacctaagcaagttttgatgatgattgttcacaagatataaacaaataaccaaagatttttgcaagggttcagaaacatagtagaactaaaatgttagtactaacaactaagaaggggcagctaggctgattaagaaagtaagtattcaagaccatatcttatttaggaagctaaagatactcatcttaaaaatataactgtgtcagtcactaattcattacctctcagcttcaaattgacgtctgtctcctttgctgctttcccggcaggctgatgtttggctttgccaatagggggcgatggaaggacactctatagcaggaagaaggggcttttcttctgatgttttccatggctgctagctaattggcatacagagctgttctcaatcaatcacctaagtacccccacagtttacccttggctcatggccttcatgttttatcagcaggcaacaccttttggcaagtttcttagccacaagtgggttgcatggtcctatggctgccagcggaaatctaaatctcagcctggtagggaggcacttagtttctaacttcctttcttgttcactctcccttacccctgggggtaaggatctgcatcctgaagttgatattctgtatcccctagagtccacttctaccccgtttagtagtaaatacaagaattgctaactagtaaaaggtggttaagtttttcaaaaaaaaaaaaaaaaaa

SEQ ID NO: 62 - DNA, 22 bp, synthetic construct
  source 1..22: mol_type = other DNA; note = Sense primer for MMP13
atgaagaccccaaccctaaaca

SEQ ID NO: 63 - DNA, 21 bp, synthetic construct
  source 1..21: mol_type = other DNA; note = Anti-sense primer for MMP13
cggagactggtaatggcatca

SEQ ID NO: 64 - DNA, 18 bp, synthetic construct
  source 1..18: mol_type = other DNA; note = Sense primer for STMN2
aagccccacgaactttag

SEQ ID NO: 65 - DNA, 18 bp, synthetic construct
  source 1..18: mol_type = other DNA; note = Anti-sense primer for STMN2
cgtgttccctcttctctg

SEQ ID NO: 66 - DNA, 19 bp, synthetic construct
  source 1..19: mol_type = other DNA; note = Sense primer for THBS4
agagaggcagggggatgtg

SEQ ID NO: 67 - DNA, 21 bp, synthetic construct
  source 1..21: mol_type = other DNA; note = Anti-sense primer for THBS4
ttcttcgtcggggtaactgtc

SEQ ID NO: 68 - DNA, 24 bp, synthetic construct
  source 1..24: mol_type = other DNA; note = Sense primer for OMD positive tissue control
cagtaacagattagaatcaatgcc

SEQ ID NO: 69 - DNA, 27 bp, synthetic construct
  source 1..27: mol_type = other DNA; note = Anti-sense primer for OMD positive tissue control
gacattcttagagtatgaagttttgga